European Patent Application EP 4 269 584 A2, published November 1, 2023. Title: SELECTIVE ANTISENSE COMPOUNDS AND USES THEREOF. Applicant: Ionis Pharmaceuticals, Inc. The sequence listing filed with the application follows.

SEQUENCE LISTING (95 sequences)

SEQ ID NO: 1 - DNA, 202001 bp, Homo sapiens
  source 1..202001: mol_type = genomic DNA
gcccagcaggtgtcagcctcattttaccccgcccctattcaagatgaagttgttctggttccaacgcctctgacatattagctgcatcattttacatttcttttttttttttccttttaaatggggtcttgctctgtcacccaggctggagtgctgtggtatgatctcggctcactgcaatctccacctccgaggttccagcgattctcttgcctcagcctcccgagtagctgggactacaggcacccaccatcatactgggctaatttttgtgtttttagtagagatggggtttccccatgttgcccaggctgatctcaaactcctgggcttaagcaatacagccgcgttggcctcccaaagtgttgggattacaagcatgagctaccccacccagctcattttacatttccacttgttaaactgaaaactggcccgagaaagcttctgtactgccatccttgcgtccttgcagatgaatcgtaacctagcatagtaggtaggcagactgaaaacctaacttagcagtaggcttctgtaacaacagctgtgtctcagccagttcctgcagccagacttcaaccactcacaggccgcaaactgttcaaactgtgttcggagaaggcgaattcatctggctgttaacgtgcctcacttctgctttctgtggccactttcccttttctgtccataaatttgctttgaccacacagcatccctagagtctccctgaatctgctgtgattctgggacctgcaccatttgtgaattgttttttttttccttgatcagctaaactctgttcaattcaatttgttggaagtttttaacataccaatggtgcaccaaggttccaatttctccacttcctcataaataagtcattttaaatggcttttcagtattccaatatttggaagtattaatgtttctaccaattttctatttttggacattgaggttgtttcattttttttttctttttttgagacagagtctcgctccgtcacccaggctggagtgcagtggcctgatcccggcccactgcaacctccacctccctcctcagcctcctgagtagctgggattacaggtgcatgcaccaccacacccagctaatttttgtatttttagtagagatggggtttcaccatgttggtcaggctggtctcaaactcctgacctcaggtggtccacctgccttggcctcccaaaatgctgggattacaggcctgagccactgcgcctggcctcatcttcttgatattaatgttgctttaacatctttgtccctgtgttttttgtttttttttttgagacggagtctcattcattctgtcacccaggctggagttcagtggcgtgatctcagctcactgcaacctctgtctcctgggttccagtgattctcctgcgtcggtctcctgagtagctgtgttcctgggtctttcgatggttatttaatacttccctacagtaatgccctgtgcgtacatgctaagtgtgatgaaatggttggcacagttaaatcttttgaaagacattgccaagtcactcttcagaaaagtgataggaggtcatagcaattttaagaagtcctcatttctacatttccttactaatctcggttggtgtctcttcaatctttcctcacacttttcttgggtttttcctgaatcatgagtctactacatttacacattttaaagcatctttagaaacaggatctcattttgttgcccaggctagagtttggtggcatgattatagctcctcatactcctgggctcaagtgatccttccacctctgaaaccccaaaatttgagaaaggtctcatttaatttagaaagtttattttgccaaggttgagggtgcacacctgtgatgatatacgagttaaaaagaaattatttaggcagatactgagggtaagaaagtcctcggtaaggttttcttttcaatgaaaagcagcccccaagcattttcttttctaacaaagagcagcctgtaaaatcgagctgcagacatacacaagcaagctggaagcttgcacaggtgaatgctggcagctgtgccaataagaaaaggctacctggggccaggcagatccaacatggcggctccatcttccctttccttgtcaaccatgtgcacagtaaggagcaggcaacatagtgtcccccgagtagagaccaatttgcataataaaaggtgagggtagggtgggcagcttctttgcatgctatgtaaacattatgcctggtccaaccaatctttgggccctgtgtaaattagacaccacctcctcaagcctgtctataaaaccctgtccattctgccgcaggctggaagacccactggggcacccctctctctctataggagacagctattcatttttctctttctttcacctattaaagctccactcttaaccccactccgtgtgtatctatgttcttgatttccttggcatgaggcaatgaaccttgggtattaccccagaaccttgggtattatgccacttcagtgacacagcctcaggaaatcctgatgacatgttcccaagatggtcggggcacagcttggttttatacattttagggagacatgagacgtcaattcatatatgtaagaagtacattggttccgtccagaaaggcggggacaacttgaggcagggagagagcttctaggtcacaggtagacaaatggttgcattcttttgaatctccgataagcctttccaaaggaggcaatcagaatatgcgtctattgactgggcgcagtggctcatgcctgtaatgccagcactttgggaggcggaggtgggtggatcacctgaggtcaggagtttgagagcagcccggccaacatggtgaaaccctgtctctactaaaaatacaaaaaattagctgggcgtggtggcgggcgcctgtaatcccagctactcgggaggctgaggcaggagaatagcttgaacccagaaggaagaggttgcagtgagctgagatggtgccattgcactccagcctgggcaacaagagtgaaactccatctcagaaaaaaaaaaaaaaggcctgggcaaagtggctcacgcctgtaatcccagcactttgggaagccgaggcgggcaggtcacaaagtcaggagattgagaccatcctggctaacatgatgaaaccccatctctactaaaaaatacaaaaaactagctgggtgtggtggcgagcacctgtagtcccagctactcggcaggctgaggcaggagaatggcgtgaaccggggaggcggagcttgcagtgagccgagatcacaccactgcactccagcccggacgacagggcaagactctatctcaaattaaaaaaaaaaaaaaaaaaaaaaaaaaagagagagagaatatgcatctatctcagtgagcagaaggatgactttgaatggaatgggagcagttcctagcttgaacttcccctttagcttcagtgatttgggggctcaaggtatgttcctttcacatacctcagcctcccaagtagctgggaccacaagtgcatgccaccacacgtggctaatgttttattttttttgtaggaatagggtctcactatgtgtccaggctggtctaaaacccctgagctcaaatggtcctcccgcctcagcctcccgaaatgctgggattacaggcatgagccagcatgcccggcctagtctacatttttataaattgctaattcaaagttccctctccaaaacctcatggttttccctgttctcatcccctgcaccctcccttcccctggagtactcacctggccttggaggtctggtgtgagcccggacttcgattctaggcacagcatgtgatgagcgcccccaggtcaaacacctcccctctgcggcctgtgcttcaccgccttgacagtgagaaaggtctcccttcggctcattctcgaagtctcaaacttcacttctcctgtgcgctgattctgaattcagcccccgtccaaggtcctggcccctttctcttctgcttggcgtgttgttcatcaccactgtgcactgctgagggtaagtgcggttctctggacctctgctttatcattagaacagactcttgcggtttcccacgacattcctttcacttctcacttggaagatgagccgtgaggaaatcctgtgttgtgtggtatgtgggctgtgcttctgcttgacttgagggccaagcagcattgcaagccatggttttaaataagaaagaacatttctaaccttcatcttctagtaaggaaacaagtgggctttagagttcttgctcaggaaagacctatgtcccagtccaaccggaccttttactaaagagatcttcctgatcctcctccccaggccaggggaggggtcctccctggggttggagcctttagtagggggtcggagacacgacgtagccttcatgacattcatagtctagttacacgatccctgtaagggtcagttgaagtaagtgctacaaaggaagggaggtgctcagtggagagggctctcttttatgtattatatttctttcatggggagggatatggatcagggatcagcagaggtgtttcagtcccgagggaaagaaagtcagcgtggcttgggagttgggagcagcaagacagtggctcaagatatcttaagactagtggagtacaccttgcatgttaaaagccttgctcagggctgcctggttcttgtaggacgacagagatggcctagctctgcatactgcacccccaggggctcagaacagtgcaaatgtcagtctatctgtcagtggcagagccagccttggagcaggggtgcaaggaggtctctgcactggccaggcatgcagaacattctgttcagtagcactggacagaaggccccatctagatgagacagagctggtggggcaggacaaagactcctggcagctcaaacggcctggcagatgcttggagagagggggcttcttgagacagcaccatttctgggaagagagtcacctgggagggatgaggccacgctccggcttggaggtgaagagaggggctgctgcaagaaagaattagagacatgccagcctttgctgtgttgcccaggctggtcatgaactcttggcctcaagcaatcttcccacctcagcctccccaagcgctgggattatagacatgagcccccatgctggccaataaaagatgattttatggaggggatggtggtgaaggttgtgggtggtatgaaatagtaagaaatatatattggtctgcacccagttcctgccacagagctcctaaaatcctgagaacttcctgggtgagcatcttttgttctaatgaggtgactcttggtggctcctggataggagtgaatcaccagaaagatcaagccagagttagaagcagaaagtgctggctataacacaggaaagctgtaacacaaataataaagtttttttttttttttttgagatggagcctcactctgttgcccaggctggagtgcaatggtgcaatctcagctcactacaagctctgcctcccaggttcaagtgattctcctgcctcagcctcctgagcagttgggactacaggtgtgtgccaccacatctggctaatttttgtatttttagcagagacggggtttcaccatattaaccaggctggcctcaaactccttaccttgtgatccgcctgcctcagcctcccaaagtgctgggattacaggcatgagccaccgtgcctggccaaaagacattgttcttaaaagaatcaactaactaaccaaataaataaaaatctaacctaattaagaaactaaaaatacacaaaaattaatttcaaggggagaaaaatcatgtaaagagagaaagataatgaatactttgcagaaatttatgaacataaacataaaacttggatgaaatgcatttctaggaaaacataatttatcaaaactaaccacaagtaaaatagaagcctaaataggatattttcaagagaagaagtaaagttgtcaaagtgctacccttcaaaaaaacaccaggctcaaacaatctgacatgggaatgttagcacaccttagagagcaaataaaactttgaatgggcttgaaatattccagactctagaaaaacaaaacttcccaattctttttataaagcaagtataaattgataccaaaatcttataaagaccttatacaaaacttcataccaatctcttttatgaatacaaaacccttaataaagtattaccagacagaacccaacaatacataaaaatgtcacatcataacatagtggggtttatttcaataatgcatggatggttcaatacaaggaaattcagtaacacaatataatagatcatgtgaatatacccaaagaaaaaatagattattttcatagatgctgtaaaggcatttgaccaaattcaacacctactttttaggtggtcaataaaataaattagttactccttctttagcatgataaaatatatttatcagcccagaaggcatcattttacccgataagggcacacgctggagggaataatgttaaaattaggaataagaggatagctagtttctttcttcttttttttttttgagacggagtcttgctctgttgccaggctggagtgcagtggtgcaatgttggctcactgcacgccccccgcctcccaggttcaagcgattctcctgcctcagcctcccgagtagctgggactacaggcgcgcaccaccatgcccggctaatttttttttgtattttagtagagatggggtttcaccatgttggtcaggctggtcttgaactcccaacctcacgtactgggattaccggtgtgagccaccacgccagcccaactactttcaacattatccttaatactgatgcttattgacttactatggggttacctctagataaatccataataagttgaaaatataagtaaaaaatgcccttaatacacctaacctaccaaacatcatagctgagcccagcctgccttagctatgctcagacactgacgtcagcctacaattggcaaaatcacacagcagcacagtctactgcagagcatctgctgtttgcccttgtgactgcgtggctgcctgggagcttcccagcttcacaagacagtattacgtagcacatcactagcctggggaaagatcaaagttgaaaatttgaagtgtggtttccattgaatgtgtactgcttttgcaccatcatcaagtcaaaaaattttagttgaaccagcctaagtttgggaccatctttattttcaggaggaacttccatgtacattgatgacggacgatagaatccgtttctatcatcctaatgaacataatgaataaatccagacaaacataaacattaacagagtaagcagctttcggggctggaagccagaagagggtgggagcgcagagagagaggccaaacaccagggctgcttctgctttgcgggtatttgctgatctggacaaggtatctggaaggctgagctaagcctcctttttttttgaggtggcgtctcactctgttgccaggctggagtgcaatggtgcgatctcagctcactgcaacctccacctccctggttcaagcgattctcctgcctcagcctcccgagtagctgggattacaggctcccgccactacacccagctgatttttgtaattttagtagagacggggtttcaccatgttggccaggatggtctcgatctcttgacgtcatgatctgtccacctcggcctcccaaagtgctgggattataggcgtgacccaccgtgccccgtctgagctaagcctcttgagcataggggactaaaaatgaaatctagcgcatgccaagtttagggtcccaggcaattcctttccactttggggtccactttggggtccaccccacccaagaagaaggatgacttggaagtaaaccagctctgaaatatggatggtcctctgggaccataccaatcccttcatatcaaccacatccagttcctcaaaactggaacttggattaagatggcctaggacttctagtgtcccaggagcctggcattgcaaacaaaaatcctctccggaagaagataataccttaagcttcaaatgactctctaataaatttcaaatacaatgtccagcacacaaacacaaattaccaggaacgtgatatgaggcctgatggatgggaattagcagaaacttcaggcatgagaaacataccctcagaggcctagaatctatctagtgtctagataatggagatatgaaatacagacacttaaacaactatgtttcccatgttcaaagaggaaatttgcaaaacttgaaagtgttggcaggaaatcagaaactataaaatgtgacaacagcatactttagagtcagtataaattacggtcccgaaaactgcagaattccagaacttaatggtaaagcaagggtttaacagcagaatagaaatagccagagagaactaggaagtaagtcagatgacactacccagaataaggcactgagaggccaaggaatggaaaatgcagaagaaaggatatggtgagaggatctaatatacatttatttggagtaccagggagagagagaaggagaagaacagaagccgtgtttcaaggacggtgactgagaggcttcgaaactgatgaaagccatcagttcacaaattcaaagcccagtgaattccaaggagaaaaaaagaaatccatactgtgaaagcaagtccagacaatgacaaacaccatcaacaatacacaggacaggcataagatgcatttaatggggacactcagaggcagagggttatcagaaggaggcacttctctcccaagttctcatcatcccagggccagggacagctggtcacaccttagggagttcactaggagagggatctggcttcttgtcattctgggtatttgtagggaaattggaagggaaccgagagcacctagccaatcgcatagcaatgggagatttcaggctgtggggaatgtctttgctggtgaaaagaacatcctgaccttagaaatctttcaccgagggggatctgcgttccagaacttctggagctggtataggtaaggctttgagctttcctactgagccagcctgttgctaggttaccaaaggggacctcgagggccatctggccaacaagcagacttgtctctccttacacccccagacgtatcactgcaaaactacagaaaaccaaagacagagaaaatcttaaaagcagccagatttaaaaaatggcatattagtttcaaagcagcagccatgaaattgacagctgatgtctcaacagcaagaatgaaaagtggaagacaggccaggtgtggtggctcaggcctgtaatcccagcactttgggaggccgaggcgggtggatcacgaggtcaggagaccaagaccatcctggctaacatggtgaaaccccgtctctactaaaaatacaaaaaaattagtcgggcatggtggtgggtgcctgtagtcccagctactcgggaggctgaggcaggagaatggcgtgaacccgggaggcggagcttgcagtgagccgagattgtgccactgcactccagcctgggtgacagagcaagactctgtctcaaaaaaaaaaaaaaaaaaaaaaaaaaaagggtgacgaagcttcaatctcctgaaaggaagcaactgccgcctttgattcgatacccaccaaaatccgtgaagaaggaaggcaaaataaaaacacttcctgattgaactggaaagatttccgcaatagaagacccactgtccaaggaattctaaaggatgctttccaggcagaagaaaatgaccccagaggaagatcagagattcaggaaagaaatggagagtgataaaaatggaaaattcgggggccaatttaaacaaaagctgactgctctacaactgttgtgtctctatcttttgtaacatatatgtgtgtgtagcttttttttttttttttgtcaagatggattctcactctgtcgcccaggctacagtgaaatggcacggtctcggctcactgcaacctctgccccttgggctcaaatgattctcttgcctcagcctcctgagtagctgagattacaggtgcctggcacaatgcctggctaatttttgtatttttactagagatgggatttctccatgttggccaggctggtcttgaacacctgacctcaggtgatccacctgcctgggcctcccaaagtgctaggattacaggcgcgagccactgcatctggcctatgtgtgtgtttatatggaattaaaacacatggcaataataccctccaaattgggagaaaccaaaaatagcatttaaatgttgtaagctccctgcataatcaagaagagaatagatttacgttagattttgatacctggaggatgaatgttgtaatttctagggtgaccatgaaaagaggagacaacggtgtatgtttttttttttttgagatggagtctcactttgtcacccaggctggagtgttgtggtgtgatcttggctcactgcaacctcctcctcttgggttcaggccatcctcccacctaggcctccagagtaggtgggatcacaggcacctgccaccacacctggctaatttttttttttttttaaatatttagtagagatggggtttcaccatgttggccaggctggtcttgaactcctgacctcaggcgatctgcctacctctgcctctcaaagtgctgggattacaggtgtgagccatcgcgcccggccaacagtgatcactttcaaactaacagaggttcaaaaataaaatcagacttaaccaaaaaccaggtaacagagctggtaggatatacagaaagactgacctcacgtatatcaacgattacagttaatattaatgaaggaaatgctctagtttaaaaacgagggttgtcaaagaccccacataagaagctccttaccagcggtgcacctagaacctaaggaaacaggacagatgaaggaggacgcgcccccgccgctgtcctgcgcctcagccatcctatgagacgggaaaggtttctgtctgcagctgggcccgtgctctttaccagctcctggctttcttctctggaaggttcctgcctgttttgccctcacacctgctcctctctcagccctctcaggggtggggctggaggccaccaaagagcctcctctgctctccagttgctcgactgctcctcatttccccctggggtctgcgtcagggtttccttcttttccagccccaccccgcgtgcatcccacctggtctcgggtcggggctgctcccgcttactgccccctgcccaggctggtgtgcaccccctctggctgctttcaaggcctcttctctcttctcggcaggacaggcacaggcaggtggccaggtgtcatgcttagctccccgcccagtgagattctttcatttaacaatcttcccctgaatagttcatgttcattgctgaaaatttgaaaaatatggaaaagcacaaagattaagatataaaccgccctcaattcccctgcccagagagagtcactgctatgacttggtgactaggaaccttatttctctctcgctcttttttttttttttgagacagagtcttgctctgtcacccaggctggagtgcagtggctcgatctcagctcactgcaacctccgcctcctgggttcaagcgattctcctgcctcagcctcttgagtagctgggattacaggcacctgccaccatgcccggctaatttttgtatttttagttgagagagggtttcatcttgttggtcaggcggacttgaactcctgacctcaggtgatcagcccacctcggcctcccaaagtgctgggattacaggtgtgagccactgcgccttcatctctcttctgtgtatgtgtacgctgttttttctttagaatgggggacgttatcaggctctacatggtgtgtagtcggctagcatgttgtaagcctttccctgtgtcacaagtgctcatctggaacaggattctaatgactgcctgtggctatgttgggattcctttaactcagctccttctgcccagcatctatcttttttccatcttttgtcctaagtgttgctataataaatcattgatcacacatgcctgactgtttgcataggataaattacgggaaatgtttttgctgttcagggactgtgcccatttttaggcctcagagacaccatgccagactgcccagtattgatctttactctttttagatgatgccaaacttttctgtgaactttaaaaacctgtgtcttgacagtccatttctgtaagtctttcacattagatttcctgtcaggatgatagtcaattctaggcagatgatgttttctcagccatggctgaagcagttgtgatttgttgtggccatgtaaagtcccgatgatccattgcctccctggatgggttggaataatttggtttgggagcatataacagaatgacctggagtcacagcagctcagacggaagtgtatttctcccttacagatgaaagaattccaggccaggctggaatgacaactgcacacagtcatctgggccccctccttccagctcccatcaccccaggatgtggcttttatgcagatgatccaaaatggctgctcaagtcccagccaacacatcccattccagggagcaggaaaaaggtgtgtctttcccttcattttatgtgattcctttctagaagtactactcattacttctgcttgcatctccctggctagcacttacttagttatatggccatagctagctgaaggaaggacagggactgtcatacactagctaagaggcaaactgcttagataaaaaggtctctaaagaaggtcagagcggctgctagggtgcaactctattacttattgttatgggacgaactgtgtccctcattcaggttgatgtcctaagccccagaacctcagaatgggattgtatttggagacaggttctttaaggaggtaaggaggctaaaatgagatcattagggtgggccataatccgactgatgtcttacaagaagagattaggacacggacatgctcagagggacggccacgtgaggacaccaagaaaggcagctgtctgcaagtcaaggacagggctcaggggaaaccaaccttgccaacaccttcatctcggacttctagcctctaggaccatgagaagatacatttctgttgtttaagctgcccggtctgtggtactttgttatggcagcccaagtaaacaaatacagtcatctgctgctggaacaaatcaccccagcactgtggcttggcagcacacatgtctagtcatagagttatatgtagttacgtgtagagccatatgtatcgtcacacgttctgtgggtcaggaatttggacccagcttaaccagctccacttctcgccagggttcagtcaaataccagctgcctcccacctgagagctcagccggggaagggtccctttccaatctcacgtggtgttggcaggatccagttcctcatggcctgctggactgagaacctcagttctcactgcctgttggccagaggccgcctttatgtcctcgccatgtgggcctctccaacatggcagctgacttcatcagagcatccatgccaagaaggcaacagagagggccagggagactgaagtcatacccttttgcgacctagtcatggggtgacattccatcacctttgcccattggttagaagcaggccaccaggtacagcccaagctcacggggaggggtcatacaagggtgtcaataccaggaggtgaggggtgctggggccatcttatgagtctgcccactgaggtaactaacaaccttgaggcctgacacagtggacaaaggcccttattaacagcagagaactgggaactttatttatttatttatttttgagacagagtctcactcttgtcacccaggctggagtgcaatggcatgatcttggctcactgcaacctccacctcccaggttcaagcaattctgcctcagcctccggaatagctgggactacaggcatgcaccactacacccggctaatttttgtatttttagtagagacagggtttcgccatgttggccaggctggtctcgaactcctgacctctggtgatctgcctgccttggcctcccaaagtgctgggattacaggcgtgagccaccgcacctcgctggaacttaatttttttagagacagtgtcgctctatcacccaagctggagtgcagtggtgcaatcctagctcacttgcagcctcaaattcctgggttcaggtgatcctcccacatcagcctcccaagaactgggaactaacagctgtttctctgctgtccttctcaagaaaagggaggctactgctaccccactggggacaatgctgggtttccctttaggacaggctctgagacaaggcggaggtgctgtttgtggccacagagcaggggactctgggttgcaggtgtggcctggctaaagtaggctttactgggctcctctctgcctgcatcaccccccggctgggcggttgtctctgaggccaaccttactccctgctgggcaggctggacagctgccctctccgtttgcccctctaccacccaaaaggcaggaggctctggagaccaggaccctgcccgccacggcctgtgtcccaggcgtgagggggtgccccacagacctctgctgagctgctgctgaatgacgccccttgggggtcctgccggaaggtcagagcaggggtgcactcccataaagaaacgcccccaggtcgggactcattcctgtgggcggcatcttgtggccatagctgcttctcgctgcactaatcacagtgcctctgtgggcagcaggcgctgaccacccaggcctgccccagaccctctcctcccttccggggcgctgcgctgggaccgatggggggcgccaggcctgtggacaccgccctgcaggggcctctccagctcactgggggtggggtgggggtcacacttggggtcctcaggtcgtgccgaccacgcgcattctctgcgctctgcgcaggagctcgcccaccctctccccgtgcagagagccccgcagctggctccccgcagggctgtccgggtgagtatggctctggccacgggccagtgtggcgggagggcaaaccccaaggccacctcggctcagagtccacggccggctgtcgccccgctccaggcgtcggcgggggatcctttccgcatgggcctgcgcccgcgctcggcgccccctccacggccccgccccgtccatggccccgtccttcatgggcgagcccctccatggccctgcccctccgcgccccacccctccctcgccccacctctcaccttcctgccccgcccccagcctccccacccctcaccggccagtcccctcccctatcccgctccgcccctcagccgccccgcccctcagccggcctgcctaatgtccccgtccccagcatcgccccgccccgcccccgtctcgccccgcccctcaggcggcctccctgctgtgccccgccccggcctcgccacgcccctacctcaccacgccccccgcatcgccacgccccccgcatcgccacgcctcccttaccatgcagtcccgccccgtcccttcctcgtcccgcctcgccgcgacacttcacacacagcttcgcctcaccccattacagtctcaccacgccccgtcccctctccgttgagccccgcgccttcgcccgggtggggcgctgcgctgtcagcggccttgctgtgtgaggcagaacctgcgggggcaggggcgggctggttccctggccagccattggcagagtccgcaggctagggctgtcaatcatgctggccggcgtggccccgcctccgccggcgcggccccgcctccgccggcgcagcgtctgggacgcaaggcgccgtgggggctgccgggacgggtccaagatggacggccgctcaggttctgcttttacctgcggcccagagccccattcattgccccggtgctgagcggcgccgcgagtcggcccgaggcctccggggactgccgtgccgggcgggagaccgccatggcgaccctggaaaagctgatgaaggccttcgagtccctcaagtccttccagcagcagcagcagcagcagcagcagcagcagcagcagcagcagcagcagcagcagcaacagccgccaccgccgccgccgccgccgccgcctcctcagcttcctcagccgccgccgcaggcacagccgctgctgcctcagccgcagccgcccccgccgccgcccccgccgccacccggcccggctgtggctgaggagccgctgcaccgaccgtgagtttgggcccgctgcagctccctgtcccggcgggtcccaggctacggcggggatggcggtaaccctgcagcctgcgggccggcgacacgaacccccggccccgcagagacagagtgacccagcaacccagagcccatgagggacacccgccccctcctggggcgaggccttcccccacttcagccccgctccctcacttgggtcttcccttgtcctctcgcgaggggaggcagagccttgttggggcctgtcctgaattcaccgaggggagtcacggcctcagccctctcgcccttcgcaggatgcgaagagttggggcgagaacttgtttctttttatttgcgagaaaccagggcgggggttcttttaactgcgttgtgaagagaacttggaggagccgagatttgctcagtgccacttccctcttctagtctgagagggaagagggctgggggcgcgggacacttcgagaggaggcggggtttggagctggagagatgtgggggcagtggatgacataatgcttttaggacgcctcggcgggagtggcggggcagggggggggcggggagtgagggcgcgtccaatgggagatttcttttcctagtggcacttaaaacagcctgagatttgaggctcttcctacattgtcaggacatttcatttagttcatgatcacggtggtagtaacacgattttaagcaccacctaagagatctgctcatctaagcctaagttggtctgcaggcgtttgaatgagttgtggttgccaagtaaagtggtgaacttacgtggtgattaatgaaattatcttaaatattaggaagagttgattgaagttttttgcctatgtgtgttgggaataaaaccaacacgttgctgatggggaggttaattgccgagggatgaatgaggtgtacattttaccagtattccagtcaggcttgccagaatacggggggtccgcagactccgtgggcatctcagatgtgccagtgaaagggtttctgtttgcttcattgctgacagcttgttactttttggaagctaggggtttctgttgcttgttcttggggagaatttttgaaacaggaaaagagagaccattaaaacatctagcggaaccccaggactttccctggaagtctgtgtgtcgagtgtacagtaggagttaggaagtactctggtgcagttcaggcctttctcttacctctcagtattctatttccgatctggatgtgtcccagatggcatttggtaagaatatctctgttaagactgattaatttttagtaatatttcttgttctttgtttctgttatgatccttgtctcgtcttcaaagtttaattagaaaatgattcggagagcagtgttagcttatttgttggaataaaatttaggaataaattattctaaaggatggaaaaactttttggatatttggagaaattttaaaacaatttggcttatctcttcagtaagtaatttctcatccagaaatttactgtagtgcttttctaggaggtaggtgtcataaaagttcacacattgcatgtatcttgtgtaaacactaaacagggctcctgatgggaaggaagacctttctgctgggctgcttcagacacttgatcattctaaaaatatgccttctctttcttatgctgatttgacagaacctgcatttgcttatcttcaaaatatgggtatcaagaaatttcctttgctgccttgacaaaggagatagattttgtttcattactttaaggtaatatatgattaccttatttaaaaaatttaatcaggactggcaaggtggcttacacctttaatccgagcactttgggaggcctaggtggacgaatcacctgaggtcaggagtttgagaccagcctggctaacatggtgaaaccctgtctctactaaaaatacaaaaattagctggtcatggtggcacgtgcctgtaatccaagctacctgggaggctgaggcaggaaaatcgcttgaacccgggaggcagagtctgcagtgagttgagatcacgccactgcactccagcctgggtgacagagcgagactctatctcaaaaaaaattttttttaatgtattatttttgcataagtaatacattgacatgatacaaattctgtaattacaaaagggcaataattaaaatatcttccttccacccctttcctctgagtacctaactttgtccccaagaacaagcactatttcagttcctcatgtatcctgccagatataacctgttcatattgtaagatagatttaaaatgctctaaaaacaaaagtagtttagaataatatatatctatatattttttgagatgtagtctcacattgtcacccaggctggagtgcagtgatacaatctcggctcactgcagtctctgcctcccaggttcaaatgcttctcctgcctcagccttctgagtagctgggattacaggcgcccaccaccatgtccagctaatttttgtatttttagtagagatggggtttcaccatgttggccaggctggtcttgaactcctgaccttgtgatctgtccacctcggcctcccaaagtgctgggattacaggtgtgagccaccatgcctggctagaataataacttttaaaggttcttagcatgctctgaaatcaactgcattaggtttatttatagttttatagttattttaaataaaatgcatatttgtcatatttctctgtattttgctgttgagaaaggaggtattcactaattttgagtaacaaacactgctcacaaagtttggattttggcagttctgttcacgtgcttcagccaaaaaatcctcttctcaaagtaagattgatgaaagcaatttagaaagtatctgttctgtttttatggctcttgctctttggtgtggaactgtggtgtcacgccatgcatgggcctcagtttatgagtgtttgtgctctgctcagcatacaggatgcaggagttccttatggggctggctgcaggctcagcaaatctagcatgcttgggagggtcctcacagtaattaggaggcaattaatacttgcttctggcagtttcttattctccttcagattcctatctggtgtttccctgactttattcattcatcagtaaatatttactaaacatgtactatgtgcctggcactgttataggtgcagggctcagcagtgagcagacaaagctctgccctcgtgaagctttcattctaatgaaggacatagacagtaagcaagatagataagtaaaatatacagtacgttaatacgtggaggaacttcaaagcagggaaggggatagggaaatgtcagggttaatcgagtgttaacttatttttatttttaaaaaaattgttaagggctttccagcaaaacccagaaagcctgctagacaaattccaaaagagctgtagcactaagtgttgacatttttattttattttgttttgttttgttttttttgagacagttcttgctctatcagccaggctggagtgcactagtgtgatcttggctcactgcaacctctgcctcttgggttcaagtgattctcatgcctcagcctcctgtttagctgggattatagacatgcactgccatgcctgggtaattttttttttttcccccgagacggagtcttgctctgtcgcccaggctggagtgcagtggcgcgatctcagctcactgcaagctccgcttcccgagttcacgccattctcctgcctcagtctcccaagtagctgggactacaggcgcctgccaccacgtccagctaatttttttgtatttttaatagagacggggtttcaccgtgttagccaggatgatcttgatctcctgacctcgtcatccgccgaccttgtgatccgcccacctcggcctcccaaagtgctgggattacaggcatgagccactgtgcccggccacgcctgggtaatttttgtatttttagtagagatggggttttgccatgatgagcaggctggtctcgaactcccggcctcatgtgatctgcctgccttggcctcccaaagtgctaggattacaggcatgagccaccatacctggccagtgttgatattttaaatacggtgttcagggaaggtccactgagaagacagctttttttttttttttttttggggttggggggcaaggtcttgctctttaacccaggctggaatgcagtatcactatcgtagctcacttcagccttgaactcctgggctcaagtgatcctcccacctcaacctcacaatgtgttgggactataggtgtgagccatcacacctggccagatgatggcttttgagtaaagacctcaagcgagttaagagtctagtgtaagggtgtatgaagtagtggtattccagatggggggaacaggtccaaaatcttcctgtttcaggaatagcaaggatgtcattttagttgggtgaattgagtgagggggacatttgtagtaagaagtaaggtccaagaggtcaagggagtgccatatcagaccaatactacttgccttgtagatggaataaagatattggcatttatgtgagtgagatgggatgtcactggaggattagagcagaggagtagcatgatctgaatttcaatcttaagtgaactctggctgacaacagagtgaaggggaacaccggcaaaagcagaaaccagttaggaagccactgcagtgctcagataagcatggtgggttctgtcagggtaccggctgtcggctgtgggcagtgtgaggaatgactgactggattttgaatgcggaaccaactgcacttgttgaactctgctaagtataacaatttagcagtagcttgcgttatcaggtttgtattcagctgcaagtaacagaaaatcctgctgcaatagcttaaactggtaacaagcaagagcttatcagaagacaaaaataagtctggggaaattcaacaataagttaaggaacccaggctctttcttttttttttttttgaaacggagtttcgctcttgtcacccgggctggagtgcaatgatgtgatctcagctcactaaaacctctacctcctgggttcaagtgattcttctgcctcagcctcccaagtaactgggattacaggcgtataccaccatgcccagctaatttttgtgtttttagtagagatggggtttcaccatgttggccaggctggtctcgaacttctgacctcaggtgatccactcgcctcagcctgccaaagtgctgggattacaggtttgggccactgcacccggtcagaacccaggctctttcttatacttaccttgcaaacccttgttctcattttttccctttgtatttttattgttgaattgtaatagttctttatatattctggatactggattcttatcagatagatgatttgtaaaaactctcccttcctttggattgtctttttactttcttgatagtgtcttttgaagtgtaaaagtttttaattttgatgaagtcgagtttatctattttgtctttggttgctgtgcttcaagtgtcatatctaagaaatcattgtctaatccaaagtcaaaaaggtttactcctatgttttcttctaagaattttagagttttacatttaagtctgatccattttgagttaatttttatatatggttcaggtagaagtccaactttattcttttccatgtggttattcagttgtcccagcactgtttgttgaagagactattctttccccatggaattatcttagtacccttgttgaaaattaatcgtccttaattgtataaatttatttctagactgtcagttctacctgttggtctttatgtcgatcctgtgccagtaccatacagtcttgattactgaagtttgtgtcacagtttaaattcatgaaatgtgagttctccaactttgttccttttcaagattgatttggccatgctgggtcccttgcatttccgtacgaattgtaggatcagcttgtcagtttcaacaaagaagccaagtaggattctgagagggattgtgttgaatctgtagatcaacttggggagtattcgcatcttaacaatattgtcttccacctatgaacatgggcaaactttgtgtaaatggtcagattgtaagtatttcgggctgtgtgggcacagtgtctctgtcacagctacgcggctctgccattgtagcatgaaagtagccataagcaatatgtatgagtgtctgtgttccaatagaattttattaatgacaaggaagtttgaatttcatataattttcacctgtcatgagatagtatttgattattttggtcaaccatttaaaaatgtaaaaacatttcttagcttgtgaactagccaaaaatatgcaggttatagttttcccactcctaggttaaaatatgataggaccacatttggaaagcatttctttttttttttttttttttttttttgagacggagtttcactcttgttgcccaggctggagtgcagtggcgcgatctcggctcactgcaacctctgcctcccaggttcaagacattctcctgcacggcctccctagtagctgggattacaggcatgcgccaccacacccagctaattttgtatttttagtagagacggggtttctccatgttggtcaggctggtcttgaactcctgacctcaggtgatccacccgcctcagcctcccaaagtgctgggattacagggtgtgagccaccacaccctgctggaaagcatttcttttttggctgtttttgttttttttttaaactagttttgaaaattataaaagttacacatatacattataaaaatatcttcaagcagcacagatgaaaaacaaagcccttcttgcaagtctgtcatctttgtctaacttcctaagaacaaaagtgtttcttgtgtcttcttcccagattttaatatgcatatacaagcatttaaatgtgtcattttttgtttgcttgactgagatcacattacatatgtatttttttacttaacaatgtgtcatagatattgttccatagcagtacctgtaattcttattaattgctatgtaatattttagaatttctttttaaaagaggacttttggagatgtaaaggcaaaggtctcacatttttgtggctgtagaatgtgctggtgacatattctctctaccttgagaagtccccatccccatcacctccatttcctgtaaataagtcaaccacttgataaactacctttgaatggatccacactcaaaacatttagtcttattcagacaacaaggaggaaaaataaaataccttataaagcactgtttaatattgtattaaattggatcaatttgggggctagaatgtatgttagagacatgatatgtccataggtccttgctatcacagtgaggtctcagggacagtcgtttggtatcatttgggatctcataagcagactctctctgcttgacctgacaaatcagagtctgtgttttaacaggttcagtgagtgacttacatgcacattggagtttgggaagctccactgtaggtgcttagaccttacctttgttgttgctaataacaatgcaagcatttgggaggaagacctgtgttgctcatatgtgtccaggtgtagctgaggtggccttgcttatctgctgtagggccgttgagcatttctgtagctgtgatgagtgagctgaggtgagcctgcggagagctcccagccattggtagtgggactcgcttagatgaactggaaggaccctttcatctgagcagccactatggagaaaaacaaccgaatgaggggagagacaatgtgcaattttatttagggcacaaaggagagctgtggttagaaggtgacatttgagtggaaagggggcaagccatgtgtatagcgggagaagagaggtccaggcagagttaacagaaggcagaaatgctttccatgtttgagaaccagtaaggaggccagtggctgaagtaaggtgaagggcagaaataaggatgaggctgcgagagatgagaggttagagacgagcgtcttgtgcaccaagataagcttgtgtggtcaaaacaagtagtttaatttatgtttttaaaagatcattttggctgggcacaatggttcatgcctgtaataccagtagtttgagacggtgtggtgggaggattgcctgaggccagacgaccagcatagccaacatagcagcacctataaggtctctacaaaaaactttaaaaaattagctgggcatagtggtgtgtgcctgtagtcccagctactcaggaggctgaggaggctggaggattgcttgagtccaggagtttgaggctgcagtgagctatgattatgccactacactacaacctgggcaagagagtgagaccctgtctctaaatatacacacacacacacacacacacacacacacacacacacacacacacacacacacacatatatatgtatatatatgcatttagatgaaaagatcactttgacaataccacatgctggtgaggatttagaaaaactaggtcacttattgctggtgggaatataatatagtacggccactctggaaaacagtttggcagtttgtcataaaactgaacataccgttagtatacagcccagcagcaactacaatcctgggcattaatcctagagaaatgaaaccttaatgttcacataaaaacctatactcaagtatgcatagcagctttacccataatatctaagaactggaatcagctcagatgtccttcaacaggtgaatggttaaactactcagtaataaaaaggaatgagctactgatagcatgcaacagtttaggtgaagttatgctaatgaaaaaagccaatcccaaaaggttatacatactgtatgattctatgtttttttgcaatggcacagttttagggatggagaatagattagtggttgcctggggttagagatggggtagtagagtaggttagtggtggcagaggagagaaaagagagggaggtgaatgtggttataaaaggacaacacaggggaatacttgtaatggaaatgctttgtctttttttttttttttttttttttggcgacagagtcttgctctgttgcccaggctggagtgcagtggcatgatcttttctcactgcaacctctgcctcctgggttcaagtgatacttgtgtctcagtctcccatgttcagagtgaaacaaaccagaggtaatgttcatccaaataatccaacacacatgacattaaaacatcaagatcaggtcggacgtggtggctcatgcctgtaatcccagcacttttgggaggccaaggtgggcagatcacttgaggtcaggagttcgagaccagccgggccaacatgatgaaaccccatcttgactaaaaatacaaaaattagccgggcatggtggtgtgcacctgtagtcccagctacttgggaggctgaggcaagagaactgcttgaacccgaggggcagaggttgcagtgagctgagagtgcgccattgcacttcagcctgtgtgacagagtaagactccatctccaaaaaaaaaaaaccaagatcaattaaaatacagcattactgggccgggtgtggtggctcacacctgtaatcccagcactttgggaggccgagatgggcagatcacgaggtcaggagatccagaccatcccggctaacacggtgaaaccccgtctctactaaaaaatacaaaaaattagccgggtatagtggtgggtgcctgtagtcccagctacttgggaggctgaagcaggagaatggtgtgaacccgggaggcagagctggcagtgagctgagatcgcgccactgcactccagcctgggcgacagagcaagactccgtctcgggggaaaaaaaaaaataaataaatagaatgctgtagtgtccttgagtttacatgcccctccttacgcttgtgtgcccgtgcagattgcttgattacacaattagaggaggctggcggaggattgttttaatttttttttttttgagacagtctggctctgttccccaggctagagtgcaatggcgcaatcttggtgcactgcaacctctgcctcctgggttcaagcagttcttctgccgcagcctcccgagtagctgggattataggcgcccgccaccacgcccaactattttttgtatttttagtagagcagcgtttcaccatgctggccaggctggtctcgaactcctgacctcagatgatctgctgccccagcctcccaaagtgctgggattacaggcgtgagccacacctggccgtttgttttaattttgaaggtgaagtgaaagtgactacatttaccaaaagtgattgaaaagccaggactgttcttaccctgtttttccagttcttgctcagagcaaggtggtttctttttcacttaatcaccatacttacttttcatgtagaacaagtcagtttgagttatcagttcatcatcttaactaaattccatgggggaaggaattagttttagtttcttaaacttccaggtttgcttattggacaaaatgagatagcaaggcagtgtttttaagttagattttttatttctttggtaatacaattttctcagaaacttagtagtcttttagtttagttgtttttagttggtcctatgttttggatcacccctctctactttattttgatagtgccaactgtgaagacatctgaagccataggtttggatgggaaggaggcatctttagcctgatcatcttcgccaggctgtttatctccttttgcttggctgagaagtcttaataggaggcttattcccagctatttggggacatagaagcagttagccattgcttatattttactgaggtctgtgtggtatgttgattgtagtcagttaacgattttgagaactgaaggcagcctggtatatatagagtaggtattagactgtgtttcttctaattgaatttcccatctcttgtaatctatgccatcatcttctgtactgctgagaaagaaagaaagtttctaatcaaactataccactggttgtaagatgcagtttggctttagtgatgttaacacatgattcaaacgtgaaattgattgagtattggtgaaatacagaggagatttaaagccagaagacctgggtttaaatgctggctgtatgacttcatatctgtgtgatcttgggcatgtcatggttggcacttcaatttcttctctctataatgggggaagtgaggccagtcatggtggctcatacctataatcccagtgctttgggaggccaagatgggaagatcgcttgaggccaggagtttgagcaattgggcaacatcgtgaggccccgtctctacaaaatattttgaaaaaattagccaggcccagtggtgcgtgcctgtggtccgcgccactcaggaggctgagacgggaggatcctttcagcctaggagtttaaggctaaagtgagccatgattgtgctatcgtactccagcctgggcagcagagcaagatcctgactctaaaaaaaagtaaaataaagtaaaatgggggaaatgaactgctttagtaacatcatctgttttttctgtgagcagcgtagcttgacagccattggtgaactcgtgccctgtgcttccctgtccagatccccattctgcccgcaacatggagtataacggtttattcatagtagtcgagaaacactcactgaatgaatgaatgaggtgtagaactaagtggagtgggtaattcaacacatattaatttccttcttttttttatttttagaaagaaagaactttcagctaccaagaaagaccgtgtgaatcattgtctgacaatatgtgaaaacatagtggcacagtctgtcaggtaattgcactttgaactgtctagagaaaataagaactttgtatattttcagtcttaatgggctagaatattctttgtgtcccagctattttaaatggattcagaaatccatttaagatgaagaaggacccttttcccatatttctggctatatacaaggatatccagacactgaaatgaataatgttccctttttgtaatcttttatgcaaaaattaaaaccattatggtaattgaacaacatgtttatgtttagttaacacccttagcaactatagttattttaaaaccatctatggtttgatatttttgcatttgttgcaatagtaggaacagcacaagacagttcagtttgtctctcttatttgctttttcttggcagtttgctgtcctattgtacctctgctcctagcagtggctggagcccactcctctgtgcttcgggattagtggggatcgtggggcattgactgtaggtcagctttccttgcttgatctttctcactgggatgaactagcagcaccttcttttgtagctgctttgcttttgactatctttctgaccgttgttcctagtagctgtagatggtaaatatatttaggcctgtttccaatggctcagtaggagacatattcacctatgatatctgaattctgttacccacatgggcatgcgtgaaatagttgccttgccttactttcccttggaataaataattcatgttattctcctggtagaagctagaaaaagcctttatagtcagtcagaaaaaaatttttagacaaataatcttgattttagtactgacaaaaacgtgtggtgattctttttttaatttttttttgagacggagtttcactcttgttgcccaggctggagtgcaatggcgtgatctcggctcactgcaacctctgcctcctgggttcaagtgattctcctgcctcagcctcccaagtagctggagttacaggcatgtgctactgtgcccagctaattttgtatttttagtagagatgttggtcaggctgatctcgaactcccaaccttaggtgatctgcccgcctcagcctcccaaagtgctgggattacaggcgtgagccagggcgcccggtgattcatttgttttttcaaaaaatttcctcttggccattgcttttcacttttgttttttttttttttttgagacggagtcacgatctgtcacccaggctggagtgcagtggcatgatcttggcttactgcaagctctgcctcccaggttcacgccattctcctgcttcagcctggcgagtagctgggactacaggtgctcgccaccacacccggctaattttttgtatttttagtagagatggggtttcaccgtggtcttgatctcctgacctcatgacccgctcaactcagcctcccaaagtgctgggattacaggcgtgagccaccgcgcccggccctctcttgtctttttattgtggtaaaatgcacataaaattgactgtcttaaccatttttaggggtacagttcagtatatatattcgtaatgttgtacagccatcactgccatctacttcataagtttttcttctgtcaaaactgaacatctgtcttcattaaactccctatcatccattctttcctgtagtccctttctactttctgtctgtatgagtgtaactgctctggagacctcatgtaagtggattcctacaggatttgtgttttttttttggtgatctgcttatttttaatgcctctgtgcatttgtattatatactttcaaagtgatttcacaaaaccgtttcattttaggttaactcatttctgttgtttgtgaaatactgtgtatgattctgttctgtttctgtctaatttgtggaaatgttgtgggaagaaaatgaaataacaaatgagcatatgtcctgaaaataaaaatataaaaattctaagttagcatgctattgtagaatacaacgctatgataaaagtaggaaaaaaaaaggtttgaattctatctctgctacctgtgtaagctgggtgactttagataagctgtaacgtgtttgagccttactggctcatttttgaaatgtaatccctagttacacagttcttgtgggatcagatggtacatgtgaaacactgtgaaaaagcaactgcatagatatgttcattagccacctgagcgggaagcgtatcccattgcgatgcccatcatccaaagctatatgttatctttacttttttttttttgagacagagtcttgctctgttgcccaggctagagtgcagtggtgcaatctcagctcactgcaagctccacctcccgggttcacgctattctcctgccccagcctcccaagtagctgggactacaggcacccgccaccatgcctggctaaatttttgtatttttagtagagatggggtttcaccgtgttagccaggatggtcttgatctcctgacctcgtgatccgcccgcctcggcctcccaaagtgctgggattacaggcgtgagccactgcccctggccatctttactttttttgtgaaatgactttaaatacttggcaaacatttggtcattgttcatctgatctccaccatccaggtctcagagaacataatttctctctgaaagcttattgacccaggaaataagatctctttcaatctgagtgcgtcaggctttattcttgtcattttgtcttttgataattttcaaatggaattcatggaatgttggcttatattcatatattagtaaagtatgttgagacatcttaagattgatttgtggttctatatgccatattaaatcaaaataatagctgttaatggttttcacattagtctgtctcttgtttttatggagtaatgctgagagttcattatgcttgttctacagaagagcatgttaaaaggagtttttggagtcagagaggttattcttggtttcataggatacactctatactttttagggatttcagagtatatagctgaaggtgatattttatgtaaatatgttttatggaaacttattgctcatcgctgtttcctgttaactctcctaaaatataattaaacttttggaacttttttatagcttttgtgctagactaatttttgtctctaatgaggttatataaatggcagcttctgacgttttcaatgtaggaagtcatttaaaacttcatgtatattgtgaaaatgtagtctgctttaagctctctaaagtggtctaagttactggttcctaagtatggatgagcatcaaaatcatctggaaaatttgttaaaaatacagtaatgaaggcacctcactgtcctttttcccaaacatacttctgcattctgtttgagtaggtagggactacacatttttcacaagtatcctcttgggaatacccaggaatgcttacttgagcaacctcttactaatatgtaccttgataaggtggctaggtaaacataaatatacaaaaatccatagatctcccatatattagcataaatcagctagaaaatataacgtttaaagatctagttcacagtagcaccaatatatcgaactctaaggaatcgataaatatgcaaaaactttataaaaacttctgttaatgtttctgaaagatataggtgaccactttctagataggaagattttatattactaagttgaattttctctaaattaacacagaaatttaaaataatcttgatcaaaattctagtagaggtatttttgaacttgttcactgcaagaataaatacataattgcaaagaatatctcaaaatcatcaccaggcctggtgtggtggcccatgcctgtaatcccagcactttgggaggctgaggcaggcagatcacctgaggtcaagagtttgagaccagctggaccagtgcggtgaaacactgcctctactaaaaatacaaaaattagctgggtgtggtggtgcatgcctgtagtcccagctacttgggaggctgaggcaggagaattgcttgaacccaggaggtacaggttgcggtgagcctagatcgcaccactgcattccagcctgggcgacaagagcaaaattctgtctcaagaaaaaagagaaaaaagaaaaagaaatcaacactaatatggtgagacttaatgtatgtgacattaaaatagtgattggatgttaaaacaggtatagaacagaaagaagagtgtatgtgtgtatctgtatgaatttatgatgggtgtaacatatatgtattagggaaatgagggaaatgatacatttctctgactttgggagaacattatatctctacctcatattgcaaacaaacataaagttcagattaattacctaaatgtgaaaaaatgaaataatttctttaaaaaatgtaatcttagtttgaggaaggttaacattataaaggaaaaaactgttttgagtggaatatagttcaatatgtcaaaatccaccttcaacaaaattgaaagtaaattgaacttggggaaagtattgacagcatatagatcaaaggttactagcctgtgtaaagagcagttataaatatcgttaagaaaaacactgtcgacctgtcggcaccttgttctccgactcccagcctccagaactgtgacgagtaagtgcttattgtttaaaccacccagtctgtatgtggtattttgttatagaaactcaagctgattaggacactagtaatcagtagactgaaactgaaacaaaaataagaaccttttttacctgtcaaattggcaaacattaagaatattcagatttttgtcagaggtgatacaaccttctaagaaggcaatttgggaaaatataaagctttagattattatatgtctgacctagcagttttacctctagggtgcttacccctaggaaagtgtgtaatgatattggtgcagtgcccttcatcccattagaaaattaaaaataaccttaatggcctaccactaaaaggggattgaaaatttaagatatatttatttatgtgtttattgagatggagtcttgcactgtccgcctgggccagagtgcaatggtgcgatctcggctcactgcaacctctgcttcccgggttcatgtgattctcctgcctcagcctcctgagtagctgggattacaggctcacaccaccgcacccggctaattttttgtatttttagtagagatggggtttcactgtgttggccagactggtctcgaactcctgacctcatgatccgcgcccctcggcctcccagtgttgggattacaggtgtgagccactgcgcctggccagatacatttatacaagagaatgttagttaacattcatagatatttatattttgtttactttttattaaaaaaattttttttagagacaggatcttactctgtcacccaggcaggatgcagttgcacaatcatagcccactgcagcctgaactcctgggcttaagtgatccttctgcctcagccttttgagtacctgggggactttaggcagtgctactatacctggctaatttttaaatgttttatagatgagatcttgctgtattgcccaggctggtctagaattcctgggcccaagtgatcctcccaccttggcctcccaaagcgctgagattacaggcatgagccaccacttctgaccaatagatatttatatttgtgactggaaaatatattaacaatgtgttaaaaaattcagttaaaaaataatgaaagatttttgcttctggctaagatagaataacaaggacagcatttatcttcttgccttgaaatagttgaaaacggaagaaatatatgtaacagtggttttcaagttattgggcatcaggcaaagaagaatagttatcccaggaaaatgaatgtggagagccctacaatttccttacattactgcctggtcatggcaagaggaaaaactgagaggagactgaggctgagccagtggtttgctgggttgaggaggcagagctgggagtgcagagatgcaaggtggtgagagcccatatggaagaataccagggaagagagctgcagagggagctccggagacctgcaccctgccctctcagtaccctgtcatgtgtgtagctgagtactgacgagcacttgcttgtgcggaaatgacccagggctggaggtagagccacctgaaaggattagaaggaacagttgctgaaagtcacacagggccaggaagaatttctaatcacaccagttggagtggaaaacctcagctctcatagagcaggtagggtactcagaagggtttgcccacctagccccagactaagtttcgttactctgaccctacctaatattaaaaagagattaattaaattgttcgcaacaaaaataatatatttcagtgtttgtaacacgtagaagtgaattgtatgacaatagcataaaggctggaagagcagaaattgacatgtatttgcgctgggcagaataatgctcccctctttccccaaaagatatcaagtcctaatccctggagcctgtaaatattactttatatggaaaattgttttatgatgtgattaaattcaggatcttgagatgagggggctatcttggatgatctgggtaggcactaaatgcaatcacatatatataaaaaggaggcagagggagattttacacacagagagaaggccctgtgaagatggaacagaaagatttgaaggtgctggccttgaaaattggagtgatgaagctataagccaaggaatgcagcagccaccaaagctggaagaggcacggagcagttctcatttagagcctactccagagggaatgtggtgctgccaattccttttttttttttttttttaagatatcatttacccctttaagttggttttttttttttttttttttttttagtatttattgatcattcttgggtgtttcttggagagggggatttggcagggtcataggacaatagtggagggaaggtcagcagataaacatgtaaacaaaggtctctggttttcctaggcagagggccctgccacgttctgcagtgtttgtgtccctgggtacttgagattagggagtggtgatgactcttaacgagtatgctgccttcaagcatctgtttaacaaagcacatcttgcaccgcccttaatccatttaacccttagtggacacagcacatgtttcagagagcacggggttgggggtaaggttatagattaacagcatcccaaggcagaagaatttttcttagtacagaacaaaatggagtgtcctatgtctacttctttctacgcagacacagtaacaatctgatctctctttcttttcccacatttcctccttttctattcgacaaaactgccaccgtcatcatggactgttctcaatgagctattgggtacacctcccagatggggtggcggccgggcagaggggctcctcacttcccagatggggcggccgggcagaggcgccccccaacctcccagacggggcggcggctgggcgggggctgccccccacctcccggacggggcgggtggccgggcgggggctgcccaccacctcccggacggggcggctggccgggcgggggctgccccccacctcccggacggggcgggtggccgggcgggggctgccccccacctcccggacggggcggctggccgggcgggggctgccccccacctcccggacggagcggctgccgggcggaggggctcctcacttcccggacggggcggctgctgggcggaggggctcctcacttctcagacggggcggctggtcagagacgctcctcacctcccagacggggtggcagtggggcagagacattcttaagttcccagacggagtcacggccgggcagaggtgctcttcacatctcagacggggcggcggggcagaggtgctccccacttcccagacgatgggcggccgggcagagatgctcctcacttcctagatgggatgacagccgggaagaggcgctcctcacttcccagactgggcagccaggcagaggggctcctcacatcccagacgatgggcggccaggcagaaacgctcctcacttcctagacggggtggcggctgggcagaggccgcaatcttggcactttgggaggccaaggcaggcggctgggaggtgaaggttgtagtgacccgagatcacgccactgcactccagcctgggcaacactgagcactgagtgagcgagactccgtctgcaatcccggcacctcgggaggccgaggctggcagatcacttgcagtcaggagctggagaccagcccggccaacacggcgaaaccccgtctccaccaaaaaacacgaaaaccagtcagacatggcggtgcgtgcctgcaatcccaggcacttggcaggctgaggcaggagaatcaggtagggaggttgcagtgagtagagatggtggcagtacagtccagccttggctcggcatcagagggagactgtgcgagggcgagggcgagggcgagggaattccttaatttcagtttagtgatactaattttggactctggcctctaaaactgtgaaagaaaaaattttttgtttgtttgtttcttttaagccacatagtttgtggtaatttgttacagcagctgcaggaaactaatttatgctgcatgtgaaatggtgtaataaggtagattgtgatgaagatacatagtataaacaattaagcaacaactaaaagcacaacaaggaattatagctaatgaaccaaaaaaggagattagaataataaaaatggtgaatcccaaagaagccagaaataggggaagaggcaaataaaggaaagaaagagcttgatggtagatttcaacctaactatgtcaaaaaggacattacatgtaaaaggcagcgatttttcagattgaatggaaaagtaagactcggtatatgctgctgcctgcaagaaacacattctaaatataaaggcaaaaataacctacaggtaacagaacggaaagaagttcactgtgcttacaagaattagatgcaagctagactggttctgttaatatcagacaaagtggatttcaaagcaaaggctcttgcccaggatgagatggtcatttcataatgatgaaggggattcgttcatcagcctggcatagcaagctgaaatgtttatgcaccggactacagagctaaaatacatgaagcaaagcctgacagaactacaagtagaaacagacaaatccacagtgatagagatttcagtagccgctctcaatgatttgtagaacacgtagccataatatctggatctagaacacttgaccaacactgtcccctgtgcaacctcattggcatttacaggacactccacccagcaccagcagaagagacactctctcaagtgctcacagaatgtttgccaagatagagcagatgctgggccataaaacaagtctctaaattaaaagcattcaaattattcagagtatgttttctgacctcagtatcattaagttggaatatattataggaagataacctggaaaagcctcagatatgtggaaaaacccatttccacatggcccatgggtcagaagtgaagtcaaaagggaaatttgaaagtcttttggattgactgatataaaaacaatagatttctaaacttgtggggtgctgttacagcatagtaaatggaaatttctagcattaaatgcctgttttaggaaagaaagatttcaaatcaatgacctcagcttctacctttggaaacttgaaaatgacaagcaaatggaatccagagttaccagaagggccaggtacggtggcttatgcctgcagttctgccactttgggaggccgaggcaggtggattgtttgagactggcagttgaagaccagcctgggcagcctagggagaccccatatctacaaaaaacaaaaaaattagccaggtgtggtggcatgtgcctgtagtcccagctaaccaggagtctaaggtgggaggattgcttgagtctgggaggttgaggctgcagtgaactgtgattgtgccactgtgttccatcctgggcaacagaatgagaccctgtctcaaaaacaaaaacagttactagaagaatggacatcataaagataggagcagaagtcagtaaaatagaaaacaaaaatacataggaaatcaataaaaccaaaagctggttcatcaagaacatcaataaattggtaaagctgataggaaaaacagtgaagtcacaaattagcaatatcaggaatgagggagatgacagtagtatagattatatagatattaaaaggactgtatgaggcaggtgtggtggttcacgcctgtaatcccagcaccttgggaggccgaggtggacagatcacctgaggtcaggagtttgggaccagcctggccaacatggtgaaactctgtctctactaaaaatacaaaaattagttggtcgtggtgctgtgtgcctgtaatcccagctacttgggaggctgaggcaggagaattgcttgaacctgggaggcggaggttgcagtgagctgagattgtgccgttgcactccagcctgggtgacagagcaagactccatctcaaaacaaataaataaataaaaaggactatatggtaatattatgaacaactttatgccaataaatttgacaacttatagatgaaatggatgagttccttgaaagacacagaaactattaaagctctctcaagaagatatagataagctgattagccctatatctattttattgaatttaaatgtaaaaatcaatatttagttactggaaaacttttaagtgtggttggaaatggtatacgaactttttcaactgaattttatgaagtctaatcacaggtaaaggttttctgatgaaaatttagtgtctgaattgagatatactgtaaaaaatgttatatatcttaattatttcttcacattaattacatgttgaaataatactttgggtgtattgggttaaattaaatattatgaaaatcttgcctgttttctttttacttttgatgcgtcagctaggaaatataaaagtgtagctcacattctgtttctgttgacagtactgctttggagcacagtgtttgaatgatctatcatttcaaagacctttcctcagttcgttattcatggctgtctgtattccacatagataaggtctgaaatactgctaagtggcatgttttgttttatgcttttataagtttgttgatcattactgatgtggacttttggtgcctcttaggctcattgctatcttccaaccattgtttgcaatttttacctagagataaagagaaagagacatttggtttcagagtagttagattgggatcatgaaagagcaacctcattttgatgcttcaaaaatagcacatcccccgtattactgggatttgctattcttgggattacttcaagaacatccttgtgttactggtttggatgcttctgaatgctgtgaagtcagtttcatgtacatggctcatcagtttagctctctcttggctttgtttagacagttggagcatgatggcctaaacagcttctttcaattaaacattttaaaatagtttacaaatagtaaacaaactccagtttttgtgactctttgtctcgcacaacaaaaacacaatctgaccatgatcatctggcatcttagggtgaaatatggttatactttggcccataccgaaagcaagattaaaaaggggcaggagagatagactgctgaactgattttcaaggttccaagaatattgtaggttaagagtaaaagtaaacttttggtagaaagcagtgggttgtctaggattgaagtatctgaagtttttaaacgaaaatttaaaaagaaaaatgagaattgccttacaagtacaatctcttcttttttaaaaaataaactttattttgaaatagttttagatttatagaaaaaaattagatagggtaggaagttttcatataccctacatccagttaccccagttattatcatcctaatttagtgtgagacattttcatgtttaatgaatcaatattgatatgctattaacttaagtccagactttattcagattttcttaatttctatgtaatgtcctttttctgttccagaattccatgcaggacaccggatacctcattacatttcattgtcatgtcaccttaggctcctcttgacagtttctcttctttttttgcttagaaattctccagaatttcagaaacttctgggcatcgctatggaactttttctgctgtgcagtgatgacgcagagtcagatgtcaggatggtggctgacgaatgcctcaacaaagttatcaaagtaagaaccgtgtggatgatgttctcctcagagctatcattgttgtaggctgagagaagaagcgatcattgagtgttcttctgttttgagtccctgaggatgtctgcacttttttcctttctgatgtatggtttggaggtgctctgttgtatggtttggaggtgctctgttgtatggtttggaggtgctctattgtatggtttggaggtgctctgttgtatggtttggaggtgctcttgtatggtttggaggtgctcttgtatggtttggaggtgctctgttgtatggtttggaggtggtcttgtatggtttgcaggtgctctattgcatggtttgcaggtgctctattgtatggtttggaagtgctcttgtatggtttggaggtgctcttgtatggtttggagatgctctattgtatggtttgcaggtgctctattgtatggtttggaagtgctcttgtatggtttggaggtgctcttgtatggtttggaggtgctctgttgtatggtttggaggtgctctgttgtatggtttggaggtgctcttgtatggtttggaggtgctctattgtatggtttggagatgctctggtatctgcctgcattgcttgccacacctgcccggtcagaaggcgctatgttgacaattgtgcctgcacggtgcctaggtcaatgaagggaaccgatggtagccactggatgctcctgggaaaatgtcactacaggcaccagagaagccagagctatgcccaaatttctatgagtctcagttttcttaaccataaaatgggatcaatgtttttgtggcatgtgtatgagtgtgtgtctgtgtatgtgtgaggattaaattgtgtatgtgtgaggactaattgccactactggatcctcaaagtggtaagaagtgttcttattaataatgacatccttacactcttacccagcaagattgatgggtgtggcactgcttctctttttccatcacatggtttccatggtatccttttgcccagggaatctttgctttgtggctagcactttgttgtttggctaatcacgctttctgtggtcaggacgctggcttctctggagccatgggattctagctccctgtcttgtccctagagtggtcactgtcttctctctccgcttgcaattcctgctttgctcgcatctcacttatgcagtgacgtatatcagtttcaccttgttctccgtgcctgctgatcattggcaccacttgcatggtgccatttagggcctgcttccagttaagcttgcttctccacaggcctaaatatccttgcttgcttcttttattctcactggcaggaccagggcggtctgtctttgcatgagacagggtctcgctcagtcacccaggctggagtgcagtggctgatcacggctcattgcagccttgagctaccgggctcaagctatcctcctggcttggccccttgagtagctgggactacaggcgtgcaccaccatgcccagctaatttttaaaattatttgtagagatgggatctcgccaggttgcccaggctggtcttgaacgcctgggctcaagtgatcctccctccttggtttcccaaagtgctgggatcacaggtgtgagccactgtgcctggcccttgatgtttcagttcttgatatttgatcctcagagtcagaaaatctaaaaagagggctatcccaggttgccttggttcatggcaaatgggacgttaagagggcagagagaatatgaacagaaactgttctaatattggtcatttaatgtgtaagtattgttcttttttaaacctccttcattttttttccaggaattgctggacacagtggcttggtgtgtgtctgaggactgtaggccatggccctaggttgtggttttaggtctcaggtgctcttcctggctgtctccttgcttctttcccatgtcctcttctttgtttccagccatttctcccttatgcttaagtttggtgcagcagggtttggctgctctcagattcctgcttcctcagatgctgtagttgtcaggcccagcgggctggcagcgggatcaggatctggctaggtttgctctcactgtggcagagtagggggaggcgtgggagagcacgtgtgaccccaggccagctgtagggagcataggcatggtcacgtagccttcaggtcctagactttgtcttctcatgagtatggctgtgtgtgtatggtgaaaactaggttctacttagcccaagaaaatgggcacattttgcatgtggtttctgtagagaaatgcactgggtatctgacatagcctggcagcatgcctccctcaggtaggttagtctcaggcggtgaagcacgtgtgtccagcaagaacttcatatgtggcataaagtctccgttctgtgaggtgctggcaaatcaccaccaccgtcaagaggctgaagtgatttttgtctagggaggcaggaaaggcttcctggagtcagcagccagtaggtgaaagagtagattggagaccttcttaatcatcaccgcctcttgtctcaaggggtgccaggaagctgtggaggctgaacccatcttatgctgccagagagtgggacaccatgagggtcaggtcaaggggttgtaccttgtttggtagagaattaggggctcttgaagactttggatgtggtcaggggagtgtatcatttaggaagagtgacccggtgaggacgtggggtagaggaggacaggtgggagggagtccaggtgggagtgagtagacccagcaggagtgcagggcctcgagccaggatggtggcagggctgtgaggagaggcagccacctgtgtgtctgcggaagcaggggcaagagggaagaggccagcagcgtgctgccatcacccagcgactggcgtagattgtgagagaccattccctgctcttaggaggggctgagttttagttttctcttgttatacaataagcttggtatttgtttacaaaacatttgtaaagctaaatcaaggtttgataaggcttctagttttatttaagaagtaatgttgaaataaatgtttgtccaattcgctttgctcatttaaggactttcagtacaaactgcaacaacaggattaggatttaaacgtttctgagatgtttttactcctcagaatttcccagaatgtgatctggttttgattttcaagcttgctgacccaataggttaacccacaagttttacgaagaccatctcagtccacttacatcaactgcccatgccacggttaaagagatcatcgactgatgtttggcacagcttcctccctcttgggtgggcaagcatttggaagagaaggctcctatgggtgagagtggggcaccaaagtcttccctgtcccatcccctagcttgagaagcccttctctaatgtggactttgtgccgttagcatcgttactagcttgaagttgaccatctggacgtactttctggtttagcctcacaagtgagcaaggagggttgagagatgtgctgtgaggaatgtggggccccagctggcagcaggctctgggtcaggggggcagggaccacgggcatacctgacagtgaggaggggccacacctgcagaaaaggatgcaggactccgccttgggaagtgttctaggccagagcgagggtctgtggtttataagtacacccacagtgctcgggaccctgcagatgtccagggtgccgtctgagcccgtatcatccaacagaatgttctgctagtgaagattaaagatttactccaggggctttaggatttattatatatatataaatcctatatatataattttttttttttttttttttgagatggagtttcgctcttgttgcccaggctggagtgcaatggcgtgatcttggctcactgcaacctccgcctcccgggttcaaactattctcctgcctcagcctctcgagtagctgggattacaggcgcccaccaccacacccggctaatttttgtattttttagtagagacggagtttctccatgttggtcaggctggtcttgaactcctgacctcaggtgatctgcccgccttggcctcccaaagtgctgggattacaggcatgagccaccccacctggccaggatttattgtatttgaaccatctaccattttaattttgatgttatgtagtatttgatgataatgaaagttaaattgtttttctttccatttttctgtttaagtgaatgacctgtatctagtttattcagtaacttcctgcatatatttgtttctttcattcttaatgaatatattcttaatttagttgctattatgttttgctttgccccaaaattgaaatcttagtttccttttagctcgttttagaactagtgatgggatgtgtcttccataaatctcttgtgatttgttgtaggctttgatggattctaatcttccaaggttacagctcgagctctataaggaaattaaaaaggtgggccttgcttttcttttttaaaaatgttttaaattttaaatttttataggtacacgtattttgtaggtacatgtaaatgtatatatttatggggtacatgagatattttgatacaggtatacaatacataataatcacaccatggaaagttggatatccatgccctcaagcatttatcctttgtgttacaaacaatccagttacatgctttacttattttattttatttttgagacagagtcttgctttcacccatgctagagtacagtggcatgaccttggctcactgcaacctccgcctcccgggttcaaccgaactttgggctggtctcaaactcctgacctcaggtgatccgcccgcctcggcctcccaaagtgttgggattacaggcgtgagccactgtgccgggcctgattgtacattttaaaataactaaaacagtcagggcacagtggctcatgcctgtaatcccagcattttgggaggctgaggcaggtgatcacctgagatcaggagttcgagaccagcctggccaacatggagaaaccctgtctctactaaaaatacaaaaattagccaagtgtggtggcgggcgcctgtaatcctggctactcgggaggctgaggtaggggaatcgcttgaacctgggggtggaggttgcagtgagccgagatcacgccactgcattccagcctgagcgacagagtgagactttgtctcaaaaaataaaaatgaaataaaattgggccgggtgtggtggctcacaccttagtcccagcactttgggaacctgaggcaggtggatgcttgagaccaggagtttgagaccagcatgggcaacatggcaaaacgctgtctgtacagaaattagctgggtgtggtggtgcacaactatagtctcagctacttgggagattgaggtgggaggattaattgagcctggaaggttgaatctataggtagctgagattgtgccactgcccttcagcctgggcgaccaagtgagaccctgtctcaaaagaaaaacaaaaaaacaaaaaacaaaccactattatcgactatatattattgtctatgatccctctgctgtgctgtcgaataccaggtcttgggcccttatttccatcactgagcaaacttcactctgttaagcagcaggtgtgggatttcatcgttattcagtaattcacaatgttagaaggaaatgctgtttggtagacgattgctttacttttcttcaaaaggttactctttattagatgagatgagaattaaaaatggtaacttactttatatctttataattgaagcccactagaccttaaagtagttaccagatgttttatgcatttaaatggccttttctctaaaattagaaagtaacaaggaaagaaaatgcttcgtttctatgcaaccctcttggtgactagtatgtgactcttaatgcaaccctcattgcaccccctcagaatggtgcccctcggagtttgcgtgctgccctgtggaggtttgctgagctggctcacctggttcggcctcagaaatgcaggtaagttgtacactctggatgttggtttttgtcgggggccagctgctactgatcctttatgtctcagctcagatgtcatttcaaaagtctgctctgccctctccaaattgcagtcgaccttgccctgtttatgtttccctcatagcactaatccatgtcagaaattgtcacgtacagtctatctgtgtgcttgtttattttctatcccacccttccgcaagagacttatgggatgtgtgccccaggacagcaggggtcttactgtcttatgctctgttgcagcccagcagcgataacagtgtctgcacatagtacttgcttaaaagatacttgccaaattgttgaaggttgaggtaccaatttcattattgctgactataggagttatagcaaaatatccatttgtctgttacatgagttaaaaatatggttgttgcactgtgaatagtttggtttagtcaaaacagttgtatcttaacggattgagaaacaaaagcaggaccacttttcatcagctccctccttctccttaaccagcaatacatgctgatgctgatatcccatagaccctcagctccatcctgagtcactgggaatgtggtctaaaccctcactattaatatgaactgagtttcaataagaatcttatatgggtcgggcatagtggctcatacctttgatcccagcacttcaggaggccaaggcaggtggattgcttgacccagactaggcaacatggtgaaacgccgcctctacaaaaaatacaaaacttagccaggcatggtggtgcgtgcctgtggtcacagccactcgagaggctgaggtgggaggatcacttgagcctgggaggtggaggtcgtgttgagccaagatcgcaccactgcactccagcctgggcaacagagtgagacctgtctcaaaaaaaccaaaatccagaaaagaacttatatggctgcagaggtataatcactaaggaaatttccttttgtataatcttttttcttttactatcatttaaaaaaatgtgttatatttctgaagcaacacatccaggttctgcacatagcagccaaagtgaccttaaagaatataactgggtcttgtcattcccttatttaaactcttgtacccatttcccagtgccgtttagatagagattccagactcgtcaatggctctgtcacctcagacaccctgcattgactcattagtctgattagagtcaggtttttcttcctcctgatggtttttttttcccccttagttctcagcggaacagtcacttccttagggaggtttccccagccaccctctgaggccgtgcttgttgccagactctgccactagagggcagggctgcaccactcctggcacctcgcacccggcctgccctgtcactctgtgtgttgggtgaattcctgtgatctgtgactcactgctctgtgtcctacacattcggcttttcttctctccccacaaccccattttataattctcctttttcaggaaagctttattcccatttaaaaatttttgtttttaaaatggtattttcttacacttattttctaattaaaaatgagtgttttaagaagtattatgatttactgcaaataatttttaaacccagccttttagatcctctgtgatcataagagaaatgaaggatgtctcccaacacttgagcttcatccacatttcatcctcctgttctttcagctgagttttccccatcccattagggactgttggaatataaaactggcttttccctaacagggaatgaattgcttctgtttctcctgaaggagagctggaagaatgacttgcgttcttttgcatacacaggccttacctggtgaaccttctgccgtgcctgactcgaacaagcaagagacccgaagaatcagtccaggagaccttggctgcagctgttcccaaaattatggcttcttttggcaattttgcaaatgacaatgaaattaaggtatgattgttgcctcaggtcacaaacatgcgagtgatgctgtgagtgagtctgtggagggtgagggcttctgaacagggagtcctgtgggagtgcttcttggggtatgttgtatgtcgtaatttagactaccatcatttgtgttatttttgaggcacctaaggacttctttccacttctcatttcttactgtggggtgaagagttgaattgggagatggtttctagatgcaaattgaaaaggcatttttccagagcagatttgttttcggcgtactagagtgactctttaacctagctgcgggaagatgactgtgccaagactgcaggtaggagaaagctcactgacgaggccttgtgggtctgaacgtcctgcagctatcagagcctgttggcttcctgttgtgcattccaacaaatcatcttcaaacccactttagtgttttgtttataatgtccagaaatagtgaccctgtcacatgctctacagattacaggattcttagcctcttcctttttggtaggtcagtcctgggtttgagcccaagtgaccctcctgggaggtgatgatacacactgggtagagtggaatcagatggacttggattagaattctgtcctctttactagttattttcctctaggcaaactgcccaacagctctaagctatttccttcgtattctgaaaaataagccttaatgggacccatatagggcaactctgagagtaaaataaaggaatatgtgttagagtgtagcatagtcacccacgggaagggcttagatgttagctgctactgctcttattagctgaatgatttggaataaactgttagcctctctcatgttttttctcttgagcttcgaagttttcttgttaatactaaggagatattcaaactagtcatggggttttggaatgacgaagggagatgatgaatctaaagaatttagtgtaatatttcttcatgctcagtaaatggtagtttctgctgctgttatttttattaccatctctttggaatgggagtaggtgctcctttgtggtcagaggctgtgagagctccacagcgccagtttgcccatctgtacactggggtctgttgaaggcagtcccctctgtgatatctctggctgtcagagctcagatgatagatggtatttttgtactcttagttctcatcattttcatgatttcgatcaccatttgagtatgatgatgctaacactttgttgaacgtagaatccgttaattacttccttcctgaacctttggcattaaaaaaaatctattctgctacctctctgctcatttatggttattcaaatttattatcaagagcctggtacagtggcttgtgcctataattgtagctacttgggaggctgaggtaggaggattgcttgaggccaggagtttgagaccagcctgggcaagatagtgagaccctatctctaaaaaaactgaaaaaaaattagctggacatgatggcatgtgcctgtggtcctagctactcaggaggctgagacaggaggctcggttgagcccaggagttggagttcgaggctacactgagctgtgattgtgccaccacactccagcatgggtggtaaaacaagatgccatttcttaaaaaaaaaaaatatatatatatatattatcaatgaaattcagtagtaccaacaggattataaacaaagatagtagttcccttcctactttttctcttaatccttgtgtctcacaggcaaacataactcttagtatttcttccaatatttactttcatgtttctttctttctttctttttttttctttgagatggagttttgctcttgttgccaaggctggagtgcaatgacgcaatcttggctcaccacaacctctgtctcccgggttcaagcgattctcctgcctcagcctcctagtagctgggattacaggcatgcatcaccacgctcggctaattttgtacttttagtagagatggggtttctccgggttggtcaggctggtctcgaactcctgacctcaggtgatcctcccacctcagcctcccaaagtgctgggattacaggcgtgagccactgcgcccagcaacttccacatttctaaataacatgcttctactgctattttttttttcaattttagacatttttttactttcactatagttctatcagaattcagtgtgtacgttattatgcctaagtaaatagtcatggttgcttacgtattatatttctttgattgtgtttcttatttgatgagaaagctgtgttttttgctctgggttgaaactggagagaggacctggggaggaggaggaggacagatgaagttggtgactgtaccttcatggccatagctgggttctcagcacccggggatctgctgatcacctactcataggccaggcccctatcgaagttctaggtgacccagtgctggggacgggggggccacctgcaaggtctaatcatggaggtgggggctacagtgttggcttgtgctggggccagcatccttaggaaggcatcttggaggtggaggagacagccgcccacttcttgattggggccttcagcagcaccagcttcttgggcaggctggtgctggctttcatcaccatgtcgtgttcaatcttcttccagatcctgacttctaggttcagctttcctcagaccctggttcctttcagaggccattgctgctgccttgctctttgctggcttgtgccttgattatatgtctttgtacaactttttgttttcctggagttaatcttcacatctgttttcttggagttaatcgttacctctatatcgcttgcttattattctttggcctttttgtcttctcacaccttccaacttctttgtaatatgtgtttagtacaatttttcatgacaggtagtttactgaatcagtttttccccagtgtggtcatccaacttgagttatccagctctctgccccagtctgggcaggttgatcttcaggtctgtagtacacttgtatcctaggacttctctttgccattagcctggaatttcctttgcagttctcccgttggatgcccagttcctagatgccatatgtttttctatcgtctagtagcttcctgagagaagatgaatgggagggaaattgtatgaggttttgcattcataaaaatgccattttttttcctgtacacttggctgggtatggtgttctggggtagaaatcattttccctcagaaatgcaaagtctttgccctgttgtcttaaaatctccaacgtgacccgattccttaacctatgaatgtacttttctttggaagctttccatttttggggaggtgaagtgctaggtacttagtaggccttttaatttggaaacttacatcccttcagttctgggaaaattttcttaacatttctctgagaagttcttgccttttattttctgtgttctctcctgaaattggttagttggatgttggtcctcctagattgactcacatcttacctttttcttttctttttctggtactttttagatatccatctcaaactcttctattcattgttatgtttttaacttctttcttttctttgtctcttgatggggtcttgccctgttgcccaggttgtggtgcagtggtgcgatcatagctcactgcagcctcaaattcctgggctcaagcagctgttctgcctcaccctcccaagtagttgggactacaggtatgcaccaccacgtccagctattttctttacttttttttttttttttttgagatggagtcctactctgtcgcccaggctagagtgcggtggtgggattttggctcacttaagcctctgcctcccaggttcaagcagttctcctgcctcagcctctcaagtagctgggattacaggtgtgcaccaccatgcccggctaatttttgtatttttagtagagccagagtttcaccatgttggccaggctggtctcgaacgcctgacctcaggtgatccgcctgccttggcctccgaaagtgccgggattacaggcgtgagcccatcattagatctttaaataccagtatctataagtcttttcctcttgagtcagctagtatccctggaaggaaattactcattttcctgcttggaggctataagcttggctatgtttatcctgcaaccggggactggaagggaggggactgacagtgttgctggtcagggtgccctcttactttttgttttctgtgtgcatctcacgtctgtcctcagcctatgtaaacacctcttgagattatccctctcaatctttgccggaggtgggggaggggctgcttcctgggctgccttggattggagggaagacctcaggtgagtgggtgggaatttgcccaaggagccatgagaccagccactatttcaccctctccatccctccactttcagatgtatgtggcgcctccaaagcccgagctcttcttggcgtctgtggcttcaataagcttgctttttgctggtatccctcctaccctcccctgtccccagcaaagcttgcatttgaacttcttcctacgggctaacaaatcagtcagttatgtagctcttgttactttttagcttccgaagttttgttgacacccgtagtctgctaatgtccctgttctgttctttctgttcgtgtaaatatatgctttatacaacttctttacatgatttttgtggggtttctgggtagcagagcttcacaagttcaatccagcgtgttggattagaaatctcccaccctctggtttattcttattctcaaaattacctgccaaacactgatactcccttgtttttccttttcctgacaggaaatgtacataccatacaggacagaaatcattagtgtatcccttggtgaataaccacaaagtgaacttaacccttgtaaccgccacccaggtcaagacagaatattaccaagcactcagaagcctctcccctattcccccgtcactgctcctgccttcctccccaaggtcatgactgctggcttctaattccagagtctgtttttaaattctgtgtacatagaccatggattaagtgttctttttgtctggtttattttggtcgacattaagttcatgagagtcttctatattatcgtgtgtattagtattcctgtagttttaggagcttcatagcattccattgtagggatataccacagtttattcattgtattatcactgggttgtttctagttcttggctattgcgagcagtgctactgtgaccactcttaggtgtgtcttttggagtacatgtgcaggtttccatcttgcacagctagaggtggagttgttgggtgatagggtgtgtgcatctcagctgcagtagaaactgccaaatagctttccttgagtgcttgtaccagctcacccttttgccactgtgtatggggattccaggagctctggtcctcgctagcacttggaattgctgatgcttttactcttagccttcctgatgggtgttttctggaatcacattatgattttaatttccattccttaaagtacccttggctctgaagtttaatgattcatgcatctcttcccttttgaagtactcttacaggtatgttgtgcatgtgttgaaaagtggcactatctattctaaaatacagtatgcctcctctgtgtttgaacagttgtagcgtggccttggggcctcctgttagctggcttggagaagggattcttgggattgtagagattagacctgaggaggccccttggagctctctgactaaattttattctttattattccaaactatttaagctcaccgtgtgctgactcatcataataatgagtagctctcattgtgcttgtctatttggactcatacaatgattttttttttttctttgagacagagtcttgctctgttgcctaggctggagtgcagtggcacaatctcggctcactgcagcctccacctcccaggttcaagtgattcttgtgcctcagcttctcaagtagctgagactgcaggtgcgtaccaccatgcctggctaatgtttgtatttttagtagagacggggtttcaccatgttggccaggttggtctcaaactcctgacctcaagtgatctgccttcttcagcctcccaaagtgctgggattacaggtgtgagccactgagcttggccaaagtagttttttaagatgttagtatcttttcttgcagctaaaaaagtttgtcagagatgattctactttgttctccaggtgttttctcagggagaaattggaggcagtaagccactgggggagtcctgtggctggggggtggggtagtcctgtggctccttgtcagggagtcctgtggctggcaaggagagaagtcctgtggctgggttgggagggagtcctgtggctggggtctcatcctgtgcctaacagtgtccagaggtgccgagaccagctcagtcggggagaccctaacccagcagcgctagaggaattaaagacacacacacagaaatatagaggtgtgaagtgggaaatcaggggtctcacagcctttagagctgagagccctgaacagagatttacccacatatttattaatagcaaaccagtcattagcattgtttctatagatgttaaattaactaaaagtatcccttatgggaaacgaggggatgggccgaattaaaagaagaggttgggctagttaaccgcagcaggagcatgtccttaaggcacagatcgctcatgctattgtttgtggcttaagaatgcctttaagcggttttccaccctgggtgggccaggtgttccttgccctcattcctgtcaacccacaaccttccagtgtgggcattagggccattatgaacatgttacagtgcttcagagattttgtttatggccagttttggggccagtttatggccagattttggggggcctgctcccaatacagaggtctcgtgtaaattccctgggaggcgataagcctctgagaaacagactatgctaaccacgccatgaaagagaaacttatttataaatcagatgccagttactagtttactgcttatttgcccaggcgtagctctgacagagtccccgactcatagtgcttgctcagtgcatgctgaacaatgattggaatcaagtcatggctcagagcatagttttgaataatgggaaatggatgttcttaagtaacatagtcaccaagataatgcgactagctgggtcaccccttttcaattttaggatatttttatcaagatttaaatggccatcattagagttatagcactttctcctttggattgtcctagaggcccatgagaaagtattccctaatttcttaggagaacagtttgtgggtagtatgcggtcatgtccagttaaattgcagatatttccgatcgaagatgttccagtcctgagaacttcgtgacattagcaggacttctacaagccatctcttagggtggggcatttactgcagttggctagtactcttttctccttaactttgtcatttgttgatttttttttaactgtccccaaatactgtgggcagagtgtatctagaattgaggcctccaccattgcggagaggacatggatgctgagcagtcccctgagtgaaggttataaagaagcaaatagactacacatgtctgtaaactgctcttgagtgtcccaaatttggggtacttcagttcagctgtaggaaaagcctcaaactgtttatactttgcaagaattggaaacttctaattcacgttaagttttatgtaatacatgataagcttcataggagcttcatcttttatctacttggacttttgcttccgtaggttttgttaaaggccttcatagcgaacctgaagtcaagctcccccaccattcggcggacagcggctggatcagcagtgagcatctgccagcactcaagaaggacacaatatttctatagttggctactaaatgtgctcttaggtaaggtggaggcatatgagtggaagagtctccagcatgtactcaagatagacctttgaaataaataaaaccagatgatccctcagcttctagaccaggctatttggcactggttgattgaatgtgaactgcactggggctgctgtgagcccgcatgggtctctgtgaccctgcagatgcagccgtgcccagggactgggcagtgggtgtgggctggtgtgagccctgtctgccacccagggcctggccctctgtctgtgtcggccatgactatggtgagtcttgtaggcttgagactgtgcctcgggttcctgcgggttctctgtaggtcagttgacagtttctcctgttgtttgggtaactgtggaaacgaacactggcaagtgctgaagcgagcatgtggacgtgcgatatgaaataacgacctggctttcaaaggcagtgaggctctctggaaaggaccttgctgagctagggatgtgggtgtgtagccattcccagtgggcctcatggcgtactcgttcatgatcatgtttgtgccatcttgatctctcaggatctcttcttttttaacagattaagccgggaatctccaaacagtgagtcagatgttaagatgtcttgcttccacccccacaggcttactcgttcctgtcgaggatgaacactccactctgctgattcttggcgtgctgctcaccctgaggtatttggtgcccttgctgcagcagcaggtcaaggacacaagcctgaaaggcagcttcggagtgacaaggaaagaaatggaagtctctccttctgcagagcagcttgtccaggtaggagcacagggtttactctaggccctgcatgtgaatgactgacattcaaagaaccgattaatttggaagagaagcggcagaaccgagagttagaggtgtggactctggagctgcgctgctcgtttccaaccctaggtgctgacctctagctgtcttccctctgtatgtccctgtcaccgtgagtcaaatgcgggtgatgcctcctcaggtgccgtgttacctaagcctctcagagaccactgctaccctgtttctaaaaccagaggtcacgatatgtgttcatccacccagtaaatactgattgagcacccactgtgtgctaggctctgggataggggctgggtatacaatggtgagtatttcagctgcagcttctgccccgtggaggctgtggcctagcacactggtctaggcacggtggtatatgctcactcaaggagatagggacgtggtcgtttggggtgtcggaacaaaatgtcggaacttctctttccaatgcagagaaaccttgcagtaattctaatgtactgtgattggcagttgacttcagttctttgtagcacgcttactcaggttatttcactaactatgtaaccatgcagcctcattttaagcaattggattttttgaactttacttaaaatgttatgtcagggtttttattgtgcttaatgtgtgccatttagctaagttttgtaggatacgaaattgtaagtggcttaaaatgattcttaatagaatcatgaattgaagataatgctaataatttaagcactgagttaggtagtgtttgtaaaatgcttagaatgcttcctggcacatgttaaggccatgtaagtgctgcgtgttgataaacagctgagcaaaagtggactcttaagaaagtattggggctgagagttctgttccaaccagctgccctttggttatttttcagaataaaagcagagtctcatgggatatgacatttatatttccttcacaaaaaacactgctgagtgttttgttgagtaaaaagggtgtagccatggtaataatacatttaaaatatagtttatttcatctttaccttgccttgttttttttttaagctagctttttattgagaattccacacatacaaaagtatcaactcatgaccagttatatttcatttataatcctacttctccctttttttattatttgaaagcaaaccccaattatcctcttatttcatctataagtatttcagtatctctatagatgaggactcttctttatttttaaaactttatttttaaaatgatggtcagatgcagtgttcatgcctgtaatcccagaactttgggaggccaagctgggcggatcacttgaacctgggagtttgagaccagcccgggaaacatggcgaaaccccatgtcttaaagaaaaaaatcagccaagtgtggtgatgcatgcctgtagtcccagctacttgggaggctgagatgggagggtcacatgagcctggaagatcaaggctgcagtgatccatgattgtaccactgcactccatcctgggtgatggagcaagattctgtctcaaaaaaacaaaactgcaaaacaacgtcacaaaacagtgccattgttagacctgaaaatattaaacatttcctacatcaaatacccaccaactcattatcaatttttctctctactcttttggaatcagcatctaaataaaattggtcgataaggattgtaaatctctttgatgaactggttcccctccatcccagtttttttcccttagagttcatttattgagaaaccagattgtttgtcttctaagttttcctgtggtctgatatactgcttccatctccactgtgtaaattaacacctttttctcttctctgtatttcctgtaaatcaataattggaggaaaagccttgtcagatttagtgtatattttatatctgagtccagtatttcttatataatattttaagataagtgtactcttttaaaaagtattgaaactatatgctcaattttttttaactgatgcttttaagaaggctgcttgatcataaaagtttagagatcattggtctgatgggaaaagcaaataattactaaaccgtttagcaaggttgaggtgcacatggtggggcctggagaagttcagtcatgagccgtcacttatgggcacgtggaatctgacccggcacagagttgggagaagacaggagctttatagacagaaaatgtggtctttgctaagtcccaggagtgaaagggtgagacagtgctcacagcacacgagtgtgggtgcgtagacagagcaagggtgggtcctgaaaaggcctgcaggctttctcatagattagcaagagtgctggttacggaggtttctaacatttgtgaacagatcgaaactgtgttaaattgggattgcagtaatcctggaaggacagggatagagggtgaaggggaaaaaagggtatggatgtgagacttaattgctgattttcttaagacctttctccaaagtaaataaatgatgtggcacatttttgaactggcaaattctaaactctagatatgattatctctataacatatcttactccatcttcttttgactaaaaactgttcttaattaaattaccatgagacgttcaattcagcaaatgtagtttggctaaccatatttaattagaatttaatataatcctaggcctggccaaactattaagcaagtgtgggcaaaatattgataattttagatatgcaggaacttagtttgctttccatgtgtgcttttcgaaaaaggaataaattgaaaaatagaggaagccctgaaatccaagaagcaaactctctcacctaggcatgcagtaaaagcaattctaggatgattgctgtttggcgcgtagttcgtattagaaaccattcttcttgaataaatagtatgtttaagaagctgggcagagggaaggcatatgcatatattatcaacaaggagggagaaaaaggcaattagtaaccatccataggagggtcagcaagatttataaaggaaatttgtgatccaagtatgaagcaaaataaggtgcagaataaattttaagcaagtaatagattagagtaagagaacccatttgaccattaaccttgggacattctctttcaaatgacatggagtagtactgaaatctttctttctttctgagtctaggttattgtgactggactcagaaagaaatatttcattattgcagtgaataacatttgtgaacattattgttcataaattatgcagtgaataacatttatgaacacgtgatgtgtaagatacatactgtttatttttagttaagttttttggctcaacttctaggcagagaacattaaatgtaaatagtgttacctaggagcatgtaaatggaaatctccatagtatgaaagcagtgctgttgctaacagaatttaggagggggcagatgaggtgaaggaaatgtgggtgctgatttccttattacattgagaggagccaggagattctttgttcaaaatggatggcttaagaagtcaaagtataagctgattacgtagagcaggtacccaaaaatgttttgtgtaaggggccagatagtaaatattttcagtcttgcaggccatcccaagtctgtggcagctactcaacactacctttgtagcatgaaagcagccacaggcagcccataaatgtggctctgttccggtgaaactttaggtacaaaagcaggtgcaggccagacctgacctgtgcactgtggtttgctgacctgggattcaggggtatagaagttaccatcagaagagctaaaagtgagactttttactttatactcttctacactgtctgattttgaaaaaaagaaacatgtattttataatattaaagatagggttggcaaatagcaaataaaaatacagaataccagtgaaatttgaacttcagatacattatgagtaattttatggtgtaagtatattccaaatcatgtgggacatacttacactacaaaattatttgttgtttgtttacagtttaaatttgagtgccttgtattttatctggcaactgtaattaaagggaaaaagaataaattcattatgttcatataatgtgatatagcaggggtccccaacccccaggctgcagagtggtactggtccatgggtccccaacccccaggctgcagagcggtattggtccatggcctgttaggaaccaggctgcccagcaggaagtgagcagcaggtgagctggcattcccacctgagcaccgcctcctgtcagatcagtggcagcattagattcccataggagtgcaaaccctattgtgaactgcacatgtgaggggtctaggttgtgcgctccttatgagaatctaatgcctgatgatctgaggtggaacagtctcgtcttgaaaccatcccctggccctgtggaaaaattgtctcccatgaaaccagtctctggtgccagaaaggttgggtagcactgtgatatagtattaaaagtgctaataaatatggcatactgcctttaaaatgtctggtagctctttctcagtggcactcataatagtgttttttgatttttaaatgtgtgtcaagctgactctcccctccgtgtatgctgggctttattttccctttcctagtcaccagttttgggaaatagagatcttcattctcatgctgctcctctagtgcaagtgctccatttatttttaaggaattaatataacaaaaaatcatgggaatttagaaaacaacatggaagctaatgatcacattggtggaagtgatagggaaatatttagggggagaagttaaggtataaactttgtcaatgaagtcctattaaaaacaacaaaaaagtgaagcttaggatgcattttataaactctgaccagaacacctgtgtttctctgtttctaggtttatgaactgacgttacatcatacacagcaccaagaccacaatgttgtgaccggagccctggagctgttgcagcagctcttcagaacgcctccacccgagcttctgcaaaccctgaccgcagtcgggggcattgggcagctcaccgctgctaaggaggagtctggtggccgaagccgtagtgggagtattgtggaacttataggcaagttattagcaaggtctactcttacaattaactttgcagtaatactagttacactctattgattatgggcctgccctgtgctaagcagtctgcattccatcttccttgccaaaacttataatacaaatttcatctttattttataaataggggagttgggctgggtgtggtggctcacgcctgtaatttcagcactttggaaggatcgcttcagcccaggagtttgagacaacctggccaagtgagaccctgtctctacaaaaaaaaaaaaaaaaaaaaaattagctgggcatggtggcacatgcctgtagtcccagctgctttggaggctgaggtggtaggattgcttaagcccaagaggttgaggctgcagtgaatcttgatggcagctgcactgagcctggtgacagagcaagatgctgtctcaaaataaatttaaaaataaaataagagaattaaagtttagcaggttgggtggcaaaatgaggccacacatttaaagcccctcctcctgattcttttctctgccttggctgcctcctgtggcattttaggtgctgagaaatgaaaacagtagggaaaatagttccaggatcctcatgttaatttgccagaaatggcatcttcaagtcgtcagagggatctgagagttccttcctggcctgacttgagaaaatccgtctgtccccagctctgcgtctgcctccactgcccagtcacctcctctccatgctcttggggctgggccctaccccaccatgcagtgctgccctggagcagtgagcttggtgggtcctgtctggcatgagagctgcctttgggagctggatcccagcctctaccactgggtctggtgcctagcaggctatggataaacttctgctgactccggcctctcctaagccactgcaacgtggtcggtgtagtgcacagtgtgtgtgcagcgtggccttactcacagcctccacattagagagaatctgactgaagtcttactgctgcctcgtgtgaacataaatgtttgccagaaccatgagcaggaaatgttaatctgccttgtttcctgtcctttacacggaagaatttttttctgtatggaatgcgtgccttacaaataatgagtggaaatacccatcgctaatgaaaagttatacttgactgttagtcagctaaataatctgagatttctaatacttttaatttggcttttacaatgcaatttatcttagcttttttgatttcttaggtcatatctttagaactatatatttgaatgttaatgtaattttcatattgaaattaaaatgttgaactgcgatgttaagtgtttcctgtggaaaaacgttcacattttctctagttttaaagttgaatcaagctgtttgaagattttcacatttcttctagattttatcagcttgttactttatctgtcactttctgtgatttgcagctggagggggttcctcatgcagccctgtcctttcaagaaaacaaaaaggtgattatttcagaaatcagagtcttgtgttgaatcttactgattttcttgtatttctgtaatgtaatgtatcttgtatttcttgtaatactgtattggactctgtgtatatctcttctcagatgagtgattatatgtgtgaatgttgctggaatctgataaccaggcctgaatagttttgtagggtggcttttaaaaattactttcatatcagaattgctttgtcataaattttgaacgcatcataaatttctaatgttcggggtcagcagactttttttgtaaagggacagagtgtaaacatcttagctttatgggccatatggtctcttttgcaacattcagctctgccctgtgacaggaatgcagttgtaaagacatgagctactggccagctatgttccagtagaactttacttacagaaacagacaggctgtagtttgccaatacctgccttagggaatgtgttgttatattttgtgagttaccttctcagtaaattttatttagtattagtcaggaatattattaagtagcttcttttccagcctggtcaacatagtgagacccggtctctaccaaaacaaaacaaaacaaaaaaacagccacgcatgtggcatgtgcctgtagcctcagctgctgctcagggggctgaggcaagaggattgtttgagcccaggagtttgaggtcacagtgagctgtagtcatgccactgcactccagcctaggcaacagaatgagaccttgtgtcttaaaaaaaaaaagtttcctttgttgggttattttaatttggacctggttatcatttttcagccatatttaactttgtacatatcagaatgttctgataaaacttaacttttattaaagtgtttgtgatataatctgctagttttggtacacattatcttttgcaatgccagttattttcttttccagtgtgggtttgcataggaaaagaattgctgtcactttctattttgaaatcttaaaagactgatccttttttgtgtcatgatttgagtatttaattgagagcctaatgcctaatattatttgcagtattaaatgggatcttaacaggaatagcattctagccttcattgaattaagtaaacatttcttaagagaacttggaatctataatatttgcgtcatcatagtatgagatacttaatcaagtttgagattttagtgaaacattgtttagaagccaaaaggattctaggaaaaattaatgtctatattcttgaattaggagagattttgggacgtgtgactaagttacgctgacacttgtttgtttcttagtcgctttttccagtggcggtgagaacgaagatgactgattcacattgctcagatgagtttatcctcttctggctgggacatgggatatatcctgtctcttttaagcctttttggtatttttcccccattgagagctgtgtcttcaaactcttctgttatagctggaaaatcctttttaagtgaaatctgcccaaattataagacagatgaaggtagagttgtgttggatataggattagggtgaaagtagtgggggtgtcctggagcctctcttctggtggcagcctagctcttgtgcctttgaggaaattaccctggggacggctctgtggaacatatttgcaaaccactgatttggaagatagagatggcttttgttaagatctgaattcacctttttggcattttatttgatttctcaaggtaaagaacttattttgtaataaagtttcctattatttagtagataggccaagttgctgtgttaattccatgtagattttgggtttcctttgctcattttttcactcttaatctcacatcattgtaagtttatggaagttatcatacttctgactttttctttgaagagcagaaattagaaattcccaataattattttgatagtgtcatttaatgacactcacatgtgatgtagccacaaagatttaatgagttcagttttaaatcatattaagactgttggtttcatttgttctcattaatgtaattctgaagatgaacaataaaatgtatttttagaactttcaaatgaaatattatttcatccttccagatcatataatgcttaagttctgattgttaatcataaagtctagaaaattaaaagataataaaatgaaagtgacttttaggtattagagttttattataaattctggtgtgtcattggagctatgacatgaatatttcaaaggccaatagcattggatctttacagttataacttaccatttttaagtttaagtagtaatatagattatttaataatcaaaatcaataaatattaattattaaaatgttttgtggtatagtttgagaatcattgcttttaactttttccatataggtttattgactttaatagcattctaaacataacatctctacattctttgtgtttaatactgtggaggtataaaaatacttatatatgatgataaactatattagagtaaattaaatattcttatgagtttcattttagagtgcatttacttaattttgaagtccttatttttagcaaactaaaaggaatgttggtacattatttactaggcaaagtgctcttaggagaagaagaagccttggaggatgactctgaatcgagatcggatgtcagcagctctgccttaacaggtagttctcactagttagccgctggtgtggaccttcactgtctgccttccaccccttgcccttcctgctcgtccccctgcacctggtggacagcacgactgggggcagcagtggagccaggttgcttaaatggggcatattcgggcttcttttataatacttactctgaagcttgtgtgtctgtggtgtttgcatcatatatttgttgttttccatggtttaggctgttttaaaattaggtttatggcttgagcatagggctttgtgagtaggggatggcaggtcgaaacatctcatgagttggatgggttatgctgggggttgggaaatgggatgaaaaattatgggatgaaaaattgcctatggatagtttaacttgaaagaatctgcctttgtttacagatagttatcttttttcttttttgagatagagtctcacactgtcacccagtgcagatacccagtgtcactggagtgcagtggtgtgctcttggtgcactgcagcctccgccttctgggttccagcgattctcctgcctcagcctcccaagtagctgggactacaggtgcccgccaccacgcttggctaatttttgtatttttttgtggagacgggtttttgccatgttggtcaggctggtcttgaactcctgacctcaagtgatctgcctgcctcagcctcccacagtgccgggattacaggagtgagccactgtgcccggccagttacagatacttatctaatgaaattctctgtgtactttataaaagatgaggattaactgaaggtactaataactggattatatgagggtggttttggttgtataatcctatctaaaagaatattttagctataactgaaagtaagacttaaatatttagagaggaaaatctgaataattctagtagtaattatttatttacaaaataaaaatagatttttttttgattacacaaattaaacaacaataaaacatcacagcaatccggatactataaagctcacatgcttaccgacccaactgccccaggagtgaccactgccaacagcttcatgtcgacctttttgccataatttttatatagccttttttgtttttaaatggtaatttagaaagtcaactaggaaaatgtgttacaggtttatcttccaggagaataggactggagtcgagatcttgaatgtggcttggaagaaggcaagcccaccccagagagatgagttgacagttgtttctgaccactgcttgcttagagggcctgcgtgtctgtgaccgcctagctttgcgcccctgactaggctgccccttaattacaaatgtctttatatattgctccagctaaggcttggagtagtcggttaagaacttgaacttcggtttttgcagtgaaacagcatttgagaatatcaccttctgataagccttattttataaggtgggtactgtagtgggaggcagtgtgagagatgcttgaaggatgcactgctgtcctgcatttcagcatcttcaggatgctgtgcagctgaaacatttgataacggtggaactgttcgttattttgcaagcctgtgattccctattgaatgttttctctcgccatttgacaaatgagtgtttctctgtcttcagcctcagtgaaggatgagatcagtggagagctggctgcttcttcaggggtttccactccagggtcagcaggtcatgacatcatcacagaacagccacggtcacagcacacactgcaggcggactcagtggatctggccagctgtgacttgacaagctctgccactgatggggatgaggaggatatcttgagccacagctccagccaggtcagcgccgtcccatctgaccctgccatggacctgaatgatgggacccaggcctcgtcgcccatcagcgacagctcccagaccaccaccgaagggcctgattcagctgttaccccttcagacagttctgaaattgtaagtgggcagaggggcctgacatctttttttttattttttatttgagacagagtctcactccatagtgcagtggaggccgggcacaggggctcatgcctgtaatcccagcactttgggagactgaggcaggcggatcacttgaggtcaggagttcgagaccagcctggccaacatggtgaaaccctgtctctactaaaaatacaaaaattagttgggcgtggtggcacatgtctgtagtcccagctgttagggaggctgaggcaggagaattgcttgagcctgggaggcagaggttgcaatgagccgagatcgtgacactgcactccagcccgggcaacagagcaagactccatttcaaaaaaaataaaaaaataaagtgcagtggctcgttctcagcccactgcaacttctgcctcccaggctcgagcgattctcccgcctcagcctcctgagtaggtgggattacaggtgggcaccaccacactcagctaatgtttgtattttcagtagagacagggtttcaccatgttggccaggctggtctcaaactcctgaccttagatgatccacccaccttggcctcctaaagtattgggattatagttgtgagccaccatgcccggccctgccacctgccatcttttgagttcttccctggagacctagacctgaaccctcctgcttgttctcttgttatctaatacccctattgacagcgcagcttagatcattaatggagagcttgacctcatctgataccttcactgaaggaaacaacttagtgtcttttgtgttgaacactgaggtaaaaaattggaatagttgattatatgaactctgctaaaattgagtgcattttacattttttaaggccttgttgggccctggttaaataattatttttaaaaatccttaaggagcctattataaacagatctgtggtcttaatgaaatgtgattaatactgtgcattattttaagaacttttgacttttcaaaaaacttttacaacatttcccatttgatagcggcataggtttaagcacttctcatctctaagttagtggacaaaaaaccctcatggatagtctaataatgtttgctacaagtccatgttgagttttatactccattttattttcagttttaaaaactgtggttaaatatgtgtaacataaaatttatgttcttaaccattttttgcgtatacagttcgctggtattaaatacatttaaataatgtcatggaatcattgctaccacccatctctgtaaccttttgatcatgtaacactgaagctctgttcccattgaactctattcctcctttcccgccaagtccctggcaaccacgattcttctttctgtcttctgaatttgactactttgggttctcatatactttaggagtcacacagtatttgttttacttagcataatgtccccaaagctcatgcatgttgtagcctatgttagaacttcctaatgtttcaggccaaatactattccattgtatggataggccacattttgcttttccattcctctgtccatggacacttgtattgcttcatgttttagccattgtgaatcatgctgttatgaacgtgggtgtacagatagctcctggagactctgctttccatttttttggctaaatacccagaaatggagttgcttttacattccaattttaatttaaaacattcatatcattgagtgttttacttaatagtatagtagttaacaaacttaataaaatagtattttggtaataatttgctggtagtccattgttcagtttttttaggtaaattacacaggacatttcaagtggacatgaaacatcttgtgatgtggaatcatgccccaagctgatggctaaacatatgaaataccataccctaaatttagtagatttagtctttgcaatttaggagataacctgttatattgttaggtttttgtcgaaaagctttgtcctcatatttccaacttgctgtaaaatttgtttgtgaagacaaatatttttgtatgggttttttctttttcatattaaaaagaaatgtccacattggaatttttttggagtttttagagctaatagagcttttcataatgtagtgggaatgagtgatcagtaagctcttagcagtttccatgcgtgcatttctgtgccttgaaataaatgacagatgagtacatttgtgttctgtgtgtaaaatgtgctctttcctcattgcacttccatgttggagggcttgtctcttggtgatcacacttcaaaattctcacagccccccttgaaccgtttaggtgttagacggtaccgacaaccagtatttgggcctgcagattggacagccccaggatgaagatgaggaagccacaggtattcttcctgatgaagcctcggaggccttcaggaactcttccatgggtatgtggactacaggtgatgcgctacaaagtggtttgtattcagacctggacatcttaattatatctttgcttccaagaagaagtcctttgatactgttttctgagttctgaatagctgatgaaaatgaccaattgaggaataatcatactttttcttgatctaaatcttatacttttgagttatcttagcataaatgtataattgtattttaagtggaaatttgtcacttaatcttgatttctctgtttttaaagcccttcaacaggcacatttattgaaaaacatgagtcactgcaggcagccttctgacagcagtgttgataaatttgtgttgagagatgaagctactgaaccgggtgatcaagaaaacaaggtgagggacataggcttgagacgacttggtgtttctgagcttgtgtgaggatttaaaatcgccctggctactgtctactttattgctttcccatccctgggcctttaaatttcccctttaaataccagctcttcccaggcctgttgttttctgcctttccaggtactacccacagccttgagaattgcctgagttctgcctcctttgagagtgtgccccagacaaatctattctgtactgaatgtttccttgtctgatttcttggatcattcatttgatggttgcgtatggcctgcaacgtttcttgttttggttctactgaactgttctaaaagtctctcttcatattatctttttacatgtaaatgtaactgtcttcacttttaattcctcaaggacaaggaatagcgtttcacagttcgtcccatcaatcagaattatagcctttggcatctccctatctaccaggcccacttcctcttagatttgggcttccccaggctgttgcctttccccaagtagcttctgcttgtcctgtagaagacctttcatgctttgcttctgcagcagccgttcctgaatgcctagtgtcaactgccttcttaccacgcccaccctccctgcatgctgcatttatcccctgccacagccctgtgaccctgtgtcctgctgcctctgacttgtctgtttctgcttggccatggtctctgtgaggtcaggtgtgcatatgggcacaaaccagggcatctctttatccccagcacctggcttaagtgctgctctggaactatctgttgaatgaactaatgcatgaatgtattgttgagtatgagacaaacaagtgtcattgtctcctttctagccttgccgcatcaaaggtgacattggacagtccactgatgatgactctgcacctcttgtccattgtgtccgccttttatctgcttcgtttttgctaacagggggaaaaaatggtgagtacaaaaggggatgtgcacagttgaaggaaataactaggtttcagaggtcagcttggtggcctgtttttgccttgcgtgcagcagaggaagtagaatctgaggatgagtttggttttcactagccgaggggagggaggaaatgatgggagcaggtaggttattgggtctggttttgttcatttgaaaacaatctgttgtttgaggctgaaggtggcttgggtgatttcttggcagtgctggttccggacagggatgtgagggtcagcgtgaaggccctggccctcagctgtgtgggagcagctgtggccctccacccggaatctttcttcagcaaactctataaagttcctcttgacaccacggaataccctggtatgttaaaagttcacatcttattttctcagatttaatcattattgtaaaaactatttcagtattgactattttagttttagagcagtaagtgttttgagttcatttgggatatttgacctgcgttgtagctcttcagaaaacacatgaatagtgaagttctttgtttcatgggttccctttagatgaaacccatagaggagaaaagtagaaacctcagcacgtaagagccaacatatatacacatcggatttaaacctaaagcacaaattgtgcctggtcgcagtggcgctgagtcgcactcagccaggccaggcattcacactcagggtgagtgggaaccaggactggctgaggcagcagtggacccaagtctccatcgcgcccatgcttactatggagccttctcgttctctctttttctttgggtgagagggtacacttgtgtttttgaatttatatgaggtaagtgtgtaatagggttttttctaatcttttttaagtggaatctggaattttaatcagatttattatctgacaacctagaattataatccagaaagtctgtggtattgaggacatattggcaatatgatgaatctctaattcttaaatcctgaaacttttttttttttaatcacttagggttattatagtgaagtcatttctgaatttggatcttctcttcacacctctttttctctttcctgagaattaagcttttgtttcgagttagaaagttgatagtagggaattgttccatggctgagcaatttatctccacagaggaacagtatgtctcagacatcttgaactacatcgatcatggagacccacaggttcgaggagccactgccattctctgtgggaccctcatctgctccatcctcagcaggtcccgcttccacgtgggagattggatgggcaccattagaaccctcacaggtaacggccagtttttcagctgtgttttttctagttatgcttactaaggtttaagtttagatgatgatgtttgttgcttgttcttctggttaggaaatacattttctttggcggattgcattcctttgctgcggaaaacactgaaggatgagtcttctgttacttgcaagttagcttgtacagctgtgagggtgagcataatcttctgtggaaccatttcttcacttagtggacattttatcattgctacaattaaaattggagcttaataggaaatatttccatgcactctaaagctgtaaccagtaatacccaccatgtatccatctctcagctttagaaagaaaacgttgccagtaaagttaatgcttcataaacttcagtttaagttctaattctcagaatatttgtttgaaatagacctcttcctaaaggatatatttagaaataacctatcattaagtgtaaagtctgttgaatatgctgggcacggtgactcacacctgtaatctgaccactttgggaggccaaggtggaaggattgcttgagcccaggagttcaagactatgggcaacatagttgaccctgtccctacagaaaattaaaaaaaaaaaaaaaaaaagtagctgggtatggtggtgcatacctgtagtctcagctactcgggaagctgaggtggaggggggattgcttgagccccagagatcaaggctgcagtaaggcgtggttacaccactgccctctagcctgggcaacagagtgagactgtctcaaaaataatagtaataataatcagttgaattaaaaaaaaaaaaaaaaaaaccactgtgctaggcccatagtatggtaagagttaaagtgagccttagggattatttactcaacctctgtttctgtataaagtggaataggctcaattctttaagtgatagcatgttgaacctttccataccaactggctcataagtcacaactggccagtcaacaagagtaaaaattaactggtaaaaatcaaagcaaaaaacctacaattgtcaaatttgtgggataactcccccttttaaaatgtcatgcctgacagtaatttctctctagtttccaggttttcagtcagttgtgtcttttttgagcagaaggaagcatgctaagagctcaatcttgtggctagctgggggtctttgtgtcagccatgcatgtgatggtgcccctgggtgcttggggctgcaggggaggggtacagcagtaggggcctgttctgttctctcgtgctgtggagtacatagtgacatagtggggtggtccttggtgtaggtcccttgttcctacccctgggtctgagatttatttagaagtggtgttggggctgtgcggcaggcccctctgtaactgatcaatgtttgtgaagttgctgtttgagagttgaaaccatgacataagcagaaatggaaggaagaaagaaccagttatgtgaaagggacacatttacttttaagcttgtatttactgagataaagtattcttaatcaatgttcttgagaggtgtgggaaaaatgcaacatcctggttgcagttaaacccagaacattgtgtgttgaagagtgacggttctcaaaccgtcaagacgcgggtactgagtgggactaacctgctgtcctcttgccttggaccttgtgttccagaactgtgtcatgagtctctgcagcagcagctacagtgagttaggactgcagctgatcatcgatgtgctgactctgaggaacagttcctattggctggtgaggacagagcttctggaaacccttgcagagattgacttcaggtaagtgagtcacatccattagatttcatgaactaagctcaattgaaagttctgggatcacttgatgcaaggaatgatgttatcaagtaccctgtccatcagaaatccgagtggtttaggtagatgacagtgattttctcctcccagtggctttttgctgaactttgccctatgcttggaattttattttattttattatttatttagagacaagatcttgctctgtcgcccaggcttgaatgcagtagcacaatcatagctcactgaagctttgaactctaggactcaagtggtcctcctgcctcagcctcccgattagctaggagaataggtgtgtgccgtcacactggctaatattttttgtagaaatggggtcttgctatgttgcccaggctggtctcaaactcctgggcttgattgatcctccatcttggcctcccaaagtgctgggattacaggcatgagccactgtgcctggcctagaattttaaaatataagtagaagagtagatttttttttttggtagtcctcgtcatttaagtattctggatagtgggaataaaagagcttagaatttttcatctttgtcttaaacttttaaaaaaatgtagcttatattaattctgcttgtttaaaaagaatatactcttcattatactgaacctaggtaagacagctggtttatattttgttgcaattaaaaaacgtgagctgtggttgcagtgagccaagattgtggccattgcacttcagcctggcaacagagtgagacttggcctcaaaaaaaaaaaaataacatgagctgtgttggcactttcattttctaagagtagttttggctggagaagttttctttcagtactttcttttagaagggaaattttcctttataatttagggtttgttttttttttttccaagccaccttttatagagcccttgtgggttatttcatttaatccttagaatgtttataaatctgggcttgttctcggctccacccacagatagggacgctgagcgtgcatgagtgggcagcaagatagcaggttatggagggcccagctcaccccttctgtggcttgagccaattttatagggcacttacagagtcttttgaaatagtatttattttgaagaaaaagaaaaacagtttactgagtactgtcttattgagtctggaattgtgagaggaatgccacctctatttatttaaagccattggccttttttgttgttttgagtaagtgctgcccaaggtccttccagggcacctggatgagcctgctctggagcaagctggcggtaagtgtttactgagtaactaaatgatttcattgttaaatgtgctcttttgttaggctggtgagctttttggaggcaaaagcagaaaacttacacagaggggctcatcattatacaggggtaagcggtttatttttgtgagatgctgttttaccttcaagaaggtgaaagtgaggctttccttgtggaatttctctaaatgcattcgtcatgttttagatgtttatttcacagtttatatcatgaaagttataatcttgtcatatggatttaagtctagtaatgttgagttctttctcactagctttccaaaatatcttacctaaaatttagtcaaatacaagattatgtttatttttattatccttctctctaaagcttttaaaactgcaagaacgagtgctcaataatgttgtcatccatttgcttggagatgaagaccccagggtgcgacatgttgccgcagcatcactaattaggtatttaccaatattttatctcttttccttttttggttgaagtactaaaagatacgagaatggaaagagagggaagaattcaaaggatgtagagcagtattcctgaatctgagctcatttcagccattctattcttaaactataatgaaaaaaaaatccaaaaaagtctaaaattataattaaaaaaacaacaaaatactaactgtccattgtaaaaagtaatgcactttcattgtaaaaattttggactatagagaatagtactaagaagaaaaaaaaaatcaccttcaattctgctgccacctggaggtaatcactgttaatattttgctatatactctatgagtttcttgttcaaaatcaggtcaaaattacatgcaattttgtaatctgacaatttccacttaatattttattagcattttcctgttatgaaacagtaattttagttatgggtcgttgttttgctatgcggttgggataaaattttatatactttttttggcaattacttattatacataaatgtttgtgtatagttttctttttctgagaattcctggaagttgagttaccaggcccggctttgaatttttttttttattttttttttgagacagagtcctgctctattgtccaggtgctatctcggctcactgcaacctctgtctccctggttcaagcgattctcctgcctcagcctcccgagtagctgggattacaggggcacaccaccacgcccaattaatttttgtatttttagtagagacagggtttcacgatattggccaggctggtctcgaacttctgaccccgtgatccacctgcattggcctcccaaagtgctgggattacaggcgtgagccatggcgcctggccaggctttaaatttaaaacaaatcttctaatagctttatggaggttataatttacatttcttgaaatgtactcactttgagtgtatagtaaactccaattttatcacatttctgtcaccccaaatgtatccttgtgcccatttgctgtaacctccggttcctgccccaactcctaggcagccactcatctattttctgtcccttaagatttgtgttttcgccaggcgctcatgcctgtaatcccagcactttgggaggccgaggttggtggatcacttgaggtcaggagttcgagaccagcctggccaacatggtgaaaccttgtctctactaaaaatacaaaaattagtcggatgtggtggcacacgcctgtaatcccagctactcgggaggctgaggcaggagaatcacttgaacctgggaggcggaggttgcagtgagcagagatcgcgccactgccttccaacctgggcaacagagagagactgtctcaaaacaaacaaagatttgtattttctggacattttatagtactggggtcatagtatagatggacttttgcatttggcttcttttacttaattgtgagattggttcttgttgtagcatgtatcagtagtttgttcatttttattggcgaaagtattctattatatgaataataccatattttatctatccatcagatggatattatagagttcatgttttggctaatttatgaattatggtactgtgaacatttgcctgcaagattttgtgtagacatgtcttcatttctcttgagtagatcacctagaagtggatttttaaataattttggtacttactgtgaaactgctcttcaaaaacataccattgttccttccttccttccttccttccttccttccttctttccttcctcccttcctccctcccttccctacttccctctccctttccctttcccttccccttttcccttccccttcccgcctgcctgcctgcctgccttccttccttccttccttcgtttctttctacatatacacatttttttaaatttcaatggtttttggggtacaagtggtttttggttacatggctgaattttggttacatggtgaagtctgagattttagtacacctgtcacccgagtagtgtaccttgtacccaatatgtagttttttgtccctcaccttccagccttccgccttgtgagtctccaatgtccattataccacactgtatgcccttgcgtacccacagctcagctcccacttctgagaacatatagcagaaacatgccaaagtatactcccactaccagaatgtgattgtgcctgattcttctcaccagtacaaatatttcaaaaaaagttaaatatgtatcagttttttgggcagaagttgatacttctctttatttatttattttttttgagatagggtctcattctatgatgcccaggctggagtgtggtggtgcgatctcggctcactgcagtctctgcctcccaggttcaagtgattcccacgtcagcctcccaggaagctggaattacaggcgagggccaccactgccagctaatttttgtattttttggtagagatggggtttcaccatgttggccagactggtctcaagctcctgacctcaagtgatccacctgccttggccttccaaagtgctgggattacaggcgtgagctaccacacccggctgatatttctttttaaaataacttaccttcttttgaaagtaatacatgtttaatgaacagaatttaaggaaaatataaaaaaacgaaataatctttgtaatcaaactactgaaaagaaaaccaaagttacattttggtgcatattctttttcattttcatcattgtaatttgcatttctttgattacttgtgagacactcctttcatttacttaataggtttatatgacttgcctattcagagattttgcagctttaccattttctgcaaatgatagcaacttctttttgtttgtttgtttgtggagacagagtctcgctctgtcactcaggcaggaatgcagtggtggaatcttggctcattgcaactattgcctcctgggttcaagcgattttcctgcctcagcctcccaagtagctgggattacaggagtgtgccaccatgcccggctaatttttgtatctttagtagagatggggttttgccatgttggccgggctgatcttgaactcctggcctcaagcggtccccctgtctcggcctcccaaagtgctgggattacaggcgtgagccaccgtacccagccagtagttacttcttatattctagaaaaaattctactcatgatcaagtctccatgaggaaagagactttaattgaagatcatggggcttgcagaccaatatgataaaatagttcattgtttctaaaagtattactgagtgttgatggcagatatgaacccttttgtttttgtaggaaaatgttacccgtattctccatttgaattcagtttagatttgttaggaatcgcagcttaagctttgccatctgggagtgtttgggacagttttgcagacaaaattgcaaaagtgcctaaggaatgcagctggcattcagacctgctctgtgctcagtactctgtggacagacactgttcagcacttgttgatcagaaggtttagaaagagaactttcaaagttggtttttaattaaagcatttaatagtgtaaatagaaagggattaaattttatgacagacaaaagaaagtacagcacccagctgggcgtgggggctcacgcctgtaatccagcactatggggggctgaggtgggtggatcacgaggtcaggagttcaagagttcaagaacagcctggccaaggtgatgaaaccctgtctctactaaaactacaaaaattagccgggcgcggtggcaggcgcctgtaatcccagctactcaggaggctgaggcaggagaatcacttgaacctggacggcagaggttgcagtgagccaagattgcaccattgtactccggcctgggccacagagtgacattctgtctcaaaaaaaaaaaaaaaagaaaaaaagaaagtacagcacccagttatgtccgagtgggtgcatgagagtgaccctgagattggagacaacgctgtcacgtgcttgaagaacgccacctgagaaagggggcgagaagtggtgtccgctggtaaccagaggtgttggcttagccatctgcagggaggagggtggtctatcacaggtgagtttcatctactttcttaagcaaattaaccttacttttgtgttaggcttgtcccaaagctgttttataaatgtgaccaaggacaagctgatccagtagtggccgtggcaagagatcaaagcagtgtttacctgaaacttctcatgcatgagacgcagcctccatctcatttctccgtcagcacaataaccaggtatgctgacccagtggcatcttcacattgtcgggaaaatgccctttcctgatgcctttctttaggctttaattgaaaacattttattttctagaaaaaagcttcagctcaggatgtttgagtgtaggtcagtcctttgataggatattatcattttgaggattgaccacaccacctctgtatttaagctctgccacaatcactcagctgtgacactgtaaatctcttaatagtttattacattccatgtgctgacagttgtatttttgtttgtgacacttacgtattatctgttaaaacattttcactttagttgtgttacctttaaagaggattgtattctatcatgcctgttgattttttggtgagcgggctattaaagtcagtgttatttagggttatccactagttcagtgatttgcgagattatcattcacatttattgtggagcttttgaatatcgtgtcaaatggccacatatatcccattcttatctgcttcttaggtgagtgggacacagtgctttaatgaagctataatcttcagaattctagcttgcagagaagattgcagaagtgataagacttgtgctttttaattttgtcttttaaatgttattttaaaaattggctttatatgatactctttttttctgctgagtaacagtgttttacaaaacttggactaaatgacttctaagcttaaatgatcacttgatgctttttttctgaattaggaactcagcttatcaaatatcaaagtcataattcctgaataaataacgtcttttttcatgtaaagactgctttaaaaaacacatggaaggctgggtgcggtggctcacgcctgtaatcctaacactttgggaggcccaggtgggcaggtcgcttgagctcaggggttcaagaccacccagggcaacatggcaaaacccacctctactcaaatacaaaaaattagccaggcgtggtggcgggcccctgtaatcccagctactcgggaggctgagggatgagaatcacttgagccccggaggcagaggttgcagtgagccaagattgtgccattgcactcccagcttgggctacagagtgagactctgtctcaaaaaaagacacacacacaaacaaaaaaaacatggagacatttttttggccaccttaatatttcccctcagataatttcctttgtttaaactcagaactggcattttctctcttggagaagattcaggacaaatactcctttaagataagtagaagcagtgaaagaggatttgattatcaggaatttgataagcttagaataaattgttgcttcttaatgtcatttcagaagatgaatatttattaatagatgccaactgagatatcattaaaattgattactaactactacttggaaaagtctcccagttccaaacttcagcaggcctcttgacaattcagctgtggtcaattgggtcttgcgtgatagatacaatgaccaattgtgcagcagagtgtgctgcttagctgcctattctgttagcattcatgtgttaacttaaaatcataatctccttagttttgttgagtgtctccgtggacaagacactgtgagggatacaaaatcagattggctttattcaaaccactggggtattataattcatttataatttattttattttttgccttttttccatgtgttctaaaggaattagagtttgtatataactataatgggggatagaaattgacatgtgccatgaagggaatgcaaaaaagtgccgtgggagatgagaagtggagaaaggaatttcttttttcttggaagcaggaataacttcatgaagcatgtatttcaacttaaacagatagtaggcaacgctgtaaggggagtatggctgcagcaaaagtgttcggggcagactgggaggaagggagggaataaattcagccattgttatggaataatgatcaaaatttattttcagcccgtttcacttaaaagttgagactgcttaactttttttaatctttaatcttaaacttttaaatgccatttgatctttaaaaatatatgttttaatagtgtattttaagtctctatatttttgttattagaatatatagaggctataacctactaccaagcataacagacgtcactatggaaaataacctttcaagagttattgcagcagtttctcatgaactaatcacatcaaccaccagagcactcacagtaagtctctttcttgatcggtcttactgacattgtaatagtttttggtagcttgtatggccagttagttgtatggtcatcttacggtgaggtgcttgtcttacagctcttacttatccatgaggcttgctaagaaattgtgcttctgtgaaaagaatctcagcttactccaggaatgtaaatgactatgttttttctgattattaaagtaatacacgcccaaaataaaaaaattcagccaatttaggaagacacaacaattaaaataagccaggcatggtggctcatgcctgtaatcccagcactttgggaggccaaggttgggggctcacttgaggtcaggagtcggataccagcctggccaacgtggtgaaaccccatctctactaaaaatacaaaaattagctgggcgtggtggcgggcgcctgtaatcccagctactcaggaggctgaggcaggagaatcgcttgaacctgggaggtagaggttgcagtgagctgaggtcaagccactgcactccagcctgtgcaatagagcgagactctgtctcaaaaaaaaaaaaaaaaaaagaaaagaaaaaagtaaactactgtcacctgcattggtaatgtatcagaagtttaaaatgtctagattataattaactcagtgacctggtaatatatactaagggaaaaatatttataatttacatttttacatttttatttttttaattttattattttttttttgagacagagttttgctcttgttgcccaggctggagtgcaatggcatgatctcagctcaccacaacctccacctcccgggttcaagcaattctcctgcctcagcctcctgagtagctgggattacaggcatgcaccaccatgcccggctaattttgtatttttagtagagacagggtttctccatgttggtcaggctggtctcaaactcccaacctcaggtgatccgccctcctcgaccccccaaagtgctgggattacaggtgtgagccaccatgcctggccttacatttttataataagaatttatgttgctgacattagaaaagaaccataatatccaagaatccaagaataattaaattatgtacatatgctagtatatagtgtgatgctttggagaatttttaacaatatggagatgtataatctggattgtaatattgagtgaaaaaaggcagaatacaaacctggtgggggtatagtcggatttcagttaagaaaaataatatttacatatatacatttctcacactggcagataatcaccaagataaattttgggattgtggatgatttttttcttctttatatttttcagatattctcaaattttctaaaatgagcaagtataacttttgttatcagaaaaaaataatatacaaaagtaatgttaatttgctggtgaccaggttaaacctttttatttttattttttgagatggaatctcactctgttgcccaggctagagcacagtggcatgatcttggctcactgcagcctccgcttcctgggttcaaatgattctctggccccagcctcctgagtggctggaattacaggcgtgtggcaccacacctggctaatttttgtatttttagtagaggtagggtttcaccaggttggtcaggctggtctcgaactcctgacctcgtgatccacccacctcggcctcccaaagtgctgggattacaggcgtgagctactgcgcccagccagacctttttattttatttgacaaaagaaatacttccatgttatagaagactaaatattgtttgggctgtctgcagtatggtcttcccttgatttgttcaaaatatcgtaaactttgcttatttatttttattgtggccgactgtgtcgggcactgttgtaggcttgggatggaaaaacaggattcctgcccttagggtttctgcaggctggtcagggagacgatgtggtaagctggagctcagctcctaaggatgtgcaggggcagttgagaggcggaagggtgggagatcattccagggtgtgggcagcacaggaacctctcttcattgggatataattgccattctgataacacgtgtttgaggtgtctaaagtaggaagttgtaccatggtgggacagatatcctgtggttatcatacacagatctcagttttcttctcattgtttgtactttttataaagggtaacaggagatataattcaataaacctttgtggtgtttgggtgtgattttattgtttctttcttctcagtttggatgctgtgaagctttgtgtcttctttccactgccttcccagtttgcatttggagtttaggttggcactgtgggtatgtattttcctcagtatatattaatagttgtctacaacagtatgacataaacatagttattaggatgccctttttctttctttttaagtcttttatcaatttggctttttggaaaaatatctgatggaatacttgtttctgctatattagctgtgtgagactagtgacaggagctgtgggaaatgaatgccaaatgttcttaggcattgatgggaatttcagggtgtggtcttcaagttcatttaagggaattttcatatgctggcaaaaggcttttctcattagcttgactctttccaaaattatttgctgtgaattagaagtttaggaaccttttttcacttaattgtgacctagcatacgaaatggtgatgatttaggaactactgttcttgtattaacagcttttatttaaaaatgattttcctccagtagatggccctactagcatctgggaaataatttcaagtcttctccagcattcaggaataggctttcattttgtgtatcaattactgagaatgattttggtgactcacatcacatttgagaagtaaacctgcagatttcttgtgtgtgtcagcaaatgaccaactgatatttgcttgaagtggattacattatctgctctagaatgattgctttcccaccttcctcacatacagactgagcagctacggtttctaatcataggtctggcactagacttcacttctgggcaactttggcattggagtaaaatgtattaatttaaagaaagttaaaaatccgttcaagtaaacatacagttctaatactttttacaatttaaaatatagatttaaatgataaaataaaaaagaaaatatgggtagacaccataatcctcgtttctgcatctgttcacaaggggttgatatttatgagttctattctccatatccattctatgttctcttaatgctcagtcagcacctcaggtggttggagttcaatgcttggtagtttgacttacactgtcttttctaggggattgagccctgggtagtcctgcttatttgaggttgcaatttgtctttcaataacttttactacaagatatggcgtgttaaaggataccattggggaaccaacataataatatcaggaaaactaaccacgtcagacctgccccattgtgtatcaagtacactatttttccatagtaataaagagttcaccccagccaattctcttttattttgtgcctgtttactcaatggcattaacatgcccaaatgtctgggtagctgtctcatctccagttcagcagaaccattgtcatatgccctagtaaaagcattccttcattggacacttaggccccaatactttcattcagatctactacctgatttcatttctcaaatgatttttatggagctctgatttataggaaagatgttagttgattaaaaataaaacaatttctgagctggtataaaatgtattgtgacatgccttcctcttggaattgcaagagaaaggaagactgttgtttgcttaaaaattgtctataatttgactttgcaaatgtctgcttccagagtgcctccactgagtgcctcagatgagtctaggaagagctgtaccgttgggatggccacaatgattctgaccctgctctcgtcagcttggttcccattggatctctcagcccatcaagatgctttgattttggccggaaacttgcttgcaggtactggtactgagttgaaacagggactccaggacttggattttgatttccttagggggaatgggggtggtgagcatatgaggggaaaatactataaggtcattgccagtgatggcttgtccctttagtcaaatttcagatgttacctatatgcataaacacatgcagttggcagctgttctgtgctgagtattttaaagtagcctcttcccaatatagcccctcagttaactacaagtaaactcattttgaatttcattttaatgggcaccatatgccagtactccctcgggcactgggatgttaagaaagtataatgtatggacttcattctcaagttagttttagattagagggggatacacgtaaacaaaagtgcagtggtcacacagagtggccctaatcactctccttgggcagatttatgggctggtaggaaagagcacaacacggagagggtgtagcaccttggcgatgataatggaggatgtggccagcaaggaagacggagtccattgaaattgattttgggagaagttgccaatctccatgaaagaattggggcctgtgctatttgcttcagggggctataggagagtttcgtgaaagggactaaaagatgagtattttaataagatcattcatccaacttgaacatgggctggaggagaaggtagggagactcaggagattaatgttgatgctaaggcaagataatggctttgggactgtagggaagacactgattgtaagagaatgaaggaggcagaattgccaggcctggttcaccaactgaacttcggttgtgaagacaaagaaacctgggatgacttcacatcctgggcaggtgtgtggtggtgacagtcatggaaattgggaacacagatttgtgcgggaaacatcagtttcagtttgagtttggcttatcagttgaatatcaggcacagatgtctggccaactctcaacatagggtcttaaatgacttcagttccccaagcaatttgtccttcccatgctattggggtggagaggtaatgtctgtgcccatatcacagccagtgctcccaaatctctgagaagttcatgggcctctgaagaagaagccaacccagcagccaccaagcaagaggaggtctggccagccctgggggaccgggccctggtgcccatggtggagcagctcttctctcacctgctgaaggtgattaacatttgtgcccacgtcctggatgacgtggctcctggacccgcaataaaggtaatgtcccacttgggtgctggattcatacagccttaatgactatgggtttccagactacctttgtttagtaatctgtcccttctttattctctttttgctttaaatgaacaaaattgctcagattgtgacactaaatttaacatcaaaatgtgaccatgtggatgggtgcagtggctcgtgcctgttattccagcactttgggagactgaggcaagtggatcacttgaggccaagagttcgagaccagcctgggcaacatcacgaaaccccctctctactaaaaatacaaaaaattagatgggttgggccgggcgtggtggctcaagcctgtaatcccagcactttgggaggccgaggtgggcggatcacgaggtcaagagatcaagaccatcctggctaacacagtgaaaccccgtctctactaaaaatacaaaaaaattatctgagcatggtggcgggcgcctgtagtcccagctgctcgggaggctgaggcaggagaatggcgtgaatccgggaggcggagcttgcagtgagccgagatcgtgccactgcactccagcctgggtgacagagcgagactccgtctcaaaaaaaaaattagatgggcatggtggtgcgtgcctgtaatcccagctacttgggaggctgaggcaagagagttgcttgaacctgggaggcggagtttgcagtaagccttgattgtgccgctgcactccagcctgggtgacagagtcagactctttccaaaagaagaaaaaaatgtgaccatgtgttttatagctcttttagtatcatcagtcactgttatccctaagagggaaatacctagctttagttttaggtttccagcattagccaagaaagctcagaattgatgttcctggccaagtacctcattgctgtctccttaaatcttggttaatggctactgtcctggctagcatagttatggagcatttccatggttgtagaatgttctgccaatctcagggacagttttgcttttctgtgaagcaataaaatcaacttcaaaacaaatgttaactatttgtacaatggatttaagatagaccagttcacatacttttttttttttttttttttgagatggagtttcattcttgttgcctgggctggagtgcaatggtgtgatctcagctcactgcaacttctgcctcctgggttcaaacgattcttctgcctcagcctctcgaggcagattacagctgggattacaggcatgcaccaccacacccagctaatttttttgtagttttagtagagacggggtttcaccatgttggtcaggttggtctcaaactcctgacctgaagtgatctatccgcttcggcctcccaaagtgttgggattacgggcatgagccaccacgcccagcctaagatagaccagttcacttactgtttatatctgattactctctctttgccttgtcttctacctttaaaaatctccctactaacttcccattctcctttagctgccatcagtcttctcccttctctgcaaacatctctggagagtcccagcctcagcccacagagcttcccactgctctgaggtggaccttgtttgcaaggcttctttggctctcttggcctggaccctgtctactacttcagccatccttccttaacccctgctggtggtttctgttgccacactccatagcagcgtttcccgcccagatcatgtctttacatctctgggcactgctctggtcctgcctgcctttccctctttgtatcctgcaggctgctacccccatcttgagtgtcctcttcagttggctttcagagggcctcctgggtgttcccttacccacttgccactccccagtcactgggttcagtccttcctgcccaccagcacatgctttctaggctctgtcctaggccgtcttctctctttgtagtctctgggccagtgctgttctagagagtggcagaattttctataaccatggcagtgctccatagctatgccaggcaagacagtagccactaaacacatatagctgttgagcccttgaaatgcagctagtgtgactgaagaactgaaccccgattcggtttaattttcattaaatttaaatttaaataaccttatgtgggtagtggctccagtattgggcagggcagcctgagagtcggggctgttctcctgtcttcagtgtctagatgagggacctcagaggacctgtctctggagctgcagttcaatgtagccagctgccccgtgacacttacatatagctgatttgtggatatgtcagacacggtgtgatgagctcagctttctgtcctcctccccacatctgcccctgccccatttaccccactttgtgtcttatcaagctagaaacaggtcaccacaagtcttcatttccactcaccaagtcttttgtttcccctactaaatattttgcgagaagaaagtgtgtacctttgtattcacatacatgtacatgcacatatacatgcacatatgcaggggtccccaacctctgttaaaaaccggactgcaggccgtgcgtggtggctcacgcctgtaattccagaactttgggaggccgagaccagtgcatcacaaggtcaggagatcgagaccattccggctcacacggtgaaaccccgtctctactaaaaatacaaaaaaaaattagccgggtgtggtggcgggcgcccatagtcccagctacctgggaggctgatgcaggagaacggcgtgaacctgggaggcggagcttgcagtgagccgagattgtgccattgcactccagcctgggcgacagagcgagactctgtctcaaaaacaaaacaaaacaaaaaaaaaaaaaaccaggctgcacaggaagaagtgagcaagcattaccatctgagctctatctcctctcaggccagtggtggcattagattctcataggagcgtgtatgagttcgttctcacacttctgtaaagacatacctgagacatataaagaaaagaggtttaattggctcacagttctgcaggctgtacaggcttctgtttctgggaaggcctcaggaaacttgcagtcatggcagaaggtgaaggggaagtaggcacatcttcacatggcccacaggaaaaagagagaaggagagagagagagagacagagagagagagagaaaaagaaagattgagagggagagaggagggagaaaggagagtgcctgtagggggagttgctacacaaaggagcaccagggggatggtgctcaaccattagaaactacccccatgatccaatcacctcccaccaggccccacctccgacactggagattacaattcagcatgagatttgggtggggacacagagccaaaccatatcagagcatgaaccctattgtgaactgcacatttgagggatctaggttgcatgctccttatgagaatctaatgcctgatgatgatttgaggtggaacagtttcatcccgaaaccatcccccgccaaccctggtttgtggaaaaattgtcttccacagaaccggtccctggtgccaaaaagtttggggacctctgcacatatgcatgcacctgtacatggacacataatacatgtacatatgcatactttatattctctgccacttctggtccagactgatatactatctcatttggattactgcactagccttttgttttggaaacagcattttttaaaaaatttaatttaatttttttgagatagggtgtcattctgttgcccagcttggagtgcagtgtcatgatcatagctcactgcggcctcgatctcccaggctcaagtgatccttctgcctcagccttctcagtagttgggactacaggcatacccaccatgcccagctaattttttgatttttttttttttttgagacagagtctcagcctgtcgcccaggctggagtgggttggcgcgatctcagctcactgcaacttctgcctcccaggttcaagtgattctcctgcctcagcctcccgagtagttgggattacaggcgcctgccaccacacccagctaactttttgtatttttagtagagacggggtttcaccatgttggccaggctggtctcgaacttgtgacctcgtgattagcccgcctcggcctcccaaagtgctgggattacaggcgtgagctaccgctcccagccaggaaacagcattcttgagataattcatataattcacccatttaaagtatataattcattctctttagtatgcccacagagttgtacagccatcaccagaatcagttttagaacccataaaggaactctgtactctttacccaaaacctccatgcctccagctgcaggcagccactaacctgccttctgtctctgtgactctacgtcttctggacattactgtggatgggctcatacagtcagtgagcttgtgactggtgccttctaccaagcagggttttcagtgtagcagcctctctgtttttcttttttttttaaattgtgacggaacttctgcctcccgggttcaagcgattctcctgcctcagcctcccgagtggctgggactacaggcccatgtcaccatgcctggctaattttttttttttttttttttagtagagatgggtttcaacatgttagccagggtggtctcgatctcctgacttcatgatccgcctgcctcggcctcccaaagtgctgggattacaggcgtgagccaccatgcccggctaacctttcatttactgtctgcatttcttccctgatgccttccagtccatgcacccgattgtagccattcatcctattatggtttaaggtgactgtcttagtcagcatgggttgccataacaaaataccatagcctgggtggcttcaacaacagaatttacttctcacacttctggaggttgggaagtccaagatccaggactttcgccttgccctcatgtggtgagggggtgaggaagctctgtggggcctcttatatatggatgctaatctcattcatgaggggtctgccctcatgacccagtcacctcccaaaggccccacctcctaataccatcaccctggtaattaagtttcagtgtataaatttgggggactatagacattgaaaccataacaagcacttttctaagatcagggagtgagtaagtagcagagctaggacctcaattccacatgtcagtcatcttgccttcactctgctccatgatggctgcctcctagagcattgggagtctcgatgttctatatgctctcatgtgttgtgtattggagatagttgaggctttatgaatacatctggatttgttgacttctagctttgctggtaaccagctgtgaccttgaataagttacttcatctctgagcctgtttcctcttttagaaacaggagtttaaaatgctgctttgggttgggcacggtggctcatgcctgtaattccagcactttgggaggctgagatgggaggatcactggagcttggagttcgagaccagcctgggcatcatagtgtgagatcctgtctcctcaagaaattaaaaaattagctgggtgatgtggcgtgtgcctgtggtcccatctactctggaggctgaggtgggaggattgcttgagcccaggaggttgaggctacaatgaaatatgattgcaccccatcctgggtgacgagtgagaccctgtctcaaaaaagaaaaaaaaaatgctgctttgtacccctttcatgtcatggcgtcatggccaacatagaatgccctggttgtttgctgttggagggcatgggcctgggggctccctgagggctccttccatcttcaactcattctctgtgcacctgttaggaagttgtgggccagtccctaccatgtatcattgtgtgggtaaaagtaaataaaatgtgtacagtgtctgaactgtacatatcagggtccaagaacaaaatgagtgacatgggttagctctttttaataaatggtaaaaccaaatattctaattttcagttttgttatacttccatcacatgtttttgtttttttgttttttgtttttgtttttctattttaggcagccttgccttctctaacaaaccccccttctctaagtcccatccgacgaaaggggaaggagaaagaaccaggagaacaagcatctgtaccgttgagtcccaagaaaggcagtgaggccagtgcaggtaggaaacagcgtggggaagggagggacatgagtgcagcatctgtcatgtagaaacataggatttaagtaacttggtgttttagagaaataaatataatacacatcagtaaagtgagagaaagtttctccaggtgcggttcaagatattagaaactaatgactgatgtacacagaccaccttttggtctgaagcatttctaagtgccactggctgacatgcagcccctacagcctccaggcttccagccctagcatggagcatcactctcctatgcttccctggttgcaggtgatggctggagaggcctcctgattttcagtaagggaagtggtgtagatgcttaggaatagatgtagtgagtgaaaaaactgattctgatatgtcaaaaattctgattggaaatggaatatttacatttggaagagctaaaggcgagagaaagtggggataaagtcatctgagttggaggagcttaaaccattcacaagtttggaggacctttttttacccatgaaaaggtcagaacagaaggggctaggatttaggtgtgactgcagtttattgaattcccatccatactgctctcggtgggcagtggcaggggcaggagaggagcctggcaaagcatgaagtgactgctgctgcctctgctatctgggacgcctggccacctgtctgtacagtctccctccagacccattctcacgctgtctcttggcacccaggggccagtgatggttctcccatttgttttgtgtatatagcatttatatcaaggctatttatttatttatttattttatttatttatttttttgagacagagtctcactctgtcacccaggctggagtgcagtggtgcaatctcggctcagtgcaagctctgcctcctgggttcaagcaattctcctgcctcagcctcctgagtagctgggactacaggtgtgcaccaccacacctggctaattttttgtattttttattagtggagacggggtttcaccttgttggccaggatggtcttgatctcctgacctcgtgatccgtccacctcagcctctcaaagtgctgggattacaggcatgagtcactgtacccggcctatttatttatttttaattgacaaaattgtatatatctgtaatatacaacatgatgtttgaaatatgtgtacattggccaggcgtggtggctcacacctgtaatcccagcactttgggaggctgaggtgggcggatcacgaggtcgggagttcaagaccaaactggccagcatggtgaaatcctgtctctactaaaaataccacaaaaaaaaaaaaaaaaaaaaaaagccgggcatggtggctcgcgccagtcgtcccagctacttgggaggctgaggcaggagaattgcttgaatctggcaggtggaggttgcagtgagctgagttcatgccactgcactctagcctgggcgatagagcgagactccgtctcaaaaaaaaaaaaaaaagaagaaatacatatgcattgtggaatggctaattaacctgtgcatcacctcacgtatcattgttttgtggtgagaacacttaaaatctactctttcagtgattttcttgcatatggtacattgctattaactgcagtcaccatgctatacagtagatctcttgaactcattcctcctgtctataaatgaaattttgtatccttgaccaacacattcaaggttttttttgagatggagtcttcttcacccaggctggagtaccatggcacgatctcatctcactgcaacctccgcctcccaggttcaagcaattctcctgcctcagcctcctgagtagctgggattacaggcacatgctactgcacctggctaatttttgtatttttagtagaagtggagtttcaccatgttggccaggctggtctcgaactcctgacctcaagtgatccgcctgccttggcctgccaaagtgctgggattacaggtgtgagccactgcacccggcctcaagcgttttaaaagatgctcttttctaaggattgactgtagtacaggaggaagattgacctgttgaaaagcctcagcctttacaagtgtaaaattatcagtatattactatcatctttctgatgaattaaataaactaaggactccaagtcaaaagtcttcaaactgaagtagaatagttgtatatagtgcttggcactttaatatttagtatcggtttaatgataatgtttgtgcctttgccgtctttaaaacatttttacatcatccctgtttgattacttggtgtgctcatgaagttgttggccactaaggaatcttaggctcagagaggttctggaattggccagtggtccttgaatcagctgctcctatgattctctaactgatttctcacaaagcaaacaagcaatcataacaaaacaactgtgcacactgctcttcttattttgttatttaaaaagtacttaggctctacttatgtttgttagtcaatttctcattacttctagttaatcaaaaggtcagaggaaatacttgaatattttcatactagaatactttaaaaaatcatgatttccagtaatctctttaaaacttggcaagttattttgatctaaaagtttatcttttgtgtgcatatttttaaagcttctagacaatctgatacctcaggtcctgttacaacaagtaaatcctcatcactggggagtttctatcatcttccttcatacctcaaactgcatgatgtcctgaaagctacacacgctaactacaaggtatgggcctctgcatcttttaaaaatatatatgcacacatacttacgtctaatggatagttgatgtttttcttatgatttgtaggatgtataagccctttgagatatgagttacatttagttttttcaagtttgtttgtctttcagctttgtttatgatagcttctatcatacaggtgttttggattttcatattgtttgtactcacagctaagattgattacagtgacagagctaggatgtgcagccaggttatagggggaagtggccctggtggagtctggagggatccgtgtacaggcttccttccctcccgtgaggctcacacaaaaatacagcaacatgctggtcctgcaggtaccctctgcctaacatgagccacaattccagactcacagaagaaaagcaggtgttcggcataaaccatgtgtttcaaatagtctgggcatggtgagccacttgttatcagctagggaaagtttatgtcagcgtaagaaactgttcaccagatacccccaagagccagcctttctgtctagggatgttttagttttttagttcatttttttttttaactttaaaattttctgttcatctgcaatttgttagatatgaagtatgtgtctaatttaatttttgtttttggttgtccccaataatgtttacagaagaatttttctgcactaattggcttgagttacttacattctcatagttctctagtttcagtagtttcatttattattttgttatatcaatctatctgtctgctcatctattagaagcatccttgttttttttttttcttttttagacagagtcttgctctgtccccaggttggagtgcagtggtgcaaccatgcctccctgcagtctcagggctcaagtgatcctcccacctcagctcctgagtacctgggactaccggcatgtgccaccacacccagctaatttttacattttttgtagagacagggtctccctaagttgcctgggctggtctcaagctcctggcttaagtaatcctccctccttggcctcccaaagtgctgggattacaggtgtgagcaactgcacccggctacaagtatacttcttaattattgtagcttaatggtatttatgaggggatcagttcccctgttgttctttagaattttctggatattcttctttattgattttgggatgtgaacaatagaatcaacttctacttgtagattgatttagggagaacttatacctcagatgttaagtcaccctgtccagaatgtgggatgctttcctatttgttcagaactttttaaattacctcagaagcacatgaaatttaaaggattttaaaaaaaacttaaagattatttcacatagctcttgcacatttcttgataaatgaatcctcaggtattcctctgtttttgttactaatagttacttcttatgggttttttttcccctgaaaatcatttatcaaacgtatgtggcttattttctgaaggatgtttgataattttggaagatatgaaagtcttcatattttacaaggtttgaggtctctttaagctgcatggttctcatgtcagctcccaaagcagaagacggcatgttgaaaaatgccgtagagaagatacttcttttccacctgttttcaactcatatcatcttgaatttcagggcacctttccatgctcctagtgcttgctatctgtttattattttccttcctgaataccctgaactccagcatgttctgctgtaattctggcctccctggcatcttggactcctgtttcctttgctctgtcatccccgcggtcagctcctgctgcgcagcttctcagctgaagtgcgtttggagtgcctggcgtgtcttgctggatctttgagtattgcctctggtttccttggttccttctgctgagttgctcagcgtctccactccccatttcttgtgtggcccttcctgcactcctctgattccttttgtcttccctggtttcttgctttggtttcgagtctccacagaacttttgcagctcttctgaagacctggaagctttttcatcttaattctcatctcatgacctcttttcccttctttgagagctagaacttcccatggtgaacttctctttccagaattccatgccttcttttccctcccacttacctgttgtccaggagaggtcagattgctgtgcatattggaggagaaccctttcttccctgggctcttcatctcacatgacatcaccacatcacctcgttccttggaccctcagtggtgtcactgctggatttttctttcctttggctggccttagggcacacccaggttgactagcgtagtcatggtatttagatccactcacattttcagtttctgtgtctgtctcttgcctgcttctgacttcgcccagagaaagcttctctttcacaagggttcttagatttatgttcactgagcaccttcttttctgaggcagtgttttaccaatatttattttcctagtcagtctcgccttacctttcttgttatgcatgtctttggtcctgacccattctctgagtctgtaaaatagaattgctgtataatttaattacatgaaatcctttagaatcttaacacatcttacacctgatttaatattttattgtatccaaattgaaccaaccctatgtgaatttgacagtgatttctcccagggatcctagtgtataaggaataggacttagtattttctattttttgatataccacataccagatactgattatgatggacatttaacccttttttctcattatgaaagaaagttaggaattatttcttccagtagcgccagtgtaacctgaaagcctttgaaagagtagtttttgtatagctatctgaaaggaatttctttccaaaatatttttccagtgctgacaacaaacacgcagacacaccctgcaaggtgagtgtacggcgccgcacagtggaggcatctgctgcagccgtcgatgtttgtgtctttggttgtacattatgagatcgtgacagggccagtaaccgtgtgttctctccttcaccttcccaaggtcacgctggatcttcagaacagcacggaaaagtttggagggtttctccgctcagccttggatgttctttctcagatactagagctggccacactgcaggacattgggaaggtttgtgtcttgttttttctccttgggttgtggctggcacacttgatgtgcgtcttctgggctgagttcatctaggatggagcctggttctccagggtgcctccgggagactcctccctgccccacgtgcttgcgtcacaggacccaagtctgactctgccttagccatgaagtttagggggaagtttctatttgtattctatttttgtctgttatcatgtattagcttagacccagtttagtttggaaaatcagtgggtttcaaaatgtgtttgtagagtcctttatttcttaacttgaccttttcaagtggaaaggggcaaaacagacgggtaagggggcggggcgggaggtgtgacttgctcttttgtgcctgaggaagtaacagagctggggttgacagtcatattctctgacacagatagtctctgacttatctcacagaaagtcagcggcagagcctgagttaaaagtctcgtagattttctttttcttttttttggtggctaatttcagttttatttatatttgtttatttatttattatactttaagttctgggttacatgtgcagaatgtgcagttttgttacataggtatacacgtgccatgatggtttgctgcacccatcaacccatcacctacattaggtatttctcctaatgttatccctcccccagtcccctcactccccatgggccccggtgtgtgatgttctcctccctgtgcccatgtgttctcattgttcaatttccacttgtgagtgagaacatgcggtgtttggttttctgatcttgtgatagtttgctgagaatgatggtttccagcatcatccatgtgcctgcaaaggacatgaactcatccttttttatggctgtatagtattccatggtgtatatgtgccacattttcttaatccagtctatcattgatggacattcgggttggttccaagtctttgctattgtgactagtgccacaataaacatacatgtgcatgtgtctttatcgtagaatgatttataatcctttgggtatatgcccagtaatgggattgctgggtcaaatggtatttctagttctagacctttgaggaatcgccagactgtcttccacaatagttgaactaatttacactcccaccaacagtgtaaaagtgttcctatttttccacaacctctccagcatctgttgtttcgtgactttttaacgatcgccatcctaactggcgtgagatggtatctcattgtgattttgatctgcatttctctaatgaccagtggtgatgagcattttttcgtatgtctgttggctgcataaatgtcttcttttgcgaagtgtctgttcatatcctttgtccattttttgatggggttgtttgcttttttttcgtaaatttgtttaagttctttgtagattctggatgttaatcttttgtcagatgggtagattgcaaaaattttatcccattctgtaggttgcctgttcactctgatgatagtttcttttgctatgcagaagctctttagtttaattagatcccgtttgtcaattttggcttttgttgccattgcttttggtgttttagacatgaagtctttgcctatgcctatgtcctgaatgttatggcccaggttttcttctaggatttttatggtcctaggtcttatgtttaagtctttgatccatcttgagttgatttttgtgtaaggtataaggaaggggtccagtttcagttttctgcatgtggctagccagttttcccaacaccatttattaaatagggaatcttttccccattgcttatgtgtgtcaggtttgtcaaagatcagatgattgtagatgtgtggtggtatttctgaggcctctgttctgttccattggtctatatatctgttttggtaccagtaccatgcagttttggttactgtagtgttgtagtatagtttgaagtcaggtagtgtgatgcctccagctttgttcttctagcccaggattgtcttggctatgcaggctcttttttggttccatatgaagtttaaaatagttttttccaattctgtgaagaaagtcagtgatagcttgatggggggatagcattgaatctataaattactttgggcagcaaggccattttcacgatattgattcgtcctatccatgaacatggaatgtttttctatttgtttgtgtcctctcttatttccttgagcagtggtttgtagttctccttgaagaggtccttcacatcccttgtaagttgtcttcctaggtgtttcattcccttagtagcatttgtgaatgggagttcactcatgatttggctctctgtttgtctgttattggtgtataggaatgcttgtgatttttgcacattgattttgtatcctgagactttgctgaagttgctaatcagcttaaggagattttgagctgaaccaatagggttttctaaatatacaatcatgtcatctgcaaacagggacagttttacttcctctcttcctatttgaataccctttattgctttctcttgcctgattgcgctggccagaacttccaatactatgttgaataggagtggtgagagagggcatccttgtcttgtgccggttttcgaagggaatgcttccagtttttgcccattcagtatgatattagctgtgggtttgtcataaatagctcttactatgttgagatacgttccatcgatacctagtttattgagagtttttagcatgaaaggctgttgaattttgtcaaaggccttttctgcatctgttgagataatcatatggtttttgttgttggttctgtttatgtgatggattacgtttattgatttgcgtatgttgaaccagccttgcattccagggatgaagctgacttgattgtggtggataagctttttgatgtgctgctggattcagtttgccagtattttattgaggattttcacatcgatgttcatcagggatattggcctaaaattctctttttttgttgtgtctctgccaggctttggtatcaggatgatgctggcctcataaaatgagttagggaggattctctctttttctattgattggaatagtttcagaaggaatggtaccatctcctctttgtacctctggtagaattcggctgtgaatccatcctggactttttttggttagtaggctattaactattgcctcaagtttagaacctgttatcagtctattcagagattcagcttttttctggtttagtcttgggagggtgtatgtgtccaggaatttatccatttcttctagattttctagtttatttgggtagagatgtttatagtattctctgatggtagtttgtatttctgtgggatcggtggtgatatcccctttatcgtttttattgagtctatttgattcttctctcttttcttctttattagtcttgctagcggtctacctattttattgatcttttcaaaaaaccagcacctggattcattgattttttttggagggttttttttcgtgtctctatctccttcagttctgctctgatcttagttattttttgtcttctgctagcttttgaatttgtttgctcttgcttttctagttcttttaattgtgatgttagggtgttaattttagatcttttctgctttctcttgtgggcatttagtgctataaatttccctctacacactgctttaaatgtgtcccagagattctggtatgttgtgtcttcgttctcattggtttccaagaaaatttttatttctgccttcatttcgttatttacccagtagtcattcaagagcaggttgttcagtttccatgtagttgtgtggttttgagtgagattctcaatcctgagttctaatttgattgcactgtggtctgacagacagtttgttgtgatttctgttcttttacatttgctgaggagtgttttacttccaactatgtggtcagttttagaataagtgcaatgtggtgctgagaagaatgtatgttctgttgatttggggtgcagagttctgtagatgtctattaggtccgcttggtccagtgctgagttcaagtcctggatatccttgttaattttctggctcattgatctgcctaatattgacagtggggtgttaaagtctcccactattaccgggtgggagtctctttgtaggtctctaagaacttgcttcatgaatctgggtgctcctgtattgggggcgtgtatatttaggatagttagctcttcttgttgaattgatccctttaccattatgtaatggccttctttgtctcctttgaactttgttgatttaaagtctgttttatcagagactaggattgcaatccctgctttttttttgctttccatttgcttgttagatcttcctccatccctttattttgagccaatgagtgtctttgcatgtgagatgggtctcctgaatacagcacaccaatgggtcttgactctttatccaatttgccagtctgtgtcttttaattggggcatttagcccatttacatttaaggttaatattgctatgtgtgaatttgatcctgtcattatgatcctagttggttattttgcccgttaactgatgcagtttcttcatagcgtcagtagtctttacaatttggcatgtttttgcagtggctggtactggttgttcctttccatgtttagtgcttccttcaggagctcttgtaaggcaggcctggtggtgacaaaatctctgcatttgcttgtctgtaaaggattttatttctcgttcacttatgaagcttagtttggctggatatgaaattctgggttgaaaatactttttttaaagaatgttgaatattggctcccactcttttctggcttgtaggatttctgcagagagatctgctgttagtctgatgggcttccctttgtgggtaacccgacctttctctctggctgccctttccttcatttcaatcttggtggatctgatgattatgtgtcttggggttgctcttctcgaggagtatctttgtggtgttctctgtatttcctgaatttgaatgttggtctgccttgctaggttggggaagttctcctggataatatcctgaagagtgttttctaacttggttctattctccccatcactttcaggtacaccaatcaaacgtagatttggtcttttcacatagtcccatatttcttggaggcttggttcatttcttttcactcttttttctctaatcttgtcttctcgctttatttcattaatttgatcttcaatcactgatatcctttcttctgcttgattgaatcggctgtcgaagcttgtgtatacttcacaaaattctcgttctgtggtttttagctccatcaggtcatttaagctcttctctacactggttattctagccattagtctaacatttttttcaaggtttttagcttccttgtgatgggttagaacatgctcctttagctcggagaagtttgttattaccgaccttctgaagcctacttctgtcaattcatcaaactcattctccatccagttttgttcccttgctggtgaggagttgtgatcctttggaggagaagaggtgttctggtttttggaattttcagcctttctgctatggtttctccccatcattgtggttttatctacctttggtctttgatgttggtgacctacggatggggttttggtgtgggtgtcctttttgttgatgttgatgctattcctttctgtttgttagttttccttctaacagacaggcccctcagctgcaggtctgttggagtttgctggaggtccactccaggccctgtttgcctgggcatcaccagcagaggctgcagaacagcaaatattgctgcctgatccttcctctggaaacatcgtcccagagcacgaaggtgtctgcctgtatgaggtgtttgttggcccctactgggaggtgtctcccagtcaggctacatgggggtcagggacccacttgaggcagtctgttcattatcggagcttgaatgccgtaccgggagaaccactgctctcttcagagctgtcaggcacgtatgtttaaatctggagaagctgtctgctgccttttgttcagatgtgcccttcccccagaggtggaatctagagaggcagtaggccttgctgagctgcagtgggctctgcccagttcgagcttccctgctgctttgtttacactgtgagcatagaaccacctactctagcctcagcagtggtggacacccctcccccagccaagctcctgcatcccaggtcgatttcagagtgctgcgctagcagtgagcaaggccccatgggcgtgggacccgctgagccaggcacaggagagaatctcctggtctgctggttgtgaagactgtgggaaaagtgcagtatttgggcaggagtgtactgctccttcaggtacagtcactcatggcttcctttggcttggaaagggaagtcccccgaccccttgtgcttcccaggtgaggcaacaccccgccctgcttcggcttgccctccgtgggctgcacccactgtccagcaagtcccagtgagatgaactaggtacctcagttggaaatgcagaaatcacctgtcttctgtgtcgatctcactgggagctgtagactggagctgttcctattcggccattttggaagcatcccttgttttttgaggtggagtcttgctctgtcgcccaggctgacgtgcatcggcacaatctcggcccactgcaacctttgcctcctggtttcaagcgattctcctacctcagcctccggagtagctgggattacaggcacctgccaccatgcctggctaattttttgtatttttagtggagatggggtttcaccacattggccaggctagtctcgaactcctgaccttgtgatccacccacctcagcctcctagagtgctgggatcacaggtgtcagccaccacgcccagccatattttcagatctccctctctttgccctaaaccactgtgcttaataagtagtttttagtggccagcagtctccatgtataacacattttagcaaaatggaaaatactatatgttttaaatttgaacgtgagattatactgaaataaaaatcatctaactgggattctttaaatagtaagattttcttttttgtatgtgggtttttttttaaccttattattatgactgtcatatatagaaatggctgtttttcagttacagtcagtgaatgtatcaaatgctgccttatccaaataataaaagtaaattattaataagtcacaatttaatgaagattgatgttagttgatctttatattcttgaaatcagccatatggttgtgtgtgtatgtatatatttttaaaggtacataaagataataagctcatctctgaaaatttttacatttggcataagaataactggataattaagcatcttattctctggcctgtgtctttacagttaaaggtagatttactcacctctccttttttgtttttctaagttcatcttttttgctgtttcaagacagaggcccattttagctttctcgcatatccttttgtttgtactttggaagcctcacctgcttaattgttgagtttttatccgtggtcttttagagggggatatgtagggtagaagctttcacaggttcttgtttgcacttggcccctgactgttttgaggaatctccctcactgactcacagcatggcaaggtttcagatctctttctgccacacagcagttctgaggcagctggaaagatatccagatgcttagattgtcaggccaggcttgagatatacaaactattgagccttatctgtgaccttgcttaggtgaaggcatcagagcccctgcaccaacatgcataggcctctgcatgtgtgcggggctgggtgttgaggtctgagcacaagtgtagctggagaggtgagcttgatgtggcgacgggtatgagcaggttttcttcagacttctgtgagtttacctagttccaggatttaaaggcacagagactttagaattaaaatagaatcattttctttttctaaatagcaacactaggaataaaaaataataattccacattcttgacaggtaatgttttttcttgtcttctaatccttatttattccatactcatttttatacataattgaaatgtattatgcattggatttttcttttgcattatattatagacgatttttcatgtaactccttactgttccattttatatgttttgtctggtttaagactttatctgcaaaccgggaaactgtctctacaaaaagaaaaacaaaaatagttggccgcagtggcatgcgtctgtggtcccagctactcggggctgaggtgggaggattgcttgagccttgggaggttgaggctgcaaagagccatgatcatgccattgcactccagcatgggtgacagactttatactgtctgttttgggtgatttgataatgatatgccctgatgtagtttttttatatcttgtgtttcttgtgcctgggtttattgaggttgggtctgtggcttcatagtatttttaaagtttggaaaattttaggccattctttctttctttctttcttttttttttttttgagacagtgtctcgctctgtcgcctgcgttggagtgcagtgacactatcttggctcactgcaagctctgcctcctgggttcacgccattctcctgcctcagcctcctgagtagctgggactacaggcgcctgccaccacgcctggctaattttttgtatttttagtagagacgaggtttcactgtgttagccaggatggtctcaatctcctgacctcgtgatctgcccgcctgggcctcccaaagtgctgggattacaggcgtgagccactgcacccagctaggccattatttcttcaaagattttttttctgccctgcctccctccttttttccctctcttaaaggggctgtgatttcctgaatgattgcttagtgttgtcccatagcttactgatgctcttttcagtgtttgattgttttatgtgttttctgttttgtatagtttctattattgtgttttcaagttctctgatcttttcttctacagtgtctactctgttgttaatctgttaatctgttgttaatcctgtccagcgtatttttttttttgtttttgaaacagtctcactctgttgcccaggctggagtttagtggtgcgatatcagctcactgcaacctccacctcccaggctcaagcaattcttctgcctcagcctcccgagtagctgggactataggcacgtgccaccacacctggctaatttgtgtatttttattagagatggggtttcaccatgttggccaaactggccttgaactcctgacctcaggtgattcatccgcctcggtctcccaaagtgttgggattataggcatgagccaccgtgtctggcccctgttcagtgtatatcactaattttgtttttatctctagaagtttgatttaggtcttttaaaaatgtctccctgtgtttctgtttagctttgtgaacacaattgtaataactgttttaatatccttctctgctagttctaagatcttctaataacttcccagttcttggtgtttctcattggttgattgatactcctcgttttgggttgtattttcctgcctctttgtatggctgccaattttttattggatgcccaaccttgtgaattttactttgttggatgctatatatttttgtgttcccatagatcttcttgagctttgttctgaggttagttgagttacatatagatggtttactcttttgggtcttgctttataatttgtcagatgggttggagcagtgcttagtttaggactaattttttttttggactaattattcctctttaggaataattaggtaccatgcttaggaggcaagaccatcctgagtactctacctaatgaaccagaaagtttgggttttccagtccgcctgctgagaacagtgactttctagccctgtgtgagcgctgagctctgctccttctaatcctttccaatgcttctttccctggcctcagggagttttctcacacacatatctctgctgagtactcgagagggaccttccccagatctccagagctctctctgtcttgttttctcttctctggtgctctgtcttatgaactgtggctgtcttggtctccttagattctcagcacctcttcaattcagagggttgcctgtccctcctccttgtgccacagcctaggaactctctcaaagcagcgagttggggcagccatagggctgacttagtctctcgtctcccagggatcactgtccttcattgctcatgtccagtgtcttgaggactctgggttttgtctgttttgttttttggtttgctttggttgtctcaggcaggagggtaaacccagtccctcaccctcattgtgctcagtagtggaagtctcactctattacattagatattagtatttgtagcagagccctggttccctggtacttggggagctcttgaaaggccagaaacagcatgctttctcaccttttccagggcttcagtttctggtgcacatcaagcattccatacacatttgttaaagtcctttgttagacaagtagtgattcacaggttctatttgtaattttttcagttaacatgtattgggtatctgctgggagctagtaaaaacaaaaagtggtgtgtgacaaattcaattctgacaagaacaaccttaaacacttagaatatactttgagcatatcagaattttaaaaatgtgtggcccttgagtatttgaaaccaacaagaatctattgcttattagtagaggatattttgttaaacaagtggagagagaggcattttcagtctaattggtgttggcttttagcagctgatggaaaccagttcgtgattagccaggcagtggtgaaacaggctgtgcattctgaatgcctaggtatctaggcattcagaatggtggcgctctttgagttagcatcttcttctttcttgattcttttttttttttttttgagatggactttcgctcttgttgcccaggtaacaactccagtgcaatggcgccatctcggctcactgtaacctctgcctccctggttcaagcgattctcctgcctcagcctctcaagtagctgggattacaggtgtgcgccaccacgcctggctaattttgtatttttggtagagatggggtttcactatattggtcaggctggtcttgaactcctgacctcaagtgatgcacctgcctcgatctcccaaaatgctgggattacaggcgtgagccaccactcccagccccttcttgattcttgaaaaggacattgggtgctgtacatctcgttatagatgttgataaaaatgcttgtgagaagagtaacattaaggtagttatttggtcatttttgcagattattttaagacaattctaggactgatttgtggtaaatcacacattgctgtatcatagttgtgttcactgaacatattcaggggctctacagatgcagggctcttagctgctttgcacacttctgaattcctgccctgcgaacaggactggatacctaatagacaacaggtacttgataacagtttattgaattaatgagtgaatgaacagatacataaatgcatgaaagaatggttgtaatgtatataacttggatttcaagactttttactgactgttcaaaataagaaattgaaaactttcctctgattttcctctactatttacacaatttaaatggaagttatcttgtaccttcaatttctgtctaggattcgtacaataacgggtcatctctgagtcgcttaatgtctcacttgtctttctacagtgtgttgaagagatcctaggatacctgaaatcctgctttagtcgagaaccaatgatggcaactgtttgtgttcaacaagtaagagcttcattcttttcctcttctgttaagacgttcgggtatgacagcaaaacgctgctactccttaagaggcaggcgctgttggcataatcagctgggaggattgtggggtccagcgcagcactttttggctcagtccatgattgagccaagaggccatccttcccttcactccccaggaggacgaggtctgtcactgtggagggcagaggacaccagaagctcctctgcaacctcgctagttaacttccagtccctcggagtttctgtttagaatgctcaatctcatttagaattgcaaggaaacccaaaacgcctatttaaggtacaaacagcacttcatacaatatctcatgaggtattaatagtgattcacaggaagaatttcacgctgtgagtctttgctaacatatccagttatttacagatggatttgatatttgtgtgggagattcttaaaagtgttgttcacgccacattgttgatgcctcatttttttcactgtagttgttgaagactctctttggcacaaacttggcctcccagtttgatggcttatcttccaaccccagcaagtcacaaggccgagcacagcgccttggctcctccagtgtgaggccaggcttgtaccactactgcttcatggccccgtacacccacttcacccaggccctcgctgacgccagcctgaggaacatggtgcaggcggagcaggagaacgacacctcggggtaacagttgtggcaagaatgctgtcgttggtggaagcacgaaagagcaagcaggaaatactttgtaaaagaataaaaacgaaaaatgttagcgaacatcttctaatagtctgctgtattcagagaactctaggagatatatatggttgatgcaaagatgatttaaggcatagcccggccttccaagaagtgtgtggccagtgagtgagatgggcttgggacttacacatctcagaggtgggggtagaggaggaggaacactgagtgggctgagaagcagccagctctcattgccaaagtgtgtcagcaaaccagaatgcagttcataatgtccccacccattcaaagcacaggacctgtagagtggtgtggcatgtgttggtggcacttttcaggcctgtaacaaggatgaaagaacagcttcatagcagcacagtagtgctggtgttcagaggtgtgtgaaggccatagaagcatcttggatatattaccttgtgttttgtcagctttatgactagaagtctcttttcacttaaatttgttttttttttttttgagacggagtcttgctctgtcgcccaggctggagtgcagtggtgcaatctcagctcactgcaagctctgcatcctgggttcatgccattctcctgcctcagcctcccgagtagctgggactacaggcgcctgccatcacgcctggctaacttttttttgtatttttagtagagacggggtttcaccatgttagccaggatggtctcgatctcctgacctcgtgatctgcccgtcccggcctcccaaagtgctgggattacaggcgtgagccaccgcgcccggcctcttttcacttaaatttatgtttgtgtttttaatgcctagtatacaggacttcttaaattgccttaagtatgaacaggtatttgagttgctaatctgtatagtagcaataatagaatcccttgtttttccttttataaatttagcgattaaatagctacaattaaaacactagagtcaggagtcaaggaaaatacccatgttccaggctgtatgttagtgatgtacttactatatattggagtttcaggagtaagtctgtttcaatgctttctgtaaccatttggggtattaataagcatgtgagtgtgtgcatgtttgggttaatttcatatatgtttcttagaagggatatcattgatgtaaatattttaaaggcttgtcctccaaaaaaatcatgtaatttcttctaaattactgatcttttaaatgaccttcacctttctctcaaatctcacttaagactgggctgagtagtcagtttcctgtagcagaaaaaagctcagacttgagtagccttctgcgagtgaggagacttgatggctgtcaggcagctgtaaactctaaatagagtgtcattatctgaagagggcgatgctgccacactgagtggcctttcaagttgtttctcaatctgacacgttctgatcgtgtgaatgtgaaattggtttgagcaggagtatatctgagtgcagaggagattatttaaagatattctcattctctgcttcccttttattcccatttggcagatggtttgatgtcctccagaaagtgtctacccagttgaagacaaacctcacgagtgtcacaaagaaccgtgcagataaggtaaatggtgccgtttgtggcatgtgaactcaggcgtgtcagtgctagagaggaaactggagctgagactttccaggtattttgcttgaagcttttagttgaaggcttacttatggattctttctttctttttttcttttttatagaatgctattcataatcacattcgtttgtttgaacctcttgttataaaagctttaaaacagtacacgactacaacatgtgtgcagttacagaagcaggttttagatttgctggcgcagctggttcagttacgggttaattactgtcttctggattcagatcaggtttgtcacttttatctttcatccatcatacctgttcctaatttagtacaaattaccctaaaagacactgaaatctactttaaagaaatgtggtctgcatgtttccctcatcagttgctgctgcttatctttttcatgcacctagctggtgcagaaggcctggggcatagccagcctcagcaagtcagcatccttgccccagctccctggactcaaggctaacctggggttggctgttagggatttccaaaggtttgtcccatccacttgcctcccctccaaaataagtttgaatttaaattgtgagatacaattaagatttattgtttggggaacatttttgcaaaatctagagttagtttaaacagattatcaattattaccataattgatcatctgcagtttcaagctatctaacaggttcacttacctctttaaaaaggaatggaatttagcaggacagtaactgagacccgtgctcctggagtccatgtgggagctgtgtggctctgcacaagcatttgcacgcttcccctcttgactgcattaccttcctcctatagttgctgtgggcaccagattctggctagtcctgtcccttcatgatgcacattttcctcaagattcgtcccagttaaatcactgcagatgaaactgccttttcatcgtcaaaatttaactgtcatttttgagccgtgatcttgggctactttcttatgtggggtaggaatatttgtgagttagaaatattacacttctctatttccttctagacgtaaatctgttaatcctgtcagcactgttactcacctgaaagggtctgtttccctaggagaactgagggcactcggtcaacactgattttccacagtgggtattggggtggtatctgcttgttttttttgttgttgttgtttgtttttttttgttttttttttgagatggagtctcgctctgtcacccaggctggagtgcaggggtgcgatctcggctcactgccagctccgcctcagaggttcacgccattctcctgcctcagcctcccgagtagctgggactacaggcacccaccactacgccaggctaattttttgtatttttagtagagacgaggtttcactgtgttagccaggatggtctccatctcctgacctcgtgatctgcccgcctcggcctcccaaagtgctgggatgacaggcgtgagccaccgcgcccggcctggggtctgcttttaatgaaggaggcatcaaggggtgggctttgcgttggcctgatgctttcatctttctttcacaaaacctgtccgaagaaaatccgtctaaatgggccattgctctcctcaggaaatagtcattgggaacttcttttcctttcctttgacactaggaggctgactggggagaagccctggtctatggctgtgggcagcaggggctgagaggagcaggctctcaggggggcacgggtaccccaagggaagccagagccctgatttgttccattctagtaagaacaaagactgctctggtttcatgtttgttctgattgcctttcatcaaccggtcccctttctcccagttcttaagattcagtacagtgacagttttatgaacaagaatagaacactagaacagacaaaccattgaactctatgctgataaagatttattgagctcctgctgtatgtttgcattctgcccagaggctctgagaaaaccaggccatatgctccatgctttatccatggaagctccccgtcaggttgggaaagctgacagctgcagggaatacagtgtgacacaaaactggctcccatgcagcccttacgtgtcgcctctcagatggttgggggacgaaggtcgactcctttgggtatcttattactaaaccagtttcagggaatctgtgccaccctatctgccattaacgtgaacagatgagtccccaaggtgtaattttgggtattgtctgatgtctcttggaatttattatttgtttttccaatgagatttcacctcagggtatagtaaagttgttgaggggattcctggatgtgttctgcaattatctaggctgatttcagaatagagttatgcttatagtcaaatttatcagctgtcaagaattttatttaaaatttatgcagataagcaggaggaaaagaagcctggtttttacattttaatcctattattgatgtgaaattttattttccttcctgtaggtgtttattggctttgtattgaaacagtttgaatacattgaagtgggccagttcaggtaatagcattttattattttagatttttttcttcttcttgtgtacttacatgtaatttaggttattaagtgaatgtttaaactactgttaggcatttttgctgttttctttaaatggaaatctgactaacatactgtgcatttttgcttctcttaaaaattaatgtatatctcaagacttgtttggaagtagttatgtatctgaaaattccatatgttgtcagtattcattgcacatttcaaagcatttaattgtgttgacagatggtggaatgaaatcttgtggtggagcactagtttttaaatcttcttagagaaagcagttttatataatgttgtctttagtaattattatgcatttgtattctctgcagctttttcttgctagatgttgaggttttaatacttcttgctagtccattacaggtttataattattaaaagttaaaattcttttagtacctaaaatgcttaataaacattgtaattaggaaaatttagtgcagaaggaaagtgttcccagattccctggggtctggaaacatagtgtttattctaattacatgacacctccactgtgttttggggcaagttactgtttctcttttgagtttcaatttcttcaagagcaaagaggcagaggagagctaggaagatcgtagctgctgtgcccctgtgccgtcgggtgccttctacctgctgcctccgaacctttacacatgtccctgctctgcgcgagggcacagatgggatgcactgtggcaggggtggggttagagtagatcacggacacctgttagcttgatgtgtgcttgctgtcaaggttgaatcatgaattattttatgttgcttatattgatatgtatcttaattttaaaagaaaggtctaaatggatgtttttgtttttagggaatcagaggcaatcattccaaacatctttttcttcttggtattactatcttatgaacgctatcattcaaaacagatcattggaattcctaaaatcattcagctctgtgatggcatcatggccagtggaaggaaggctgtgacacatggtaacgggacacacctttcactgtcgtcttcggtgtcgtgatgtgcttggcagtgttcgttttcatatacccactttgaacgttgtcagtggcagccatgtgcttctcaggctctgcatgtgtgtctgtgtatgtgaaggtactggttagagacgtttcaaaagagaagagagcatattctttactctcagcaatttgtaatcttctcagggaaaaaaattcaagaaacagtaagataacctaaggtacagatagattctgaatataaagttcctgttcattcacatgaaacgctaaaagttcttcacttgatcttagccaaaaggccaagaagcgatgcaacactaaaaattcttaaatcgaacttgccgtgaattaaattttgatctctcatccagtggtattggagatatagtttgacttgggttcagggctttctgttttgcctgatgattttgctggagcttaaataaggaacccaggagatggccagctgtgcaagcccccagcctgtggaaggagctagtgtggttttatgaatgagttgcaaatctttctttgagctttttgaactgatcttccagcattgccctattgacccctccctgactcctttgctggaatctgtaggcttttgaactttgacagggacacatcctaagacccttgcaaactcccagatgtgagaatggcactactacttagagtcttttcgactcagcgtgtgtgcagaagagcatcaaccgggctgtgttgcgaggcagggccttggctgacctctcagtgtttacatagctaagccagttagtgtttgccacggcctcacaagggcttcagattcacacagccaaagtatagattattaaaggcataggtgtttggtttcctggacttggagggtctttggacagaaaatcagtaggcaaccacacccagtactttgtgctgggaagcttggtcatctgtgagagggtcagagagtatacccatgcgtgcatgccaccgaagggtcagtgagtattcctgtgtgtgcatgtctcagggccggagagagtatgtgtcactgagaggtcagagtgtttgtgtgtgtgtcaaagagggttgcattgtgcccttcactgaggggtcagagggtgcctcgcgtgtgtgtgtgtgtacgtgtgtgtgtgtcactgaggggtcagagtgtgcctgtgtgtgtgcttgtgtgtgcgtacatgtcactgaggggtcagagtgtgcctctgtgtgtgtgctcatgtgtgtgcatacgtgtcactgaggggtcagagtgtgcctctgtgtgtgctcatttgtgagcgtatgtgtcactgagggggtcagagtgtgcctctgtgtgtgtgctcatgtgtgagcgtatgtgtcactgagggggtcagagtgtgcctctgtgtgtgtgctcatgtgtgagcgtatgtgtcactgaggggtcagtgttcctatgtgctcatgacattgagggtcagagtgtgcctgtgtgccaatgaaaggcatttcttatatttttttatatgtggtcatagtagaccagttaatttattttgactcctgtgttagaccaaaataagacttgggggaaagtcccttatctatctaatgacagagtgagtttacttaaaaaagcataataatccagtggctttgactaaatgtattatgtggaagtctttattgtcttttcagatgaatcaagtagattattcttgagaccaggaatgttgctgttttggttatttggaaagttttatcattttcaaattgacttttgaatttgagtcaccttttttcagaagtggtgttaaattataggagccctaggttttttttctttttttagaagtcatcacaaaatgatcagtgttcagaggaagagctttgaccttccacatggtataatgattgataaccttaattcatctcttaccataaaccaagtatgtgtaagggttttctttatttcttgaaagcattttgtagatgttgagagcagttttccaaatgtaatttccatgaaatgcctgataagggtacccttttgtccccacagccataccggctctgcagcccatagtccacgacctctttgtattaagaggaacaaataaagctgatgcaggaaaagagcttgaaacccaaaaagaggtggtggtgtcaatgttactgagactcatccagtaccatcaggtaagaggaatgtatgttggaactgtcgtggatactttattgacccgtgcagatggaaggaagtgccatgtggtaacgctcactgttaactgtgttactttgaaccaggtttgggctttctggggcctgggtagatgccggtgcagggggatggggagggaggcggggggtgggggggtgtggtggagttggggaggtgcagtggcaggaggtgttgttggtgtgtatcctttttttttttttgagatggagtctctctccgtcgcccaggctggagtgtggtggcacgatcttggctcattgcaagctccacctcccgggtttaagcaattctcctgcctccacctcccgagtagctgggattacaggcatgcaccaccatgcccagcaaatttttttttttgtatttttagtagagatggggtttcaccatgatggccaagctgtttcgaactcctgacctcaagtgatcctcctgccttggcctcccaaagtgctaggattacaggcgtgagccaccatgcccagcctggtgtttatctttaaagtgggcacagccacaggagttcacctgactcctggtctgagagtcacgagatcgttcaagatagtgaggccctcttttccaaaacgaggaccaaaaatcaattgacagtgttggtcaagatggtagaaaccttaaaatgatagaaatctcaactctgaaataaaaactttatttgtatatttatttaccactattttgacatagggctaaggtctttttctttgagctgatttctggttttgttttcttaaagtggcataagaattcaaagacattttgaggaaggctgagtgcagaaatctctctttttaaatgacttctcctttcttttaacttgcactgttgtctagccctcacttattttgtcaattctttttagctgtttgtctttgaatcttcataaagccatagcttttctcataagaagcagcactttctttgttcattcatattttaatgaacccctgtagtatttaattaaatacttaatgcctaattaaatcacataattgcaatgcaaaagtacatgtatcataaagaggtctgaaaatgagcaactggcaagcaggtggtggcaggcagagctgcttgggtgggtgggtgtcatggagaggagttcatcagccacatgttcagtgagctctggatatgtctgtttagaaatgatcactaataaacttgtgctcaaccatgtatacctctgggaagcaggtgctcttcagtagattgcctctgcagagaacacagaattgaagtgaatgtccacaaaggcaatgagccacctgcagaatagtttagtcaaggctgtgtttgaagtttgccaaagattaatatacatttgattttcatgttgtgccttttctctgattgtgaaatattacaaattctatacaaataacaatgatggcaaatcctcctgagcaaagtgtgcaccttgtatgtgccctagaggaacttgtgtttcgttctgattcccctacatttctcatgtcatagagtgggggttgcattagtgtccccctgtcctcgctgggatcacatctgtttggatcctagagtcttccagctgaactgggacaagtataacagacggacacgtaggggtggaaaggcgtctcttggcagcagactttctaattgtgcacgctcttataggtgttggagatgttcattcttgtcctgcagcagtgccacaaggagaatgaagacaagtggaagcgactgtctcgacagatagctgacatcatcctcccaatgttagccaaacagcaggtttgtccccgcagccttggcttgttgttgcatagtgatggtagcttaaggtccttgtgaaaggtgggtggctggaatcagctcttccttcagtcctaatctgtgccttgatagcagttctccgtgctagtcatgggacagctgacttcatttcttctcacaatgccatctcaggttggtattgcccacctactttacaggggggatcccacagctccgagaggttatggaggtgatcaggcagcacacagctttagagtgctggggtgagggcgggccaaggctaactctaaagcccgaacccttacctcctacactgcctcctgcattctggtcaacccagtgttttatttggtggttagatttttgtttttgttaccttactgcttgtaatttagcagttttcctttcctttcccttcctttcctttccgacagggtctcactctgtcacccaggctagagtgcagtcgtgtaatctcactgcaacaacctctgcctcccaggttcaaccaattctcccacctcagcctcctgagtagcaaggaccacaggtgtgcaccactacgcctggctagttttttgtatttttagtagagatgaggtctcgctgtgttgcccaggctggttttaaactcctgggcgcaagtgatccaccaaccttggcctgccaaagtgctggcattacaggtgtgagccacctcgcctggcctattcatcactaatcagaatttctatgatcaaatgacatgaatcattgtttccacaactgcagtggaaggaaatggcctggcagtgccagtttcagaagcagcctgcccccagtcaggcacaggccactgtgcccccagtgtagcagcacctctgtagctcacagagaagggtggtggggacctccttgaggcagctctgccagaaaatctcatgagctgcctggcacagcttgaggttgccttttaagtggactcagcaaatacatgtttgttcatcttgattatacacaataaacaactactctgtatagtacgagtagtccgtggtttttggcatttgatttaaacttagaggcatgtgatattgatgttactgccttcatgactgcacccccattctgatttcataatggaatgttatcttgagaccagttagacaacaggacagggatcttggcttctggtgagattgacagcagttttagtgtggtcagggtctccctgcctacagatggttttagaatggtgccctggaagctttatcccattcttttctgtgcgtaatctgagtagagtggagatcgaaggcctgaatacatagtaaatacctgacttaatatctgccgcaatggaaattgtgtgatacaacatttatgaaacgcttagtgcagcacctgccaggtagctcaccacaggtgcatgttgcattcagaagtagtgctagatactatcctgttactggcagtgcatacatcagtgatcaaagcagattaaagaaagaccccctgccttcttggagtgaagattttgttgggatgcgggtaaggggacagacaatagaaaagcaagtgagtgaagtctataccatggcggctgatcaggaacaccgtacagaagaatccaggagggaagagagttaggtggtgtctgcggtgggagtggcattgttcagctggtgatgagaagaagctttggtgatctggtgacatttgagtgaatttgcagaaaggaaagatacaagcctaggagatacctggggaaggaacattccaggcagagcaaatagcagtgcaaaggccctggcggggggcggacatgctgttagggtacaagcaatgagggtggaggagtggggcagccatggggagggaagggagtgaggcctggtggggtgaggccagtgtggaggagccttgagagggtttgcgctgatgtggtgtaggttttagcaggatcattcttattcctgagttgagaatagccttgagggggaggtgagggcagagcagggccacccatgtgagacccggcactggagtggaatggcccaagtcagcatcccttggcagcatgaaagcaaaaccagcaaggtttgctggtggcttagatgtggcatgtgagagagagcagggctttgggggtgatttcagggtgaggacagggtggctgtggacaaggtagggcagacattgggggcagcaggaggtcagagcctgtctggatgtagcagttgagaccccataggtgcctaatgaggtgaggccagcatcaggtgtatgagcctggagttgtcgagagactgtggggcagggggtcagcatctgagatgtccactcacagtggacccagactggctggagaggaggaggagcttgaataccgagcctgctgagtcccagctccaaggtcaggtaggtgaggggagccagtgctggggcagggggagtaggcaggtgtggggttcctaaagccaagattttttttaaggcattttgtgcaggagggcgacatctgctgtcagcaccttgggaacttggcccaggtttggcagcaccgagggcactgatgagtgcttttggaggagcaaagggagccaaaccctaatgggaatgtgttcctgaaaggacaggagagagacttgggaaaaggttttacttgaagagggaacggagaaatagggcagtagccagaggaggagaggagtcggcaatgggttaagttggcagaaatgaaggcctgtttacgcactgagggcagaagcaacagggaggatcagttcatgacacaggagacacaaatcgccgttgtggtgttcacagacatgggttaggattggctgcatggatgacagagcactgtgggttctcccagagttgctggggaggaggcagagttggtgagcacaggcgagggtccaggatgcaggaatcctggagctcaagtcagttgttcccttgttgtaagatgtggccagtgttgtgagcttcacatctgtgccttgaaaaacaccacatctgtttgcagagttgtttactatgtatacacactcagtagaaacaaaaattggaaacagtcagtgcccaccatcaataagtaatggttgaacacactgtggtataagcttagactattttagcttgggctattttgcatgattaaaaatgttctggccaggtgtggtggctcatgcctgtaatcccagcactttgggaggccaaggcaggcagattgcttgagctcaggagtttgagaccagcctgggcaacatggtgaaaccctgtctctactagaaatacaaaaagtagctgggtgtggtggtgtgcgcctgtagtcctggctaactcaggaggctgaggtgggaggatcacttgagcccattcgtgcgccactgcactcctggggcacagagtgagactctgttagaaagagagagagagaaagaagagagagggagggaggaaggaaggaaggaaataaatggaagaaatggaagggaggaaggggagggaggaaggaagaaaggaagttcagccagttgccttgggagttctccattgcactgggttaagtgagaagagcagagacgtttatgatttttcaaaacaactaaaacaaaacctctgtgggtgagggggcaaggatatggctataggaacatggggcagattaagaaagggatatacacacaccacttagcatttgttacaactgttgtgggagggatggagtgcagaaaaagaaaaaaaaaagtgcacaccatcccatgtatgtgtatacaaagggacgcttggaagactggtccccaaaatgttggtaatgattgtgtcagggtgctgcagtgctagttgattttttttcacacttttgtatatttgagtcttttacagaaagcatttattatttatgtaataaaaatctaaatgacaagatttctgttatgggaaaaatgtagctatacagtgttgttgtaaaaatgtttgcttggttcaccactgaacttaaaatgcttttaaatgagggaaggtgacgatgagatgattatgatgatttgcccttgagttacatagctggtgtacaggaagctgtcgtttcttttggcttacgtagaaatgtttgtggtgtctaattccacagatgcacattgactctcatgaagcccttggagtgttaaatacattatttgagattttggccccttcctccctccgtccggtagacatgcttttacggagtatgttcgtcactccaaacacaatggtgagtctctcgcctggctcagcagatgaatctggacggcttgttcaggctctgattactgggaccacccccagaatgtctgagtcagtcagtttgggtagggcttcttgagagtttgcttttttttttttttttttttttggtgtgggggtggtgcggaacagagtctcactctgtcgcccaggctggagtacagtgtcatgatctcggctcactgcaagctctgccttccagcttcacaccattctcctgcctcagcctcccgagttgctgggactacaagcgcccaccaccacgcccggctaatttttttgtatttttagtagagatggggtttcaccgtgttagccaggatggtcttgatctcctgacctcgtgacccgcccatctcagcctcccaaagtgctgggattacaggcgtgagccaccgcacccggcctttttattttttttggagatggagccttgctctgtcacccaggctggagtacagtggcgctacctcgactcactgcaacctccgcctcccgggttcaagcaattttcctgcctcagcctcccgagtagctgggactacaggtgcgtgccactgtgcccggctaattttttgtatttttagtagagacggggtttcactgtgttagccaggatggtcgcgatctcctgaccttgtgatccgcccgcctcggcctcccaaagtgttgggattacaggtggctctcgcaccaagccaagagtttgcatttttagcaaattcccaggtgaaactaatgcctgcttttctgggagcacactttgggactcagtgatagagaggtttattggtaggatagtaaaataggagttattttctttcacaaaattggcaattgggggaaatttaatcttccttttttcttcagctgtgacttatgtattatgtttattttaggcgtccgtgagcactgttcaactgtggatatcgggaattctggccattttgagggttctgatttcccagtcaactgaagatattgttctttctcgtattcaggagctctccttctctccgtatttaatctcctgtacagtaattaataggttaagagatggggacagtacttcaacgctagaagaacacagtgaagggaaacaaataaagaatttgccagaagaaacattttcaaggtatgctttctatctgagcctataactaacccatgccttttgggaagtcacgtgatgtttcacagtcagtaagtctggaataatacctggtcttgcttcacttctgagttgggtaaagaagtctgtatcagtgtaattttctaatccgtcctgcattatctatggctcttggttcatacctgtcttgaagttctgtcatgttctgtctcttgtcctcagtagagatgctacagcagtggctcgcctcaggcagggcagggcagtggggtggctgtcctgggggcaggcagtaggggcacgctgacgtcagggaagttgaaacccaagagaagccagtaaaagtgagtctcagattgtcaccatgtgctggcagttttacacgctgtcagtaataaaagtcttctccctgcagggcagcctgcctccaataaatacgtgtagtatcaaatcctgtcttccctcataaattgtttggaagctccccaaggacagtgatgaggcactcgtaagtgcttgctgcctagatgggtccctctccacctttgctagattctgagcattcactgagttagagctgcttctgcaaatgtgctgcttctgctaagtggctgtgacttcatgcagccttcacttggtttgtcatcagtggagatgccctgtgttgtcgaaggagataagcccagtaagcctgctgggcaccttttggtttgcaggttcagcaggcagcccatggctttccctgtgtcgcattgaagcagctggctaaaattgatgatacattaaattcctgtgacagatgatcagcttgtatttgtgtaatggtgtacagttcacaaagcttaaaaaaatgctacctgccatttcatcctcagtgaggaaggtgatacacagagagaccaagtgactgtgtccacggcgacggcgctctgcatttcactttagcggttaatgtactctacctatatttttactttatatttaccatatatcttttcatgtatacttggcgtaagtgctttatagtagtcacctaattcactgtcatcttttttgtttcttggaaggtttctattacaactggttggtattcttttagaagacattgttacaaaacagctgaaggtggaaatgagtgagcagcaacatactttctattgccaggaactaggcacactgctaatgtgtctgatccacatcttcaagtctggtaggtgaatcacattagtcttcctggagtgtctcgttccccattctgcactatacactctcagagtgtaggagctgtgctgcccggtagaaactctgccttgcccagtgtgccagttgaaaatatttgttgctgtaagagtacacctgataccatgtgacccagcagttccactcttgggtatatacccaaaagaatggaaagcagggtggtgaaaagatatttgcatgccagcattcatagcagcattattcacgatagctaaaatgtggaaccaactgaagtgtccctcgatggatgaatggataagcaaaatctggtgtatatttacagtggaatattattcagccttaaaaaaaggacattctgacacatgctacaacatgggtgacccttaaggacattatgctaaatgaaataagccagtcacaaaaggacaaatactatgtgattccacttacatgagggacctggagtagttaattcatagatatagaaagtagaatggtggttgccaggggctgcaggggaggggagttatttttacaagatgaagagagttattctagaaatgaatggtggtgatggttgtataacattatgaatgtacttaatgctactgaactgtacagttaaaaatagttaagaggaccaggtgtcatggctcatgcctgaaatccaagcactttgagaggccaaggcaggaggattgcttgagccaaggagtttgagaccagcctcagcaacatggtaggaccccatctgtacaaacaaactagccggggatagtggtgtgcatgtggtcccagctactcaggagactgaggctggaggatcgcttgagcccaggaggttaagtctctagtgagatgtgttcatgccactgcactccagcctcggctatagagtaagaccctgcctcaaaaaaacaaaacaaaacaagacaagagccaaaaatggttaagatgggccaatcacagtggcttatgcctgtaatcccaacactttgggaggtcaaggtaaaaggatcacttgaagccaggagcttgggaccagcctgagcaacatatcgagacccctatctctacaaagaaaatcaaaaactagctagatatggtgggcacatgcctgtagtcccagctacttgggaggctgaggtgggaggatctcttgagctcaggagttcgaggctgcagggagctattattgcactccagcctgggctacagaatgataccctgcctcttattaaaaaaaaatccaaaaaaaaaaaaaagtaaacctgagagcttcctcctcctgtgttaaatttggaggccaagatgtttttgttacttttacaaatgatcaaggacggtgaaggttgggcatggtagctcacacctgaaatcccagcactttgggaggctgaggcggggtgatcgcttgagcttgagaccagcctggacaacatagcaagagaccccatctccacaaaaataaaaaaataaaaaaaaatagccaggagtagtggcatgagcctgagcccaggaggtcaagctgtagtgagccatgatcatgccactgcactccagcctgggcgagatcgagaccatgtctctagagaaagaaaatgacaaggacagtgaacccaagaaagtcataagatgccagctgtgcagcaagcatggaaagcagccagtccaaattaggacagtgtgttttccaagaagaacgatcgtttgtaatgagaatgctttgctttaaataaatgactaaatagctagaagcctagttctaggggataggcacgtctttcttctctcaagaaaatagaaaggcaattctaatttctagtaacagcaaacagcattaagtcatggtccaaatatgaggcaaaccaaaatgtggcttgattgttcagcagttgatctgttggaagcccttgatattaaaaaggttctcctttaagcggcttaggagtcacgatcaaagacctatagaaagagatgccatccttctaggatccttggctctcttgggaactagattcagatagtcataatgtaaatactgcttgagctttctttctttctttctttctttctttttttttttgagacagagtttcactcttgttgcccatcctggagtgcaatggtgccatctcggctcaccgcaacctctgcctcccaggttcaagcaattctcctgcctcagcctcccgagtagctgggattacgggcatgcaccaccacgcctggctaattttttgtatttttagtagagacagggtttctccatgttgaggctggtctcgaactcctgacctcaggtgatccacccgcctcggcctcccaaagtgctgggattacaggtgtgagccaccgcacccggcccgagctttcatttttgaaatcaatgtatgactgaaacactgaagacttactgacttaattatggtttcagaacagaatgaaaatgtcttcggttctgatgaatataaaaggaaaactaaccaagttaatttggcaagtagatggtagagatagaggtggggagtggaaggggaactaaaatcttcacctagcattgttgggattatatggttacatcatctgaagttgacagaccaaaatatagaggcttcagaggtctccaaatagaactaaacatgtaattcagattgttaggaggtagtataaatgagctaaatctcatctttattacggtagagttaatgggtgatgtctaaagttgtctgaagtctataaatcatgacaaattatgatgtggtgattgtattcaacagtctttcagttgcagggataaaaccccagtttaaactagagtaagagaaagaatgtgttggtttaagctcctggaaagtgcaggcaagggtagttggtaggactgcatctagtgttgtaattctgtggtctgcattgtatatttatgcatctcagctctgctttcttcttttcatttatataatttttaaattttattttaaagatagggtctcactttgtcgcctaggctgaagtgcagtggcatgaagtgcagtgcgaggctcactctagcctcgaactcctgggctctagagttcttcctgcctcagccttctaagtagctgagacaataggcatgtaccaacatgcctggataggttttaaaatttttttgtagaaatggaagtcttgctgtgttgcccaggcgggtctttaactcttagcttcaggcgatcctcctgcctctgcctcccaaaatgctgaggttataggtgtcacccaccacgcccagtctcatctctgcttcctgtgttagttttgttctctggtgggctgttttcacatgaccgaagatgacctctagcaggctgtgttctcagcccctcaagtaggcctatgtgattggccttgcatgagtaatatgggtgaccataaacccctgaatgctctggtccacatgggccaaatgggagactggacagcattccattgatgaggaggtggggctggtctccgggagtaagggagaggagcacatgcagtaactgatggtctgctgcaagggatagcagcacagcagttagaattttggaggtaactaccagaactgaaaacagaaatgataacaagtagttgccttaaaaagggatgggagcagggtgcttttgtgatcaaagctcctttctcttactggatttttgtacacattttgcatacatatcttagagtaaaagatagcattttcagccttggtccatttgaggatactcttggcgtggcccgcctccatgctagcaggctctggttgtgccaagttcagttgagcatcctggctcttgcctgcacggaacttccagtcagtgcgtcagtatcacaagtcttgatatttcctatgaagaagaacagtagtgcagtgacagacgaaatgggtgggcaggcagaggcaggatttctgagggagagaagtagctagctttttgcagagaagagttccggcacccaagagagcagctgagagtacaggcaggcaggcaggatgccggtagggcccggccgcacggcgccacagaatcctggagaaaggggcctcttcatggcctctgcattcagctgctgtcaccctccgcacaggccatggccaaaatttaattttcatagtggactctagtttttgagccttacttgctattattgaaataattttcttgtttctttttaaagatcttcggattatgcttcactgaccactgtaataagtttaaagttgagaaaatatggcttgttaatgaatgataggtcaattttagtatgttggtcattttaatattttgccaccagttggtttggatttgatgccaggaggagacagcctcatttctaaggactagtcttgcctttgtgggataagggtggtgtgttctgtgtccttctacatgtccgagcgatctctgtgcagctcaaatgtggtcactgtcttattgcgctgatttcctctccttccatctcacaattgaggcaaaatattgttactgttgaagtgttgtccaataggacttccagcagagacaggatgtctgcactgtctaatttagttgcctttagccacatgtggtgttctgtacctgaaatgtggctggtctgattggatagcttaatttataattttatttaattttaattaacttaaatttaaacagctctgtgtggatagtggctcctgtatgagacagtgcaggtctgttgagaagcagctttactggtgggagtggagggcttggagagggcacgtgggtttcctgctggtatcttttgaccttatttaatctgcccaacatttgcaagtaagttgtgtgtgtgtgtatatataaatgtgtgtttctgtcttcttgtttcctttgactgcatttatttgaaagacactaggtggcagaattactgtatttgattggtttcaagataagagttgaaataattcatctcgtgtttttatataagtaaggtgtgtttagcatgtaaaattggtaatatgtattcacgtactgcttaaacaaaggctatgaattccacccataaaccgaaaatgaagacctttaaatttgtccatttcaggcgtgggtacttcttaaataatacctggttcaggaactagtcagaatggcacccttgactttttgtttcctgcttttcctcttgttgggagaggagggtattcatcccaaagtggtttgcctatttcacattccatctaggataagcagaatagccaagaaagatagctgtcctcctgtttacaacatttggggtaaccagcatccctctcttttggtccaagatagactggtttagaaacagatgatggcaccagaggcccaggaggtggaaacatcagctttgtttgttgtccatgtggctgaattagagctgtctggccttgtagcctcaacacggccttccagctttgctcaccgtgattttcaaggacacatcttgtgctcttccctgcctgccatccagactatacccagtcagggtggcaggagctgctgccccttcctccctgagtcctggtcgtgggtggtggagatgtgccatgacgctcacggaggcatgctcaccccttcctctgtggcagaggggatggctgcacgacagctcttccctgtcctttccaaagcgtctgtggttccactttttggggcaaagcaggaatactggaagagagagaaagtggtcctttctatagtaataaagttgacattgattcaagttcatgcttggggaaaggacagggctactaacaattataatgctgggagcaatggaattttctcatgggtatgtggtaggtttaattttaattatcccagttaattcttagaactgctctgtgaagtatttcccgctttgtgcttaagttctaaaagatcctgtgccaaaaccaagaatgaaaacccaagcattctttcttgcccatcgatctttctctcatcaggccacttcttgggttgatagtggtgagtgtagccgctgccactttcagaatacccaccatgggccccagtcactgtgtggcgtggagaagagatggttctctctgtgtcatagctgaacaagcccagcccagagaggtttctgccctaggagctctcgatggtggaattgggatgcgatcccacatcctgcctgttttgaaaacagcattctttatttccaattcctgcttccattgttccttttaatatttctttgtttagctcacaaaaacacggcttgcggagctgctgcgtgcagctgtagctgtttctctgggtgcagcctgcatccgccttcctgcccgcctcctttcctgcactgccatcgtggtctccgggcacttggtccctttctcttcccctgagtccctttggctcccctgtgccacccttgtgatccacaggctctgccttctttctgtctcagactgctgctcatcactactcgggaccctaggaagggaggttccaccgagaagcatcttctcatctcagccacgttctcagtgccactgttgtctttgttaggtaatggtagctactgtaacaaataaaccaacatttccatggcttcacaccagagaaggttgtttcttggttttatgacaatgtattgagggtgttcttggttcacggatggttttcctccatgtgggaattcggggacccaggctcctttccttcttttggttctgttctccaggccttcacatcctctgtgtctggttggggacaaggagagggaaggtaaagaaggctttgtggccttggataagtgacaggcatgcctttgctggtgttctctcgtggtgacaggtcacagccccaccctgtaaaaggggactgagagacgtcgtcctgctgcttcccagcagcagcactgtggtctctgatgtgttttctgtgaggataaaaacaggtgattccaggatgaggaaagtcagggaaacccttggaaggaggggaccaggcgggtgtcaccatgggattagtggtggcttcagaatgagctgcagcgagtgccatgccttctaaagcttttgctattctgatatgcccacaccatgcccagcaggtgtctgccttgctctccgcagagagagtgatgaatccttctcatgagcctctgtccagttgttcctccctccacctggaagggaccctgggttcctcataacatcccagcggaacaggggaccttctatcctgtccccaagttcatcctcatcctcctgccggcttcctggcccctcttatgtctgcttcctgacgccacatccttctggattctctggaattgaattttgcctttgatgcttatttaaaaatatccattgcaggccaggtgtggtggctcacacctgtaatcctgtgcactttgggaagccaaggtgggcagattgcttgagcccaggagtttgagattagcctgagcaacatgttgaaatcctgtttctatagaaaatacaaaaattagctgggcatggtggcgcacacctatactcccagctactcaggaacctgagacaggaggatcaattgagccccggaggccaaagctacagtgggctgtgatcgtgccactgtactccagtctggtcaaacagagtgagaccctgtctgaaaaaaaaaaaaaaatccattgcatacttcaccgtagcgaaacatgtatgtcttacctttcctttcctgcctgtagctgctcttttacacttaacagccacactaagccagccttaaatgaaaaacaaaccagcacttcctgtgccctcctgcttccttcatgaggggtccctccctctgtgtacactccattctcattgcccatggtggtttgtttccctcttgtttctcaagccatggcagcctgcctcttgccctctttactaaaaaggcctttgcagaggctgcctgtgttctttctttctaggtctctctcatcctaggccctccagcttgattctgtggagctgccctcttgtcactcagtagcttgtggggtcttctctgtctagccacttaattgattgtgttcctcgagttgctgtccatggtctctcgttactgttttctctgtgtttctgcctctctccttggccttggtaggtccatcccctttgtgaccttggctgttgctctcatggacaactttctcttgctggtccttgtagtcctggcatccagcttctcgacacgggacttgtcctgccagtacctcagacttgcacttaaaattgaactagcaccactgtcactctccagggcctcttcttgttaattagatcattagggatgttcagaatcccagcatcatagtatgttcctcctcccgctaccccaggaaccctaaccttacctcctcctctctatctactaggaggtggccctcagagtccgtctcatcttccacctgaacttccctaataggctccagcagctgccaccccgggggctgagtacttcctccatgccttgtgcagtgctgagccctttacctgggttctcctgtttgctccttattacagccctgcgaacagatactgctcttaattccatcttacacctaaggaagctgaggccccaggtaaggtgcatccaaggtcacccaggtagtagacagtagagccacgatctgaaccaggcagtctgattcagagcctgtgttgacactcagccacctagaacacagcttggattgtgggtttctattacctgttcaaaacccctacatcccgggtctgtccctgcacgtgctctgtggcctggctgcatcttccttgaaggcagtgcatgcctcttcactcagggggcccatgcaggaacagagggccccacagaaggatgaggccagtgcagaatgggctggaggggacaatgctgaccaggaagcaagtgtagagaaatcccaggaaacctggaggagccagagacaaggcattagaactcctcgtcgtgacctggtctgcattctctgagtgtgctgcttctgttagctcgcttccttggtctcaggttatagtttaaggcattgtggagccctaaaaagcctgtactctgtttttacctgttttaggaccctttcactttggggatgtgttgattttttttttttttttttttttttttttgagatagagtctcgctccattgcccaggctagagtgcagtggcacgatcttggccactgctgcccctgcctcctgggttcaagcaattcttgtgctcccgcctcccaaatacctgggattacaggcacccgccaccacactcggccaatttttgtatttttagtggagacagggttttaccatgttggtcaggctggtctcgaactcctgacctcaagtgatctgcccaccttggcctcccaaagtgctgtgattataggcgtgagccaccacacccggcctgaaatttaaatcagaaataaaattttgatcccaacagtgatgccaggcagcccagatctgggggagagggtggccttggccagctgggcctttctctgtttcccaagtcttgctgcctctccctgctgggctttgcagcctgtgcatgtctctgtgcctttgaccttgtttatccaaaggagaggatagaatgaagtcatgattcctggagccctgagaaggatgctgtggagaaatttgccggtagaatctagctgagtgtgttgctgaggtgccagcattgtgtgtggggaggctgaccgcttggcctgcctaggcccaggatgctccatggccgggcacagaggccacttggctgtcaggtgtcaggagcctgcagagggcacacagagcctggaccgcaggggggtcctgctttctcacctggcctccttcagcatttctgtccctcagtccttagcaagcccaggagctgttgagtttggcaggtgccgagtgctgttcctgcctgtgtagctgtggctcagtcctgtgggggccccgctgtggcccgagtgcagtgattcgaggcgctgagtgttccctgactccttctccaggagctgtgttcagactttcgcagctcttggcttggagctcctggagggcttggcattgccgaccaatgtggaggtcgacagtgagagaggaggaatgctagctttcttgaccagtccattaaataagtgggatattggccaggcacggcggctcacgccttaatcccagcactttgggaggctgaggcgggtggatcacgagctcaggagttcaagaccagcctggccaacatggtgaaaccccctctatactaaaaatacaaatattagctgggcgtggtggcaggcgcctgtaatcctagctacttgggaggctgaggcaggagaacagcttgaaaccggaaggtggagtttgcagtgagccaagattgcgccactgcactccaacctgggcaacaagagcaaaactctatctcaaaaaaaaaaaaaaaagtaggatatctgtttctgcttagaaaaatcagaattttctaaatgccaggtgttctgaatacgtaagtatgggagacgactcagcctgtttcatttttatgtaaaatcttcgcgtagccatgtggcactggaccgagatgaaagcaaagacatttctccttaactttgtttctaggaatgttccggagaatcacagcagctgccactaggctgttccgcagtgatggctgtggcggcagtttctacaccctggacagcttgaacttgcgggctcgttccatgatcaccacccacccggccctggtgctgctctggtgtcagatactgctgcttgtcaaccacaccgactaccgctggtgggcagaagtgcagcagaccccgaagtaggttcataatgccccacagcccagggcgccagcccagcaccctgtcctgagactcccagtaacctgagctttggccaccgttaaagcattttcattttccattttttgtgagggcttgtgaaatttctgctgcatattaatattcctttcatggacagcatattattgggacaaacatgcggtccagctaaaggcattcaaaatagcagttgctttctaaatgcgattttctttggcaggttctttgacaccattgcatcttgtgggatatgcttgtcatgctctgtggctcctactaagttctagtccttaaattggttccatagccagacatgttgcaatgtcttaacctcattataaagtaaatgtggttctggttatccttagataatgaagtaacagtgtagcaaatttcaaaacctcttggaaatgttattttaccattcaaaaaggcttactaaggttctcgttatgggtggccctctttttgcaaaaggttttcaggcttaagctccatttctaggtgctccaacactccattatttgtatatgtatggaaataaaagctgtgaccacccccaaccctggcccccgcccagctgaatcctcagcacagtatttctggaaggctcaagatcccacgctggggaaaagaagttctggagacaaaagagggcaggtgctgccgtgcctctctgctcagtatggatactggaccttgtgctgccagggctcccagtagggccagttcatggcactcagctggaaagtccactgttgggaggcattcttaaccatccactctgtgccgtatgtagtggggtctggtcattctgttggaggagacagaccagtgacgacatttgaaatgcttggtggatgtcttaggcctgttacgatgactgagcactgtgggggcaggagacagaaagtcagtgtctcctagttctgtgctgctttaacgtgcatagaaatcagctgcggattcagcagatcactccttttctgacagatgggcctgcttactctgatgttatatcagaaagctctgaatctgggaattgtgtcccctgaattggagtaacagaaatgcttagatgatgagtgtttaaaagaaataaaccaaaggtaaatttagtttggaattcagcaagcgtcttcattcagccctctgagggcaaactacagctttttgtaaatgtaggtaaattctgtgactgtttcgtgaccccctctgatccagttttcctttataaccttctgtattgttccttctattatcctgaaataacattaatagattaggctgggcgtggtggctcatgcctataatcccagcaccttgggaagccaaggcgggcagatcacctgaggccaggacttcgagaccagcctggccaacatgatgaaatgctgtctctactgaaaataacaaaaattagccgagcatggtgacaggtgcctgtagtccctgctactcagaaggctgaggcgggagaatcgcttgaacctaggaggaaaaggttgcagtgagctgagatcgcgccactgcactctagcctgggtgacagagtgagactccatctcaaaaaaaaaaaaaaaaaaaaaaaattaatggatcaatggatttttaacctaataattaaatttcaaaaaatatcgttctttaatggtaatgtaaaggtaaaattaagataatatgtaacaagcatgtgagtgtctaaggtgtccccgtggtggaaggaaaaaataaatccccataagtgtccaagatgcccatagagagcagagctgttctggtttaaacccctgctcttagcactgtgtttttccagctgtgggtggtgggggatgagtatctttttatttccatgagatgagaaaaatgaattactagaagtgtgaaatacaaaacacagctgctctttttttagccatagactcagcagccataaaattgctgtatccagttgcagaaattcctgctgcttactcttgaccctctctcggtttgtgtgcatctcctctcaggctggctcccagatgggagctggctccaggcgacactgggtgctctgctccaggaggtccttatgtgggtcctgccctagcctagcccctctcttatggactctgtcactgtgggtttatgattcactctcaatctgtcttacctcttggtgaactgttagagtcctgcctatactttggcgcttgtgggtgtgttgtggtacacatgatgtgttggtcacttcccagctcatcttgttctgagtcaccctagatttgggacattcattcgccaccagtaccgggcggtgtatggcctgagatttgggggggcttgtgctgctacaaattggggctgaatttgagttgacagtggaccttctttatgtctactgctcatatttgaattgcaaatactgcctcttctctttcagaggctcattaccctatagctgtattattgcaaagtgcacaattacagcttgagtgtaagtcacactgcgctggcaggacggcccactgagaaagggcacgtttcctgttcgttagttttcacattgacacataatttacaatacagtaaaatgtacttttctatcaactgtagtcagtaacagcccccctcccccaaccacatcaagatatagaggagtgctgtcacttcaaacagttccctcttcctctgccacatcctgcccctccccaggtctaaccaccaatccgtgctctgtccctctgttcagcccattgcagaaggccatagaaatagaatctataggctaggtgtggtggctcatgcctgtaatcccagtattttgagaggctgaagtgggaggatgacttgaggctgggagttcaagactagcctgggctgcctagcaagaccccatctccagaaaaaaaaaatttaaaaattacaatcacgtccctgtagttcagctgcttgggaggctgaggcaggaggatcacttgagctcaggagttagaggttacagtgagctatgatcgtgccactgtgctccagcctaggtgacacagcaagacgttgtctctggggaaaaaagaaagaaacggaaccacgcggtgtgcagccttctgagtctggcccctttcggtgagcagtgtctaaagttctgtcgcgtgttgcccacgcgtcggtggctcgctccttgcaactgctgagcattgtatggctaggctgtagtttgttttcacttcaccagttgggaaacagagaaaaggcactttttaaaaagtttaaatctgtagaattttggtttttaccagttctcttctaaatcctgagggattacaggaaaagttgttgtatttcagaatattcttagcttgatgtgacctctgtccccgttaaggccctttgccgcaatgggaaggacgtcgctcggtcagaccctgaaggtcagaggggcagtttgggagtgtgtcaacattttaactgtatggactagagccaagagtctcaaggtttataattcccacgtattcaaaaagaaaaaaacaataaagtgagaagtcagtgtagagtgaaataacctgtgttagtggggaagaagtgtttttaaacaggatttccataacgtataacatcaacatgtttagagtggtgatgtttcattgggaaacgaacagtaaaacatgaaagcagggaggttttcattctggcagttggcaactttcacggcagatggagaatttcaaaagcaattgctcaattatcaaacatagccagtgtgagttctgaaataaaggtgctgattgaatgtgcagctttatggtggattttgctattcaggcaagcattttaattttctgcctgttaaattctgttttctttagtttttcatatgtggtttattgtagcttaggaatagataactgagagtatatattacacatacaacattctgatatggcaatatttaaaacaacttgtctgttttagaactagaattaaacataatcatcttcagtattttgcaaataagctcactgccatccagaaacattgtcaatgcatctgttgctccttctagaagacacagtctgtccagcacaaagttacttagtccccagatgtctggagaagaggaggattctgacttggcagccaaacttggaatgtgcaatagagaaatagtacgaagaggggctctcattctcttctgtgattatgtcgtaagtttgaaatgcctgtaaacggggttgagggaggtggggaccaggagaacatcctgtgtagatgacacttgcatggaccctctggaacccagaccgcccggtgtcctgccaagctccatcgaaactaaatctagaatgaatgtttacttctgctgtgacatataattggagaccaggcctggccttccagtcactggattctaagttggactgtgagagtttttgcagctgactcatttatcaaatgcccggctattggctcacgcctacatgatgctgggtatgtttgttaatttgagggaagcaatggaataataataactaatgatttaaaaaacaaagtaagtgcattgactgtagtggggttctgattttaaatttttttaaaaattaataccaggagcagtggcttatgcctaaattccagcaactcgagaggctgaggtaggaagatcacttgagcccaggagtttgagacaagcctgggctatggtgtgagacacccatctctaaaaaaataaaaaataaaaaattatccaagtgtggtggctcgtgcctgtaatcacagctctttgagaagctgagggcggaggatggcttgagcctgggagttcgagaccagcctggcaacacagagaaaccctgcctctaccaaaaaaagaaagagaggaagaaagaaaaattagcctggcgtggtggtgcatgcctgtggtcccagccacctgagagactgagaagggaggattgcttgagcccagaagtttgaggctgcagtgagctgtgactgtgtcactgcactccggcctgggtgacaaggcgagacccctgctctaaaataatttttttaagttaatttgtagaaaaggtgttagatgttctttgtcacattttatgatggattcctgtttaaatgccgttctctttaaagaaaaaaaaataacttgtgggagtttttaaccataaaactagcatcacatatttaccatggagaatttacaaaaaaacaaataaacggaggaaaataaaacctcctgtaatcatactactcagagataacttgctgttagattttggtctagatttaatactttttctatatttatattaaaaatatttaaaacatatgcatttctttgtcacaaacatggtatcttatagatactactgtcacatagcaaaacagtgttaaatattctgaatcagaaaaggaagccgactctccaactgaaagaggtgttatcctagagactttttctggtgatgacaatttattaatagtcactttttgctttactttctctattgaagtagtttttctattttgttctacttttaaggataatataatttataatgctgtttttcacagaaatataagaaaaaagatactaattttataagttaataaagtttgatcatcccaaatccaaaaatctgaaatccaaaatgctccaaattctgaagctttttgagtgctgacattatgttcaaaggaaatgttcattggaaggtttcagattttcggatttagggagctcaacaaataagtataatgcacatatttcaaaacctgaaaaaaatcctaaattcagaatacttctgatcccaaacatttcagataagggttattcaacctgtactgtcagatgatcccaaatgaaaaatattaatcgttaaccaaatatcaaggaattgatcacattttacagtttctgcctaggattatgaatcaagatgaaaaggctctgcatgtttaaaaatatatatttttattttcttataaatcttaaatatctacacttaagatttatttgatatgtgggatccattcatattttggattcaacagttctgtcaaaactgtggcagtgataggggattctttttttcccactgaactatcacaaaattggaaaaagagtaattggagaaccccactggcttagccggcccgaagcccgggagagggcaggcagtgctgtggatggggtcatcccagcgcaacgctgcccctgctacctgcggatctcgctgaggcctgcctttgtcctttgacccttggccatttgttagtgtctctgagagctggactgctgtaccctacttccccagggggcctaacttcacacagcctctgccgcagtgcgtggttggaggtgacggccttggtaaatcgagtttcctacctcctcaattatttgtgctcatacactgtatatttttagtgaggtttatatttgggatgtgttttctccttcttaccctttctggcctttctatggcattaatacctggtctcttcttgtgtacttgaaaatgaatctctcatcatatttttccttagtgtcagaacctccatgactccgagcacttaacgtggctcattgtaaatcacattcaagatctgatcagcctttcccacgagcctccagtacaggacttcatcagtgccgttcatcggaactctgctgccagcggcctgttcatccaggcaattcagtctcgttgtgaaaacctttcaactgtacgtcttcatcctgccgactattgccagttgcagttttccctgccttaaaaatggagtattgaaatttttaactttaatttctgatttgcaaaatagtcatcttttgttcttttccttcttgctgttagccaaccatgctgaagaaaactcttcagtgcttggaggggatccatctcagccagtcgggagctgtgctcacgctgtatgtggacaggcttctgtgcacccctttccgtgtgctggctcgcatggtcgacatccttgcttgtcgccgggtagaaatgcttctggctgcaaatttacaggtattgggaagagaaaccctgatattgatttatattgaaaatttagcaggccaagcaaaacaggtggctggctttttcctccgtaagtatggtcttgacatggtcaccgatagaaacatggaaacatctgcaaacttgccgttactcgtgtgtccgatctgactgtttcttgtatttttttctagtctgcccttactaggatgaactgtacacatcagttcatcctttttaaatgagcatgaggttattttgggttgttaggtgttacaaacacactaatgtgtttttgtctattagagcagcatggcccagttgccaatggaagaactcaacagaatccaggaataccttcagagcagcgggctcgctcagaggtaatgctggaaacacaggtcgtccttgtgttaggacaacccaggatataaaggatatagatttgtacgggaataaattcacaggacaagaaatcgatgtgccttataggtgggtttactgcagaagtgccataatagaaccttcctacttttaaaacaaccagatctcactttctaaagagtaaaggatgaccggcaggatcacgtctgtgacgtgagtggaggcagtttgcactcctggtggctgtttgagaggtagcatttagaatgcctgtattcactgtcctgtgatgagtgggaaaataggttatcaggtttatcttagcaaaatcaaagcatgtcatctaattgctaaacaagagttggcaaatctgagagacattactcaatccttggcatgcaggacttacatctgcatcctgttgccattttatgtcttcaaagcatttaatcatttagttgtgtttgcaaagtctttgagaagcctttgtcagaaatccctacatctcctatgtgagtgtatttccatgactgcagaataagttaaacttttacctttttccttcccttgcggggcggggtggggggcagggattgtgtgtgtgagagggagagagagacagcagagaaggagaatataattatcatgctgtgtactttgagctgaaactgcaaaaaaggaaaaacacacaaaaattattatgcttttcagtctttagagtaccttgtctattatgcttttcagtctttagagtaccttgttgatggtgtttttaaatgggattgggcacaattaggtggacagtttgggatgatttttcagtctgtagggccaagctcttttgtaatttgcattatgaagttgtcactctcatagcagatggcgggagataaactattattactttttgaccctagacttagtcttcagtccagatgagggagattaaaagattataaatatcttgtgccagatgaggtgattttattttgaaatgaccatgaattcctatcagttgtcttactgggatatttgatagtggaatttgtgcatttgagtcttagatgatctgttttacatttattaagaaagcctttattagcttttatactgtgtattgcctgttgcagtgtttgagtataaatgaaatttctggaaaatattaatggagtacaaactgtgatacttaaaagtaaactagggcctgcatttgtatcatgacctgtttgagtattgatgagaagatagctgtgaagaaaaaggtttaaacaagtgtattttcctttaagaagccactaatagtgcatctccttagagtgtatatttctagaatcctagtgtgcagagtttagactaagactaaaaaaaaaaaaaaacaaattatactgtaatttcatttttatttgtattttagacaccaaaggctctattccctgctggacaggtttcgtctctccaccatgcaagactcacttagtccctctcctccagtctcttcccacccgctggacggggatgggcacgtgtcactggaaacagtgagtccggacaaagtaagtgtccagcgtgtctgcatgggaggcacagggcgctgagtgcctctgtcacctgtggcagatacagagagtgcagaggaggtgccgtggacccaaggagttctggcgctcggctcggctcagtgaagctgtggttagagacgtggggggccatcaaggtctgagggagccaagcagtgctgatgtgggacccttttggtaggagtgtggggtgagtagttagtgggtgaatcaaggaatagtcggccgtggcctgcaggcccctgactgcacaggccttcaagcacatgtcaatgccgttagcctccctccatctcctcataccttctggccacctgtgagttgcactgccactgccagccattctggtatgttgtcagcacctccactgctcatacctcatggttagggaccacctggagccttggtagagccttggtagagccttggtactctactttcctggacaaagttcagcttatgaatatgaatttagatttcaaaaaccagcagcccaagtataagaaagcgaaggttcagtcctgccttcttaggctctattcgctaagcacctgccctgccctggttgctggggagagatgagtaaagcagacaacccaggagaggatggcaaaggggccgctaacccttagtggtttagctatatttggaaggcctattggaagttcaccaggtgaagggggaggctgtgagggtgcccaggcaggtaacagaagtccaaaggggaaaacctgtggtgtggtgagccgtatagccacagcctgccggccggcagccctctcagcctagtgcggtgttcccaagcactggcctaggcctgtagctccagggatgtgaagtccccttgaacgccgcccatcatgttccccttatccatttttttcttcccaggactggtacgttcatcttgtcaaatcccagtgttggaccaggtcagattctgcactgctggaaggtgcagagctggtgaatcggattcctgctgaagatatgaatgccttcatgatgaactcggtacggggggagcagtggaggcaaggaatcctcagcttttcttgtgacttccaagtgggatttgtctcatcatcatgtgacccacttgttgacaacacatgttggggactccagtctgggcagggacgggatgtcggagagactccactctgaatggggccgggaagtggggaggactccatttcagatggggtcgggacatgggggttatgctgatcgagacagaaaagcacattgtttcagccacattagaatccacggaggtgttgttttgaaatccagctggccccaaggctgggtgtatggtttgggatgagaactatctggcctccactggaggaacaaacacaggatgttatcatctaagctccatggccaagacagaatggaagtcaaggttgcgtatttgccgtagacttcaacacagtgtcgtaatgcgtgacgtcaataacttgtttctagtgtcttggaagttgatctttagtcgtaaaagagacccttggatgcagcgagatttcctctactcacacctctgttagatgtagtgaggttcttcaccccccaaccccagatgtcagagggcaccctgcgcagagctaggaggccatgcaaagccttggtgtccctgtccctcacccgtgggcaggtcctgtgagcagtgggggggccacctcttgggtatggtgcagccatggcccaagcagggcttcttctcagacctactaggacgggagaaacctcctggtgctttagccctgcgttgatatgcagcaaatgggagggaagtgggcacctgggaggacaaatgcctgtagaggccgggagtgacggcaggtgttcatgaaaagagaccttgtggggagggcaacacaacagtgtgttctgatgtactgaagagctcaactgaaaacaacaggagaattagcccaaaatccatttactaaaattgtttatctttttttttttttttgagacaaagtctcgctgttgtcccccaggctggagtgcaatggcgctatcttggctcactgcaacctccgcctcctgggttcatacgattctcctgcctcagcctcccaaatagctggtattaacaggcatgcaccaccacgcccggctaatttttgtatttttagtagagacgggatttcaccatgttggccaggctggtctcaaactcctgacctcaggtgatccgcccacctcggcctcccaaagtgctgggattataggcctgagccaccacgcccggcctaaaattgtttatcttaagattcatgcagtgaaagctaacttactgagtgataaatttgcttagtgatctgtttattaggttttccaaatttgctaattgggctttgaacagctgtaaaagttctgactgtaaaagaaagcttcaacttttggcattcatgatgcttttctgagtattaaactaagatagatgttttacctgaaggatcggccaccaatctttaaatggctaaacaaaagggttgctaaaacataatccaaattgacataagaaataccatttttccaaccaaaattttggcattcatatggctacttttacgtatttcagctgcatttgaacatctttttcaaactttagggtggttggtgtatcactgaggtcttggatgacactttagctttgattttgtttttatgaattaaaattgtcataccaaaatttttatttcaagcaaatccaagagcataaaaaattaaaatattacttaaaatactaagagagaacagatatatattttactaagcatatgttgaatgaaattgttcaaatatttataacaggcatagagtagaattttcttaaaaatatttttgatggtataccaatttgtattttctcagaaacatttgccttattcttttttctgttgtgtttttcttacctgattgaaagctcataatctgttgttattgtttgttaacctttaatgctctgatttcaggagttcaacctaagcctgctagctccatgcttaagcctagggatgagtgaaatttctggtggccagaagagtgccctttttgaagcagcccgtgaggtgactctggcccgtgtgagcggcaccgtgcagcagctccctgctgtccatcatgtcttccagcccgagctgcctgcagagccggcggcctactggagcaagttgaatgatctgtttggtaattaaaattaaaatttatcttatttttaaaaagcattccagggccagtatagtactttgcaccaagtaaatgtacaataaaggcagtggatctaatacattgaaagcgtttacagaggtagctaaagagcagcacgggtgtcctcggctcagaatttcttcctgtgtgtttgccactttgccattcattgacatggtcatggacatagggctctaagcccttgaggaaggctgggccagacctcaggggagatgcagccccaaaccacgtgcagtcctgtggacggatgtgtagatgtgccactgaggaacaatgtcttgagctttcatcagattctcagagaattgcttgactgcctttcgaagttgatgcatctgtgctcacgtttgcacccacccacgaggtccttctgtttcaggggatgctgcactgtatcagtccctgcccactctggcccgggccctggcacagtacctggtggtggtctccaaactgcccagtcatttgcaccttcctcctgagaaagagaaggacattgtgaaattcgtggtggcaacccttgaggtaagaggcagctcgggagctcagtgttgctgtggggagggggcatggggctgacactgaagagggtaaagcagttttatttgaaaagcaagatctctgaccagtccagtcacttttccatctcagcctggcagtaagtcttgtcaccgtcaagttattgtagccatccttcaccctcacctcgccactcctcatggtggcctgtgaggtcagccaggtccccttctcatctgcacctaccatgttaggtggatcctaattttagagacatgaaaaataatcatctggaagtactttatgtcttaagttggcctggacatgtcagccaaggaatacttacttggtttgtgttagtgcttgtaattcgcccccagaatgtgtacacgttctggatgcattaaagtctggcctgtatccttaaagggccatcgctgtgctgcctgccctcagcaaggacacactttgcagacccacagaggctccgcctccacctcacaccaaagaaagggaggagtccaaagggcatcagtgccattactcacaaaatgataaatacacccttattctgaaccacgtggagtcatatggtttgtgatccctgtccttcaggtttcagcttagtggggaagtgggaaagtcagcgtgtgatcacagcacagggtgattgctgctgattatattatgtgcctgctgtatgcaggatgaaatactttatatgcgtcatcttatttgactctcacaaccccctgtgagataggctctgttactcccatttgacaggtgaggaaagcaaggcttagagaatttcagtgacttgcccaggtcctctgagctaggaagtagccattctggcatttgaacccaaggcctgctatccctagaacccacgctctcaaattcaacctatgacagaggcaagccctggtgctgtgggagccccaaggaagagcctctggcctggtggccacgtagcccaggagagatttctacaggagcccacagcgctgaaggagagagaggcagcagagtaagggggctttgtggcagagaggggactggcactttggggaataggtgggtcaggactgaatgtaatggagccatgtcagagctgtccttctggaagggcaagggcacctggacgcgctgcccctcagtgctttggacggttccacaactgtgattcacacggcttccccaaacgaaggtacacgagtgggcattctgtgactcggtacttccctttaggccctgtcctggcatttgatccatgagcagatcccgctgagtctggatctccaggcagggctggactgctgctgcctggccctgcagctgcctggcctctggagcgtggtctcctccacagagtttgtgacccacgcctgctccctcatctactgtgtgcacttcatcctggaggccggtgagtccccgtccatgaacggtgggttcctatcatagttcctgtctgcttcaccatgtttttattttgtgctgcctgtttgccaggtactaagctaggaattggggatggagaggtagataaaatatgcatcaggaagggctgggccccatctcttactctccaatatattggagtctacactggaatttaactggaatttgcttttttagtcattttatttagattttgaagtttcagctttcatcaaaaatacctctaaactttatgtctctgtgatctttggtcttagctgttttatgtatttagtcttatatgatcataagattaataacattacattcagaagattatttgttttctgtcagagttaaaatgtttgtttttatactgcattgtaatattaacgtactgtaaaataaaagtggcttgttcttttcaaggaacagtatcctcaacaagggtcattagccacaatttttaaaaaattggacgtcatagtttacatgttagagggcgttttgaagctttgtatttttaaattaaatgttatagagtgatgttttcatgtttcataattgttttcatctgtgcatttgtagccaacttgaaaacaaagatccagggattactacttaaaagccagacttcttggaggttatagtgatgattttgatagtatcttgagccgtctcataataacctcagggtgagagatggccaacaggagacagtcgagggacttagaaatctgaatgaaatctgaagttcaaatcttcagacatataccactaaccaagagattggtacctcagtctagtattgtctgtttgtctaaaattggttctaaggaatctaggctagtctgtctatccctttcaacttttgtgaggctgcacaaatgtaaaatgttgaataaaaagcactgatggaagtgtgtagaaattcttctctttgttctgttgtaattttagttgcagtgcagcctggagagcagcttcttagtccagaaagaaggacaaataccccaaaagccatcagcgaggaggaggaggaagtagatccaaacacacagagtaagtctcaggacccatttttttcttacatgttgttcctccaggacttaaaaatcattcacagagacgtgcaccgcggtgagtgtggactcctggaagcgcaccgtagctccgctgtgtcctgctgctcctccctagctgtcagggaggctgtagtccattgctttgccagctcttttgtttccgagtgaacaccttatccgtacacatgcggctgtctctgaccctacagaccagctgggatgccactgggggagcgctcccttccccccgcacttcccacactctgcagttattctgagatccttgagggcagggaacaggtttgtcttctttgtgttctcagaaattaatgctcggcctctggtcagcaagcaacaaccttttgttgagtgataatgaataaataaatgtttcccacatgagtattcagtaacctcagtgtcaggttcagccatctgttttggtggatatttaaaagaaaattccgcttttcctacagaaaaaaaaaaaaatccaaatcccagtgatttaagccagttatagacttagacatatactacggcttttcatgcactttcctcccaattctagagtaggtattttactaggaaaatggtggcagtgcctgttgggaggaagattctttggccaagtgtcttttgttcttgccagggcccctaggctgctggggtgcttcagcttctttagcccagtgtctggtggggaatggcccctgttgcctgtcccacagaggtgggggtgcctcacctggagcctgtccacacattttacacagcacgcttacctggagcatcaggcatcttttccatgctctgtggctcaggaaacacgccttttcaatcatgagtgcaccagtgcttttgggctttttctccccgcttttgtgcaatcctggttgtggatggagttttcctgtctttagtcttctgcatagtacttttctcttctggttcccggttcaaggttttgtaattagagaatgacccagaagcaatggcattttaatgcacagccaaggacttctctgaatttgtatctcaaacctctgtgggtccttcaggcttcagtttgtgatttcatgatttcttgttgctacctaaggaatatgaaaacacccacctccctactctgcatcttccagccgagtggcacctcaggctgtggatcctgtgcttctgtggtgaggataagaatagtgccaaccgtgtggattgaaatcaatcagttaatccctccatgtaaagcacctggaacggatgacagtcttgttatgaatactcaacaaatgctatcatgatttttagttagatttccattgctttaaaacagttgagacatcttggcggtttgagttagagcaacgggccctgaagtgggttctgtttgggtgaagatgattatgcttattccccatggccctctttaggcaagagtgggaagctttctttgtttttttaatcacctcgataggacgttacttcttaaaggtcatccaataaatattaataggccgggcgcggtggctcacgcctgtaatcccagcactttgggaggccgaggcgggcggatcacgaggtcaggagatcgagaccatcccagctaaaacggtgaaaccccgtctctactaaaaatacaaaaaattagccgggcgtagtggcgggcgcctgtagtcccagctacttgggaggctgaggcaggagaatggcgtgaacccgggaggcggagcttgcagtgagccgagatcccgccactgcactccagcctgggcgacagagcaagactccgtctcaaaaaaaaaaaaaaatattaataaagccaactcgttagcgtggggcttaattgcttaagtccaatgagaagtccttctctatcctaggaagttgcccaaactgtagaatctcgtggcctgtgggtaatagccacgtaatacacactcactgcctcaacaaatcatattttagtaggtatgatattctagactcaagacaccattctgtggatcttcccaagggtgtgaagtgtccacagcgtctgccttgggagtttccatgcccaccagaaccatgccccaagcccctcaagcactctgacctaggaaagccagtgaagcaaggatgacaacatggccctttgatactagctgagggacagacacaggtcctgggagaccagagaaagacgaggggcagaggaggtgtcctaaaggaagtctgaggctgaggagccacaggatggcttccagctgtcacaggctgctgctggccttatcacagagagtgggccagagggctgggaaccaaggccagagctcaggttcaggaccattccagcaatcccagcagaaaatggggagaattgtatggtataggcggatatgaaggtagaatctgcaggccttcagtggccaactcagagtctaagtggattccacagttacagcttgagcagctggttgtaggtcatgctttctacactgggcatataggatgtgttttttaaaaagtcctctcttaaccgttgcttgtttagatcctaagtatatcactgcagcctgtgagatggtggcagaaatggtggagtctctgcagtcggtgttggccttgggtcataaaaggaatagcggcgtgccggcgtttctcacgccattgctaaggaacatcatcatcagcctggcccgcctgccccttgtcaacagctacacacgtgtgcccccactggtgagtctgctcgttccttgcagaagaccaagtacggtgaaaggcaccggtaggccctgggctgggcacacgtgagagggcgggacagaatccccgcagcccagaggctgcctgctgtggttctggtgcccactgtggttctggtgccaggctgctttcctcaggcaccacgtgtggaggtcgctagtagaaatactgggttttctaaaatgaactgaggccctacatccctaagagattagtgttagacctgattctagagcaactagaccactttgcttaatagcagaccagaaaccacaccccctcgagtgagtgagattttcctttggagataattcatgtttttctacacagttttgcagttgtcttcagaattggtttaaagtaggtgttattgccaggcgcagtagctcatgcctgtaatcccagcactttgggaagccaaggtgggcggatcacttgaggtcaggatttcgagaccagcctggccaacatggtgaaaccccatctctactaaaaatataaaaattagccaggtgtggtggtgtacgcctgtaatcccagctactcaggagactgagacaggagaatcgcttgaacccaggaggcgaaggttgcagtaagccgagatcgcgccactgcactctagcctgggcaacagagcaagactccgtctcaaaaaaaaaaaaggtaggtgttattgatcagaacccttgtttcagataacatgaggagcttagcttgaggagagtgagggttgatggagggggactgacttctgcccagtgaaatggcatcatctcccaccagcccgctgaaataagatgatggggcctgttccttagggcctgcagcatcctcaggcaggaaagaaaggccgacctggcagggtgtgagccagcaggtgtaggtcagggagaatggagccaggtcccagggaagaggcttgtggctgcctgagaagggtgcgtgcctgcctgtgtgtgtgtgtgcacgtgtgtgtatgtatgctggagagtctagggaggcttgctccaaggacgcagtattgtttgatcctgagagataaggattctgccgcagggaatgaaggtattccagatggcgggcttattccgaagaagaggccagtgcctggcggtgctggaagcagttgcagaacagggagttgtaggctttcctgggaagagagcagcaggggtgctggagaagcaggccacacttgctgcatggggttgctctcggccccactcttggtgcacagcgagtcactgtgggttcattagcatctggttatgagacagtaactgctcctttggaggggctcgtggagaccatgcaggagggcacggtcttgaggtcatgccgtccagagcacacctgaggataggccaggacgggctgcacgctgtaggtaaaattcctccagcaagctcttcactggcattgaggagttccctgagtgcggtcatctggaaggcagctgtaacaggcactgcagtctctccctgggtgggtaccagagaggagcataggggagcataaccgatttaaagagagggctttcctgtggtgaggtaagagattagctggtcattatcatagagccccctctgcctttgtgcagatgggctgtgggaatcctggggttccgttgggtcctttgtcacctcactgaaggcatgtaagctgagctggccagaccgtgagctgatcctgccacttgaacagcatcaagcctgcctctggattcttctgtgcatggcacttgtctgagcacctcacgcacagagaactggacttcagagtttacagaaataagctgtatggttcattttcatgcctgcttgccaataaacatatctgagctgaacctcattgaacgcctgcctttattctagcacagcacctgctgtttgtgggcgaggggtgctgtctctaactcctgcctgcttctcccagcactccctgagtggggtgtgccagcagcctcaggatgaggacaggaagtgggagggcagagcagatttgggagggccacttgatggggaaggaagtcccaggaagcagttggagctgttttctgggggagaaggtgccagctctgggacagtgttggggtagtgaggagggagcccagtggagagaagtcgggcttcctgcttcctcacagtatgtctgtcctgactcaactcggatgatgtcacttccttttcatcttctcaggtgtggaagcttggatggtcacccaaaccgggaggggattttggcacagcattccctgagatccccgtggagttcctccaggaaaaggaagtctttaaggagttcatctaccgcatcaacacactaggtactcttggggcctctccttcaggtcaccattgtcggacatctaccgggaggaaatccagagcccccagtactgggatcttctcatttgactccagaaaagatttaagcatgataataatacaaacctatgtgaatacattttgcagtgttggcaaaactccttttatactgagaaaatagatcccagttcctgtgttttgtggcttgaatcccagctttgtgtattccgggcttgtttgaagtcaggaaaggttcatgtgtagtggacaacgtgagaccaaattctgccttagattttgcatttaggctaaacagtggcagcacttgtctcagaatgttttcttgtgttcaccagtctgatcctgttgtgtctcagtggtccattttctcatatgggaacaagcagacgggagcagatggagtcaggtttcttggcactcgccttccccagagcctagaggcagcatggggagaaagcaggcttggggctcagacagtcctggtctgcttccagccctcctacctgagcagcgcagggcaagtccgtctaacctctagagaccctcagttttgtcatatgtaaaatgggggtcgtgtctatttcatagaattgttgcagatttagaaattacatttctaaacaaatgttaccccttatttctaaataagtgtctaaatgaataagtcaccacttttgcccctatttgatggcaagaggtgtgatcttgtggtgggactgtaatcagtcagttctcagtgactgtgccctgctgtggtgtttcctggaatgttcctgtcttgtcctagaaagtctggcaggggcaccctgactccactgtccagtcctctccccagtccctcgggcttctgcagatttgaggcttgtttggatcccagaaggttgtggcaggagacaccttgcctctactttcccctttataattcaatgtccaaagagagccctgagcaggtacctcacgccagctgcctcacggagctcctcctcttcctggctgtgaggatcggtatcagtggcctcctgctctctcccccttgcctaacacgagcacctttgcttacttgggtgcccttgctcttgaactgcccatcggacgtgcgtgacccaagactgtgccgcagtccttgccttgtctgtgctcattttctttgttcatttttttccctgtaacgtaaattgttatatttgtctgtatctgtgtctgaatcagtcctgcacgctctccttctctctgtctcttgttctttctttaccccgtttatcacggggaccccgatgtccattgctctagttctcctgtcctaagcaccccatcccgtctctctggccttaccacaagtggcgtggctgcctcagacatcatgatggggacatgaagcacagctgtcagaaacaactgttcgttagatacactcgaatgcagctcatcaatagggatggagggtctgtcggatgtattttcactgaatccccgttcctaccttgatacactctttttaatctattcttctagacaggtcagaggaaccattactttgacttttaaatttttagcagctttattgaggtagaattcacatactacagatttcacccactctaagcggacagcttggtggccattagttttatccacagagttgtgcagccagctgcacagtctcagggctggactccagggaagattttagcccatttagtgagtggggcagaagtggccctggccctgcacgaggttgcctgcatgggcgtccctgccctgtccctgtgtctgctccactgggggttgaccaggctgccagggccgacttgggcctgtgccacctgcctctcatgtgtctcggacagtgcagccgatgtctatacttcggtttcctcaatgatgaaatggaggggatagtgttccccgcatcatagaactgtgtgaggtttaagggactcactgcccttggcgtggagccttctccaggggccgtgctgtgtcggcgtagctgtcagctctccgttacaggcttgagaagggttgacactctctcatgtaacatttatatttctaggctggaccagtcgtactcagtttgaagaaacttgggccaccctccttggtgtcctggtgacgcagcccctcgtgatggagcaggaggagagcccaccagaagtaaggccacaccctgtgctggttggcacatgggcagttatggccgcttgcaggcctttggtggggaataaaataaggcagcaagctggtgttctttttttctcttaccttatttttgaaagagtagctgaatggtgtcttgactgatattccagagcagggacaaagcctgctgaggtctgggggctgcgattaccaatggctggaatgcattttattacggtgcattccatgttaaggatcaatacgattgtgccctttctggaaaatatcttttagtttatcaatattcagaggagtgtaggttgaattaaaatgaaaaggcactttataaaggccatgagtagtacctggtttcatttttctaatgtcttgcagagattttatcaggcttcttgaagtgttcacgtacattacgctaacacgatattaataataactgtgctctggtacagcggagccagcagaatgggaagttgtggaatgcaggcccttgattctgatagaaggtgtggtttgaactcacagaaatgacagtttggagggtagacatatgtcacaagtcatcaagattgtctttaaattcatgcatagaagctaacagggtgtcataagcaaggcctgtaaaatgtatgagggaattcaaagataatttattaaaaagtaattcatgtttggagttttgtgcccaaaggagtccttgatttgaaaaatgggcttttgcccatcagattgtttcagggcccgtgtgtgcggaggccctgccttgtgccccgtgagctcagcctgacagaaatcctttggtagcacttaaggctcctcttcctcccattgaggcagggaagactctgggttctgcaggcagaggtggttgtgggtgtcttgctgctcttgttgacatgtgggctctccttccaggaagacacagagaggacccagatcaacgtcctggccgtgcaggccatcacctcactggtgctcagtgcaatgactgtgcctgtggccggcaacccagctgtaagctgcttggagcagcagccccggaacaagcctctgaaagctctcgacaccaggtttgcttgagttcccacgtgtctctgggacatagcaggtgctggggacagtgggttccccgctgaagcgtccagcagcttcaaccaggccgttttccttcattgctagaattgaaaacaccgtccgtgtggcctgtgcaggagatgcagacccaaaggtggcctcctggtcagtgagaagctggaaacgtgacaggaactgacgtggggttattgagcatttaggggaagacgttagcagagcaggaatgagcaggcaactagtagaacacccacttaagggctcacggacaggtgctcacttaggaagtgagtttcatttggtattacaccaggttcctttaggcaaagcggagggaaagttctggtgtttttcacttgtaagattttgaaggaaacaaaacactctttaccttttttctaaaatgtaggtttgggaggaagctgagcattatcagagggattgtggagcaagagattcaagcaatggtttcaaagagagagaatattgccacccatcatttatatcaggcatgggatcctgtcccttctctgtctccggctactacaggtacctgagggaaagggtgcgggggagcggttgtacttgggctagaatgagagaagactggcatgctcaccacaccagtgatgcgggaagacctgagtgtggtctgagttggaggctgtggtgctaaatacgctgcccctttcataagcaggagtcttagtcaggcccagggaggaagtaaaatctggaaatgaatgagaagcattctctcctgccagtcaagaaatgagaagcgaaagaattctcacgggctgtaagaccagcaggatttaaaagttgaattagttgcttatgttaagaactcaaccaagttcatctacacaagctgaatctccagcttttcctaagaaaccatgtgtggcagtggctgcagggcagggcacagctgggcctgagcaccccgctccctgcacctctcccctccctgggccctgcctgtcactgcccactctcccaccaagccttccggttgtgtgcctgccctatcacaggcatcggagcttgtcacctggtttaaaagaagagagttgtgtggggatttgggatgcacgtttttcactcaaaagtattttagcgtagagctctgtgattccgtagctatttaggagtttaagcaccttgaaggctttaattgcagaaagttctatgtggacgtgcaatgtgttatacgcagtgtctatgagactcaaatgtttattagggcgttgaagtaaactgagcacttggagggccatggatccagccttcaaggagctcataagtcaggaggacccaggagcaatgacctgtcatagaaggcagaaaagaggggcacagaggtgggtgggaggcatacacaggcagctcctggagctccaaggggagcaagtgcttccagggaagggggcgtggaggcccctttggaggaggcaagttgatctggggtctggcagagggttagctggggacatttagcgggaggctggtgcccgggaattggggggatgcccagcagaaagacatgaggaggctggcctggggcgtgggggggtgtgaaaggttaagtgggggcattatcctgctcccgctcctgccggctgtatctggtcagcctgggcaccgaggtggggttctggaaggcactgttcaccaaaatgcttatctgggtcccccagagagcttgcctgcctggactgtcggctcgcctgcaactgctgactcctaagcttttgcagctcagcccacaaccagttcctattcacagaggtgggagctgaggggtgacaagtgactgctgcagtcttatttgtcatagagaaaaagtgacagagtccagcttgcccactggccctgccagcttaactggttataaagtgacaaatccccaagacccacagggctctgcacaacctgggccctcctgccagtggcggcgagggcaggtggctcacggctgggtgcctgtctgggcaggagctgggctggtatggggtgggcctgcggccctgcccccctgtgcagatcaagactcagggtgctggtgttcacaggtgccctcatcagccacgagaagctgctgctacagatcaaccccgagcgggagctggggagcatgagctacaaactcggccaggtcagtctcgcgcccccgccgcctggcctctgtccgtttctgtcctcagactttggcgcttgacacacccaggagaaaagctcagtgcactttttaaatgaaaggaagttttccttttttttaaaaaaaaatttaatgttcattgtttttatctgttttattcctaggtcccgcaagcagaggaagcattagttttgtttttatttatgttctgtattccagaaagtagttaagagacctcacatgtagcgatagagatgtgtgtaagagacagtgagagggcgtgacttggacttaagcaaggaccgtgagacacaaaaaggggggtgaggacagagtggagtcagctgaaatgctcaggaggaagtagacgccatgaagggccatggtatggggggccgcaggcgtggccgtgagtgtccctggggccagctcttggggggctccctgagtgtccctgtccctgtggccagttctgggtgggagccccgtgtgcaggcagacagctcggccacttcctagcaggtcacattggtctgtgcttctgtttcctcctcagataagtgaagggattcaagggtctgggtgtggtggctaacacctgtaatctataacattttaggaggctgaggcaggaggcttacctgagctcaggaggttgaggctgcagtgagccatgattgcaccactgcactccagcctgggcaacagaccagtactctgtcccttaaaaaaaaatgtaaacagaaacgtagggccatttgcatatgatggcacatggcgtggagccctacaggtgtatgctgggcggggcccggctgtgctggccgacttgcacctttccctccaccccggtgctgtgtctttcgctcaccgggttcctgatttagtgaaagcagttgtgcaggacagttctctttgtagcttttgtttctgtggaaatgggtcagaatatggtgtttagaaacacttatgagctctgagagtttcctcttctgagttcctggcctgcagccttcacagcagaaaccctgtgatgtcacaagcctgtttctgttccctgctctctgcctgtactgtcctgttttgtgcctgccggtttcagtgacaggaagcagggagctactggaccagcctgtatttttctagacatagttggaaaaagaagtcccactcttctgtcctttcacctttgacagatgtttccaccccaagataagtgaaaatgaccaataggatgcactgtatttttcatgaaagtgtttctgaagggcaggctgagagtgagaggcctggggctcactgggtgcctctggccttgtcctgggcccagggacactggtctgtgcccgaggtattccctatccccccaaccccgctgcatttggccacatccttcaatgtttgcgttgtgtccagcgtccgcaaaccaactgtcatgggatcatactggggctgaagtacggtcccacccctgccctgtctggggctgaagtacagtgccacccctgccctgtctggggctgaaggacagtgccacccctgccctgtctggggctgaagtacagtgccacccctgccctgtctggggctgaaggacagtgccaccccttccctgtctggggctgaaggacagtgccacccctgccctgtctggggctgaaggacagtgccacccctgccctgtctggggctgaaggacagtgccacccctgccctgtctggggctgaaggacagtgccacccctgccctgtctggggctgaaggacagtgccacccctgccctgtctggggctgaaggacagtgccacccctgccctgtctggggctgaaggacagtgccacccctgccctgtctggggctgaaggacagtgccacccctgccctgtctggggctgaaggacagtgccacccctgccctgtctggggctgaaggacagtgccacccctgccctgtctggggctgaaggacagtgccacccctgccctgtctggggctgaaggacagtgccacccctgccctgtctggggctgaaggacagtgccacccctgccctgtctggggctgaaggacagtgccacccctgccctgtctgggatgtttagcccctagatgccactggactgagccgctacttgcttttgggaaagaggggtgggggttaggggtctgggcgaggggagtgcaggggctcctccttggcctgagagctgttcatacagactcctcgcccactccctgcagggtgctgggtcccaggggggaaatggcccttggtgccaagaacgtgagttggggctagtgccagtgatgatggagaacagctttttatgggcacacagcccacagcactgtgccaagtgctcgaggcttcccgagaaccaggcagaaaggaggacagtcgaggtgtgctgactgcgtggtggctgcgtgatctagagcgcgggtcacaaaggcgcgagggagctctggccttgggtttaccgcaatgactgccagtgcgggagactggaaaaggaatctcacgtattggttccgtgttttggggactccattcagatgtcacttaggagtgaaagcatcccttcgtagagcctctttctgtgtcaccctcctcagctgctcctggggttgactggcccctgattcatgcctttagcatgtgctggagcttcccagcagctgtccagcccctgccccaccctctctgtgggctcccttgcccgtaacctggggtgtctgaacgacccttgctaaggggcagactgttagacggtaggcatgtgctgagtcccagtggccacacccacccaccaggagcctggcactgtggccgcagcactgagcagtgccccgtttctgtggcaggtgtccatacactccgtgtggctggggaacagcatcacacccctgagggaggaggaatgggacgaggaagaggaggaggaggccgacgcccctgcaccttcgtcaccacccacgtctccagtcaactccaggttttccaatggcctttttctttttaacagaaatttgaaatttcttatcagtcatttgatttgtttgaggtgcttcttgaaatgagcctctcatctcatgtacttggaaaatacccatctcgcatattccacaggaaacaccgggctggagttgacatccactcctgttcgcagtttttgcttgagttgtacagccgctggatcctgccgtccagctcagccaggaggaccccggccatcctgatcagtgaggtggtcagatccgtaagtgagccttcccattcccctcacacctgcacgtgccacacgcaccacacacgccacacaccccacacacacacaccgcccacacacatgccacttgcacacacacccctcatgcatgcaacacacacacaggccacacgcaccatagacaccacacacacatgccacatgcacacacatacacggcatgcaccatacacacaacacacacagcacacatgccacacacacacgccacaccacatgcaccacacacatgccacatgcacacacactccacatgcatgcaccacacacacacacacacaccacacacaccacatgcaccacaccacacaggttacatgcacacaacacacacatgccacgtgcacacaccccacacaccacatgtatgtgccacacacagcacacaaccacacacatgcaccacacacatgccacatgtgcatgcaccagacacatggcacacactacacacacgccacgtgcacacaccccacacacatgtacgcaccacacacatgccacacacacatgcaccacacacatgccacatgtacacacatgtatatacacaccccacaccacacacacaccacttgcacaccacgcacacacaccacatgcgcacacacacaccacatacgccacatgtacacaccatacacacaccatacatgcaccacgtgtaccacgcacccacacagacacagcacacgcatacaccacacacacacgcacacatgcgtcccgcacagtaatgtctcttgggtgtaagaacacgacttgccagtagtagcgttctggatgcgttgcctggattctaacagcgcgattctccccttgccctcctggttttccacatctccagcttctagtggtctcagacttgttcaccgagcgcaaccagtttgagctgatgtatgtgacgctgacagaactgcgaagggtgcacccttcagaagacgagatcctcgctcagtacctggtgcctgccacctgcaaggcagctgccgtccttgggatggtaagtgacaggtggcacagaggtttctgtgctgaagccacgggggcccatctgccttgggacctggtgttggccagaggtgccgggtgcggctgcctccttccaagagttgacccgaaccggactccacggcccacgtgagctgcagtgcttctcagatggagggggttcagcgacggtcagtgccattcacaggtcactgtgatgtgggttgtggcggccaagccatggtttggggtcccgtatccctgggcttatgacatcattgtagtagcccatccccacagaaccacggtgtgtggtggcgctgaggcatcgtagatggtggaaatgctactggcttccccatgctctgccctgaggcctgactgcctcactccccttctcagttatgttccaggccccccgagcttcctggctggacagcttctctcctgggggccgttttgtcacagtgaccctgtgtttctagtcccaaatctgggtgctatagtctctttttagcgtggtggttgtcttagtcttttttggctgctaccacaagttaccttagactgggtaatttataaacagtggaaatttacttctcaccgttctgggggctggaagttttcatggtcaaggtgccagcagatttggtgtgtgatgagggctgctctctgcttcatagatggcatcttctggctgggtcctcacggtggaaggagtgaacaagctccctcaggccttttagaagggccccaatccacaagggctctcccatcatgacctcatcacctcccaaggccccaccttcttgtactgtggcactgcaaattaggtgtcagtgtaggagtttcaggagggatagaaacattcagaccatcccagcggtcaagtgttcatcctcttgagttcctccttattctgcttctggtttatcaggattcagccagtgcagcatggtacctgtattctgtggcacatcaccacatggtatttgccaagtatccatcacctgcacacgtgaaatcattgcccgtgggtcccgacatctggcgaagcatattcaaggatggcagaactgtcagagctggcacctctggttccttgtcatgtggcattacctagtaatccattttatgatagcaatggaaactcatttcttcaacaaacacctgagtggctgccgtgtgccagccgtctggggcccttggtgagaatggcatggtggtgcccatcagggcctgcctagcccgtgctctggacgggctcctgtgtgtcaggaacgacaatgctgtcatgacggtgaatgatttttttttttgccatcactccagccgctaacatttgcggagctcttcctcccgcacccccacctgacaaggccaagggtgaccttggccccaccctaggcggccaaggtcagaggttagctggcttgtctgggtcacacaaaatgcagcagaggttgaggtgagcacatgtccgtgacctggagcctgactccctctctgcgagtcttgactgctcttgcctagactctgtcctccccgagcccaaacgccagtcatcttcccttgtgggtgtccttcagcctggtgccatgctggtgactcagcagccgtccagggagtggaaacaattgagtgtgtgggttccctgtgtgggcatctctcttcacggcgaacaccctctgggtgttgcccacacgatgtcaaagcggctcttggaaggggtccttctcctttgtgggaagtttcagctgctgggctaacttgaattgtaactgtggttttgtgctcaggcccagatccccctaggcaagtgttgtgccatcagtaatcaaatgagaaataatcattttgaaaagcagatcctaaggcaggatggtcatggacactcactcccagctctttgtgcactcatgctttctggaagatggccatcctctgtgaaggttttcagcgcgtcatgcttggtacccacgtatccagagcatgtcgttttgaggtatttgcccaccgttgtgaaatccgtgccacccgagagcaggtcctgatgtggggctttcagaagtgggacctggggccgtacgcagtccttagggaggggccgtgtggcgttgtgcgtgtgaggggatagcacagggtgaggtgggggcccaagaaggaagtgacccacaaagaacagcctcctcttttggtccttgttcctgggatggctgggagtggcttctgtgtcgtccggccatttcccctgcggagaggctcctaccactgccgagaacctcatcattccacaaaaacaagaggccgcctggccatccagcgctccatgggaattctgtgtccccatagtcttgggctgaaggagggtgacattccttgctgacttctgcaggggtctcctcactgttaaagagcagattgaaagtgaagaacgtgggctaagtgtttaggtcgatatttaaccctgctaggttttggatactaagtgaaattgaggccattttggttgaagttgacagaaaccactatcagggatccccaagactaccccaggcttttctagaaagactctcagctaagatgtgttatggtaaaagcacacaaaacaaaatcagcaaagaaaattagcaagggcagaggcccatggggcgatgtcccgaggacaccaggcttgagcttccagaatcctctcccagcggggtcgtgcaggacgcacttaactccccgcacagtgagccgtgacagcgcgtgtgcagtgtcgtcgccaggaaagcacactagagactcggtgccagggtttttactgggggctgggcacatgggcaccctctgcctgcctcgtgcccagactctggactcccggagggaaggcaagttctcagcaccaaccctggtgcccacacaagcagctgagcacagggagcccctcctcagtgaggatggtgggcaccgtcccaacaccagccaggggccagccttgcacacaggcctctcaggatggtctccggcctgctgtgtagtctcttctgcacacaagcgtgagggcagcgcccccgcctcggctgtggggaggagccactgggacgtgagctctggtggcatgcagcagcttttgtctgtgtgtgcctaggacaaggccgtggcggagcctgtcagccgcctgctggagagcacgctcaggagcagccacctgcccagcagggttggagccctgcacggcgtcctctatgtgctggagtgcgacctgctggacgacactgccaagcagctcatcccggtcatcagcgactatctcctctccaacctgaaagggatcgcccagtgagtgggagcctggctggggctggggcgggggtctcagaatgagctgtgaaggaagcagcatcaccctctccaagtgcccaggctcctggccagatggcaggccaggtatcagtgggaacccaggtgggtgccatggctgaggtcagtgagacgcaagagcacaggtgcgtcctagaggcttcctcgggcacctccagcgagctggagctctcgcctctgctgctgtctcatgtggcgcttagcacactctcccacgtgcccattcctgactctgctctcgaggccatcggctctcattctctgctcccagaaccctgttattacccaggctagcctcctctctgcaccttccccgccctggcccagtacctccctcttgtttccactgtgattccgacctcaccttatcttaaagctgctggacggcaggttctgtacacacgtgtccttgacaaagcacggctggtgccgcaacccctcagcgagcaagtcaagctcttcacagcgatgtcttacaagcgcagagggctctgtgacaccctggtctcaccgccactcttccaaagtcgcagaggctttagcagagatgggcccagcctctctgagtcataggcttctgcacacgggagctgtctttagagggagggtggaatttcatcagccacccacatgggggagttgagggcaagaattaggagcaaagatgggaaggggtctgggaggaatggccagtgatcccctttgacaagtgggcaggaaacgggggctaggtcaaagttgagtggaagacctggagggagacgggaaggtctctgtaggcacagttcagacaggagggaggtgtgagccagggcacatgccggtggccgtctggcaggatttgggacatgctggagcagggacagcggctcatcaggggccattgccctcatccaggccagagtgtcacaagcccgtggggaggcccttctcgcctgtcatccttgctgggcagtgggtgctgtgctagcaggacaggcggacggctggcaactgtctctgcatccctggagcctggcatagggccaagtcacacggggcacaggcctgcaaatcaggcacatatgttggtgcagtgacgtgattttggggggcagccccagaacaggccccagacacaggccaaagccctgcctgtgctggtgtgttgggctgttctatggctcttgctgtgggcatggaggactcagggaaggagagttgaggtggtccaggagttgcgtttgggatgcagagagcttgtggcatccaggtagaaatggtgcgtggggctgacctcagcaccatgggcagaggggccgtgtcacgtgcctccgaggtggaggtgggaccacgtggtgacagatatacgcatcactgggcacgtttttgtgggtgttggggggcatcgtattggctcctctgttcacagtggccactcattcagtccctggctaccaggtcctcactgtgccatggggaaggccggcgctgtcgggggatcacagaaggcagcacgtcatgatggcatgtgccatgaaggaaaagcacagggcactcaggaagtagaggggactggcctggggtgtgggaatctagggcctcgttgagggacagagagaggaagtgtgtggtggccagcatggaggtggccacaggggaggctgagttaggccgagagggcagggcgttggggaggtagacgggctcagccactcagggagtggtcaagcagaggctgaagggtcaggccaggttgcaggggcctgggggagccactcagggtaggcgctcccgggagcccgcctggcccatagctctacactcccgcgtggggccggacatgctgtgaagccctctccacgttggatgggggtggctgagcctggatgctgtctcccgttttcagctgcgtgaacattcacagccagcagcacgtactggtcatgtgtgccactgcgttttacctcattgagaactatcctctggacgtagggccggaattttcagcatcaataatacaggtgagtgggccctggctgtcttcctctgcacacggggagtgggcttcccttctcttttccttgcaggatcataccagtgggccagttttgacttggtcgggaggaggcatgaacacctgagactgtgcagcgattctttgacacagaggcctttctccctgtgcagatgtgtggggtgatgctgtctggaagtgaggagtccaccccctccatcatttaccactgtgccctcagaggcctggagcgcctcctgctctctgagcagctctcccgcctggatgcagaatcgctggtcaagctgagtgtggacagagtgaacgtgcacagcccgcaccgggccatggcggctctgggcctgatgctcacctgcatgtacacaggtgagcatgtacacggtgcccataaggccagcccaagtcctgttcaagggaggcaggagcatgctcactcaagggacctcgactaggtgccctctgatttcacacttctggtgttgccccaagccggccccatcaccttgcaagaaaggctctggagcccccagggctggagtacctggtcagggttgaccgtccctgtggtcactcatcccatgtggctgagctgggctgggtcctgggcaagcaaggggctgatatcacctgctttcagatctccagggactcactggacccctgtgtacaaagcactgtctacagagcctattgggttgtatagaggtaaccttcgtactgaacacttttgttacaggaaaggagaaagtcagtccgggtagaacttcagaccctaatcctgcagcccccgacagcgagtcagtgattgttgctatggagcgggtatctgttctttttgataggtaagaagcgaagccccatccctcagccgttagcttccctagaactttggcctgaagctgtgcttttgtgtgtgtctgctgatcccctggcgctgttgctggagtcctgccagtgattccccaccacagcctgaccatgggctgccttggctcagggttccactggcgagctggtggtccttggaccccagcactcaggtgtagcgttgaccagttccaaggttgtcccagtgcctgcccatctctcctgagggctcagggacagtacctggcagttgggggtgtggcagggggcaggaatgaccagcctctgggagggtggggcagaagcctgtacagtgaggaggagctggctcagcctggctgcctatcgtgagaggggagcccacggggctgtgggaggggggccgtggtgcctgtgagcagggtgaggagcagcggcaggaggatgaaggtggaacccacacatgcatctttgagacccgtgtggtcagtggcttctgccccccaccaccccccactgctgtgcgtgcatagaattggcttccctcacctgctctggaagtgggttaggagcttggtagggctttttctcaaggacaagggcccctgatttgctctcaggcctcagtcctggcgacatggtggatctggagccttgttgcactgccttgcctgtgctctccaatcagggtggccagtggggagccatttggcttttctcaagagcatactcaggtggaccttgctccactgtttgaccagatgaggcattctgaacagccaagcctgtgctggtctgttttcatgttgatttttttttttcttttctttttgagatggagtttttcccttgtcacccaggctggagtgcaatggtgtgatctcggctcactgcaacctccgcctcccgggttcaagtgattctcctgcctcagcctccctagtagctgggattacaggcacacaccaccatgcccagctaatttttgtgtttttagtagagacggggtttcaccgtgttggctgggctggtctcgaactcctgaactcaagtgatccaccctccttggcctcccaaagtgctgggattgcaggcgtgagccactgcgcccggcccccatgtcgatttttaaatgcacctctgcatcgttcttcagtccccatatgctcactgagcaccactgcgactggcagacgggcacagggaggcgccacgaccagtcctggccttcaaggggcttgtggtctagtgggcccaatgctaggtggcgagtgctccaaagagtgtggtgcacgccttccgcttgaccgctctccagacgccacagggaggcacctcgcagctgaccacagatttctctctgtggagcagtgtcttcagagcggctgccatgccactgctgggcgagggtctgcgggcgggtagagccaggagcacctgtgaggaagtgcactgccattttcgtagctgcttcccgtgtgtctcagttacacacggctggcatgtgtgcactgatgagacgggaacgtgatggttgcttttcagcactgaaagggatactgctcagggggcgtgtttcaggatctggttagggaagaagcagcgagagcacagatggggccctgtgtggtaacaagaaaaaagtcctggttgacaacagtgccacgaagcgttagaacacatagggatgtttgtggagcatttgcatgtggaaagcagcaaaaacataatgggaacgggttcttttgttatgatttttaaaaatctcttttgtaacatccttcccgctgcgccgtttctgcatattcctttatgtagctttcaaactcctcttaggagttctggtccctacagggcgtgggagcccaggctttacgtagctttcaaactcctcttaggagttctggtccctacagggtgtgggagcccagggcctgtgccgagcagcctgcctccacgagctagacagaggaagggctggggttttgcctttttagtctcaaaattcgtactccagttgcttaggctctgactttccccacttggaaagtccctcacggccgagggtccctcccagccctgatttcacatcggcattttccccagtattagagccaaggccctccgcgggcaggtggggcagctgtgggagctggtgccagtctctgacctgcgtccctcctcccaggatcaggaaaggctttccttgtgaagccagagtggtggccaggatcctgccccagtttctagacgacttcttcccaccccaggacatcatgaacaaagtcatcggagagtttctgtccaaccagcagccatacccccagttcatggccaccgtggtgtataaggtgaggttgcatgtgggatggggatggagtgggaaagcctggaggtggagttgcctccgacttcccagcagattcgccagcagagcccagctcctccgctttaaagcagcaatgcctctggcccccaccccacccccgccacccaggcgcagcaggtgcttcccgtccccccagccctgacactcaggcacctgcttgctccttgcaggtgtttcagactctgcacagcaccgggcagtcgtccatggtccgggactgggtcatgctgtccctctccaacttcacgcagagggccccggtcgccatggccacgtggagcctctcctgcttctttgtcagcgcgtccaccagcccgtgggtcgcggcgatgtatcctctctgggtccctggtgctggccccgtttcccttgtcaacaccgaggctcatgtttcatgataaggttttgaaacctaacctttgcaaaaaccccacagatgccagggtgacaggccctcagccccagggaagtaaaatgctgacaggggtacagaaaggagcacgtccagacatttgctgaccagggcctctcagaggggccggtgtatggcaggagggtcgcagctgaggggcctttctgtggagggcctgggtgaggggagcgagggtgggcggtggtctctgcagacgtcccgcccactcgcgggctctgtgtggctgggcttctcctgacactgcttctcattagctttggtcattgtgcctcgatcgccctctcggggaaaggcttaagtaaagatccagttcccacccccagatgctggctgccaggagtttccctttccacagcccttccccaagacagaccacaagagcctccaagcagcacagttgtcctggtgctgacagcacagccttgcccggcgtgcctggcacggctctgccctcactgcattggagcagggctagtggaggccagcggaagcaccggccaccagcgctgcacaggagccaggccaggtgagtgctgccgagtgggtgccctgcctgcagggcatccagccagccaagggttgcaggaatggaggtggaggcgctgatgcagctggaggcatccaggtggcccttccggggctctgctcgctctccaggctccctggacccctttgtagactgtttcaggagaggaactcccaggtgaggacagggaggcagcattcccctcatttgccggcctttttccttaactcctgcaccagcctcccacatgtcatcagcaggatgggcaagctggagcaggtggacgtgaaccttttctgcctggtcgccacagacttctacagacaccagatagaggaggagctcgaccgcagggccttccagtctgtgcttgaggtggttgcagccccaggaagcccatatcaccggctgctgacttgtttacgaaatgtccacaaggtcaccacctgctgagcgccatggtgggagagactgtgaggcggcagctggggccggagcctttggaagtctgcgcccttgtgccctgcctccaccgagccagcttggtccctatgggcttccgcacatgccgcgggcggccaggcaacgtgcgtgtctctgccatgtggcagaagtgctctttgtggcagtggccaggcagggagtgtctgcagtcctggtggggctgagcctgaggccttccagaaagcaggagcagctgtgctgcaccccatgtgggtgaccaggtcctttctcctgatagtcacctgctggttgttgccaggttgcagctgctcttgcatctgggccagaagtcctccctcctgcaggctggctgttggcccctctgctgtcctgcagtagaaggtgccgtgagcaggctttgggaacactggcctgggtctccctggtggggtgtgcatgccacgccccgtgtctggatgcacagatgccatggcctgtgctgggccagtggctgggggtgctagacacccggcaccattctcccttctctcttttcttctcaggatttaaaatttaattatatcagtaaagagattaattttaacgtaactctttctatgcccgtgtaaagtatgtgaatcgcaaggcctgtgctgcatgcgacagcgtccggggtggtggacagggcccccggccacgctccctctcctgtagccactggcatagccctcctgagcacccgctgacatttccgttgtacatgttcctgtttatgcattcacaaggtgactgggatgtagagaggcgttagtgggcaggtggccacagcaggactgaggacaggcccccattatcctaggggtgcgctcacctgcagcccctcctcctcgggcacagacgactgtcgttctccacccaccagtcagggacagcagcctccctgtcactcagctgagaaggccagccctccctggctgtgagcagcctccactgtgtccagagacatgggcctcccactcctgttccttgctagccctggggtggcgtctgcctaggagctggctggcaggtgttgggacctgctgctccatggatgcatgccctaagagtgtcactgagctgtgttttgtctgagcctctctcggtcaacagcaaagcttggtgtcttggcactgttagtgacagagcccagcatcccttctgcccccgttccagctgacatcttgcacggtgaccccttttagtcaggagagtgcagatctgtgctcatcggagactgccccacggccctgtcagagccgccactcctatccccaggccaggtccctggaccagcctcctgtttgcaggcccagaggagccaagtcattaaaatggaagtggattctggatggccgggctgctgctgatgtaggagctggatttgggagctctgcttgccgactggctgtgagacgaggcaggggctctgcttcctcagccctagaggcgagccaggcaaggttggcgactgtcatgtggcttggtttggtcatgcccgtcgatgttttgggtattgaatgtggtaagtggaggaaatgttggaactctgtgcaggtgctgccttgagacccccaagcttccacctgtccctctcctatgtggcagctggggagcagctgagatgtggacttgtatgctgcccacatacgtgagggggagctgaaagggagcccctcctctgagcagcctctgccaggcctgtatgaggcttttcccaccagctcccaacagaggcctcccccagccaggaccacctcgtcctcgtggcggggcagcaggagcggtagaaaggggtccgatgtttgaggaggcccttaagggaagctactgaattataacacgtaagaaaatcaccattccgtattggttgggggctcctgtttctcatcctagctttttcctggaaagcccgctagaaggtttgggaacgaggggaaagttctcagaactgttggctgctccccacccgcctcccgcctcccccgcaggttatgtcagcagctctgagacagcagtatcacaggccagatgttgttcctggctagatgtttacatttgtaagaaataacactgtgaatgtaaaacagagccattcccttggaatgcatatcgctgggctcaacatagagtttgtcttcctcttgtttacgacgtgatctaaaccagtccttagcaaggggctcagaacaccccgctctggcagtaggtgtcccccacccccaaagacctgcctgtgtgctccggagatgaatatgagctcattagtaaaaatgacttcacccacgcatatacataaagtatccatgcatgtgcatatagacacatctataattttacacacacacctctcaagacggagatgcatggcctctaagagtgcccgtgtcggttcttcctggaagttgactttccttagacccgccaggtcaagttagccgcgtgacggacatccaggcgtgggacgtggtcagggcagggctcattcattgcccactaggatcccactggcgaagatggtctccatatcagctctctgcagaagggaggaagactttatcatgttcctaaaaatctgtggcaagcacccatcgtattatccaaattttgttgcaaatgtgattaatttggttgtcaagttttgggggtgggctgtggggagattgcttttgttttcctgctggtaatatcgggaaagattttaatgaaaccagggtagaattgtttggcaatgcactgaagcgtgtttctttcccaaaatgtgcctcccttccgctgcgggcccagctgagtctatgtaggtgatgtttccagctgccaagtgctctttgttactgtccaccctcatttctgccagcgcatgtgtcctttcaaggggaaaatgtgaagctgaaccccctccagacacccagaatgtagcatctgagaaggccctgtgccctaaaggacacccctcgcccccatcttcatggagggggtcatttcagagccctcggagccaatgaacagctcctcctcttggagctgagatgagccccacgtggagctcgggacggatagtagacagcaataactcggtgtgtggccgcctggcaggtggaacttcctcccgttgcggggtggagtgaggttagttctgtgtgtctggtgggtggagtcaggcttctcttgctacctgtgagcatccttcccagcagacatcctcatcgggctttgtccctcccccgcttcctccctctgcggggaggacccgggaccacagctgctggccagggtagacttggagctgtcctccagaggggtcacgtgtaggagtgagaagaaggaagatcttgagagctgctgagggaccttggagagctcaggatggctcagacgaggacactcgcttgccgggcctgggcctcctgggaaggagggagctgctcagaatgccgcatgacaactgaaggcaacctggaaggttcaggggccgctcttcccccatgtgcctgtcacgctctggtgcagtcaaaggaacgccttcccctcagttgtttctaagagcagagtctcccgctgcaatctgggtggtaactgccagccttggaggatcgtggccaacgtggacctgcctacggagggtgggctctgacccaagtggggcctccttgtccaggtctcactgctttgcaccgtggtcagagggactgtcagctgagcttgagctcccctggagccagcagggctgtgatgggcgagtcccggagccccacccagacctgaatgcttctgagagcaaagggaaggactgacgagagatgtatatttaattttttaactgctgcaaacattgtacatccaaattaaaggaaaaaaatggaaaccatcagttgttgctgtgtgaggcttgctttgcttcatgagaacctagaccttgctgagctggagtcttaggaagcagtctcctaagtgcttctccagcaggggcagaaactgtcccaccagctaacatctggcattatggagggtcccccaggcagctgccagcagggacaggccccgtgttttctgtagccagggatgaggaagtggccccagggcatgggcctggctgggtgcttctgcaagggccttcccaaaccacagtacaggtggtcttcctgccctgcagatgggagctgtgggagctgctggagctgctggagccttcatggtcaagtgacatcataagcttatatgacatacacaagcctcaggacttggcccatggcactgaagcaggtcatcaggcccagcacagagactagagctgtgttctcacagggcccaccacccttccacctccttggccattgacacctgcgtccctggcccagctgctcccaggtaacccccaaagcagctggcacatcccacctctggtgtggccggggctgctgtgtgtccgcagggcctgccccgtctattctagcttgtttgtcctgtctgaaccagcgcctactccaagaagcctctgctcagcccagcggggatgcttctaagctccggacgagcctctcggaagccttggtgattggtggtgtagtcatcttgggatgcagatgtcttaccaacctgcaagaacaaaaaccctgtggcttcctctggtgcagggtatttagtcaatgtttgctgaggtcccgtctggttctggctaattggcaggggtcgtccacccattctttccctgctctgctgtctgtgccaggagagacgggggccagtcggccaaggggccagctcctgctgcctgctcctcttgggcacgtgcgggggccccctttctctgagcagggatagggatcagtctgccggagggatgtggtggacaggcctaaagcatttggggcggggcatgccacttgagctccctaaatctgtctcctcataggtgacaccgctccagggccccccagtggcctctcctttcagagctacctaaattctggtcacttcagagaaatggagcacccccttctccctggtccaggtgtggacagcctggcacactgagcacacctggcatggctggtaatttcagaaagaagaggggccggggtccagtgggaagcagcggtgaacccctcgtgagtgggctttgcagtccctccccatgccacggcagagctgccctcaacacagccttcctcttcctcatcggagagcacaccctgtccccttgccgagctgtgccctgtgccttcggtggtatttgattttggctgctactggctttgttgggatctggaagtcgcttcccctgcgtggtgcgtggagcactgtaagtcagatgagggaagtagccagggtgaggtgagtaccgggtggagccgccactgaagggactgggtaggggggccttgcctctacatgatgtgacacagccaaccgaggacagaggaagccccgttcctgggggtgtggggtgcacccctcagggaagcctgcagtggggcctgaggaaaggcatcctccgcgagcccacgagtctggtccatgagcaccgtgacagtgtctgtgggtagaggtggacccggccttgtgtcatcaccaggacctcttttgggaaaccatgtggacatcgcttgcgggtcccccaggctctgcagccccagcagcctggctgccttttgggcaagtggcttgagccacagaggacccagtcctgttgcagccacatcctctgggggggcccgccagtgtggccggctttctccaccctacaccaggcctccaggtgtcctggtcgggggtgtctgggccctgggtgggccctgtggacctgtgaggtcagggtcagggcatcactggaggcagagggctgaagttgtgggtctgggttccccttgtgtgcacaggcccctgccctccatgcttggtcaggcagctacccccaaaactgctaggacaggctggtcctgaggtggatcctggcccctgtaccctctggacagcccacccgcccaaccttctaccctgccccagcggcggcagtgttggccacatccttcccctcctggccccaattgctctggggaagtccaggctccggagcctgcccaggggccccccgtgatttgggcccaggactccacgtggttctctgccttcacccaagccctgaactcctcagctgccaaatccccacccatctgcacaggctgtgctcaccactgctgctcctggaaggtgcccctcagtgggacgcccacctcctctctgggcttctgtgtttgggagccctgctgcccccacccttggtcagtccccatgtcctgctggcctgtcaggcagggcagaaaatccacccagaaatgctgagcaggatgagagtctagttgggcccagcctcattatttagaagggatggaggcctagggagcatgcttctagcctgagcccagcagggccccgcccatgtcccaggtctgcaccagggacagctcctgccgaggcctgacctgccccttctccctcaggtgctgctggttgaccagcctctggccctaggagaccccgtagcgactgagggtcccagcaggccatgcagctttgccaaggtacgagcccctccccagcaggggacagatgtggggaccctcccaggcaggagcagctgggtgcctggtgctgccatctgctgcctgcctggttcttgtcctcacattggaggtcagtgtgagggctctgcctcgggaaaggccatggagcttgccctgtccagggcctcccatgtgcactgagcctgggaagagagggttggagttgagccttttaccctgggaatgctgcctggaggatggtgcgggtgtggggtggcaccctgccaggcagggccctgcctccctgcgcccactggaactcgggcaggcaggggtgtaggtgcctcctctagagccgtccggtgggggcccccggcagtggtggtggtgtccactggccagcagctgccccttcagccaggacagtaggcctgacgctgtccccagcagctccaaggtggatttgtggaagggggtagagggcacgtagaggccccatgacctccccagggttctgggagggctgtgcccccttagccagcaccatgctgggtgatatagtcagatcctgttacccctgttgtggaggtgaggaaacaggttagtggggaggacatgactaaggtccatgctgagtcgctagagctgcacccagaaccactgctgggaccccatgcctttctgcttaccccttgtgccgggagatgccaagagatgctgggagccagccccacctctgcccttggagtcatggctacggaaagggcattcggaccggtccctgacctcaccggggagggccgaaccctgttcctgaggagccagggcttcctagaggaggtaggccttctagtcactccttcatctgcaggcactccacagagctctctgtgccagcccccagcacggagggctgaccttagtcgagtggagatgccccagtgccaggcagtagggatgatgtctcctgaggcccagatggaagggactggactagtctcatggggctgatggtggggccaggccttgaccagggacccagtgtagggggtgcagagacccctctgagttcctcacacatccctggggccctccccatacacttcctatcctgactgcgggcaagagggagccccagttcgccttccctatgctgggcacccacagtggggctgggcacccccgccatgcccctgccctgtccttcccctgagagcctcggtcccacctccaaggtgcctcagaggacagcaggggcagcgggcagaggccgagatgcctcctcattccaggctcagctgcccttcttggggcagcccacacctgagagtctcctgcagttggtcaggcctgaggagggcaggggggtgcctgctgtccctctgctgaccacagtggcatttagcctgggcaccgcgcccagcacagtccatgctgcacaggtgccgtgggctccacagagccctgcctgacatgcatgtgttacgtttcgggtgccgatgcccttgggcggcacttctccgggcagaacccccaggccaccgctccggttccggttccgctgcatctggggctctcggcaggctgtggtcctccggccagcctgggggcatctcagtccctcagccccacaggggcctgccccgcagcctgggcctcgagccccgtctccgcacgctgtgccgaatctggctgcccatcagctccctgcgtacccagactgtgccctgccatgcccgtggctcttcccaggagtgccctgtggcctccccctggcttgctgggctgattccctcctgtgtctcaaacagagctcacctttgccatcactgctgtcctcaccggccggtgccagaggcccgtgtctgtgtaccctgtgtctgcacctctgggcagggcctggctctgaccaacccgggcttccagtgtccacagacctaaggcccagggcgcctgggggctggagcaagagaagcaaaaggagccaagggtgggggtttggggttcttgtgagggcccagccccaggaccccaggaccaggacacccaggagccccagggcccagccccagttcagaaggcaggggccttctgagggagcttaagggtcccacagcccaggacccccaccagggccagtggccagcgttgggggactcagcctcctcgtcgctcgtcctctctgtttctcccaccttttgccccctttctccttgcctgttcccacccgaggccccctcttggcctgcgtgagccggggcggcactgaactgggggccgatccgcctgggcggcggtgagaggcagggccgggagccgggccgctgggtttgggcctggcccgctcgccgcaatattgatggcccgtcagtgcagccctgattcctgtgctttcagttaaaaggtttctgttgttgtagcttatgcagttgctctgttgctatggaaacgtgacatcaaaatgacgtttcccgtttaaaagcttttaactaaattcctgcctgtcagatgtaggccccattttgagcgtggagctgccttcgagcgagcgtgagcggcgcctcccgcccatggtgcgtggggccgggccggggccctcgctgagcgcgctctctcaccccacaggcgcctccggcatggcggcggccgaggggcccggctacctcgtgtctccccaggcggagaagcaccggcgggcccgcaactggacggacgccgagatgcgcggcctcatgctggtctgggaggagttcttcgacgagctcaagcagaccaagcgcaacgccaaggtgtacgagaagatggccagcaagctcttcgagatgaccggcgagcgcaggctgggcgaggagatcaagatcaagatcaccaacatgaccttccagtacaggtgggcgagcgggcagtgtgggccccaccaggacgggcgggcccgggcgtggcgggccgctcctgactttcttggagctctgagtcgggacgatgtgtgggtcgtggcctgcctgtcggtctcctctggccgggtatgggcagaaccccacggggtgagacggggcccacggaaaccgtgtgtgcagccttccattggggaagtggggaaactgaggcccagcaagggcaggaaaccagtctaagagctgaggggtagcaggggtggggctggtgctgggcagaggccaggatggctcccaggacgtatgggcggtctgggcactgtccctcggaggcagcaacactcatggtggtgcccactgacctcacaccctgctcccccatagggaggcggcggctgccagtgccctccccaccaccaagctcccaagctcagcaggggtttcaggggcctactgcgtcattggggaaattgagactgcaagtgagaaggaggctcagtgctctgcgacttggagcatccactgagcctctgccatgagccggtgagccccactggggctggccctagggtcacggtggggtatttccagaaatcaccaggtgaggtgcaggaccagccagcgcatgggtggggcttacggtgcgaagaagaaagaggtggaggcctgccctggcccaggactcccagcgtgggggctcccggcctggccccacctctgctcctgctacatggcaggtgggcccttcctgccctggcaacctgcagggaaggccggaggggaccacccagccagggagatgttggcgtctaggaggggacaggtgtggtcccacacacccagcatcttaaagtgcgtgggtccccagcccattaggacagggtcccgggtgggcaggggtcatggtggggtgaaggtctcaggcacaggcaaggtcacaggtgcggtgagggtcttgcagggtgtgaaggtcataggtgtgcggtgaaggtcacaggtgtggggtgatggttttgggtgtggggagggtcttgcacggagcgagggtggcagcaagagctggaagctgcagggggagaatggcagcagagagcacccggccctgtgggcggcctggacagggctgggcctggggctgccggagagcctgtcagcttccaggatgggagtggcctcactcagctgctccacctccgggtcaggcaggtgagcctggggcagagaggctgagagcacctgagccacttgtgggagaggccacccccactgcccccctcaggcgaggagccggcctccagcacagcagaagggaacccccagtccccagccctagtgggagtggggaagaggcccagcaaggccccggacagaccgccagcctgtgaggtctccgctttcagttgcgttgatttgattttttctgagccttgaaggaggggtccggggcctggccctgcccaaaggcccctaggcaggccccaaagccgggacctagggtgctgagcatgacggatgttgggtttgagcggctggcttgcgacgtgagggctgaggtgtgagcctgggtatcttcagaggttcggtggacacaggcagctgcccgcggccccactgttcccgtggcctcctagtcctgctcaggcacctggtgaggaagggacgcagagggcagtgggaggtggccacgactgttccagcaggctcccctctgactcaggaattcacgggcaccacctccctggctggctctggttggtgtctggccaggttattcattatttatgctgaaagcctcttcagagtcccaggggagggtttctgtctccattcctggaggctgagagatgagggtgcagcagagtgggggcctccactccagaccctgcagtctgggctggccaagggctgcaccggtgcactgcacgtcatggctgatgaagcacttccacaccgcagcccctcagagctgccacagtcagccttagttcaccgagggggaagctgaggcccagagcatgagagggacttgcccagggccacatagtccttagcagaggaagctgtggctgggtgactcgatctttgtcctttttctttatacccgcagtctccccatagcagaggcttttcttttttttttctttttcttttttttttttttacaagaactctttatatattaaggctgttgggctgaagaagcctgagagggtggctggttctgtggagcatggtttgttgaagtacagtttgggggcctcctacactgagaataggccttttctcgtttctccaaagagtgggctggctcaagtagggcagagagagaagcctggggcagaggttagggatgggcacccagcgcctgccctcacacgctctgtgctggtgtcttcacagccacgtgccaccctgggcagcatcccctgctcaccatctggctgtgcctgtttgctgggggcacctcattcagaatccagcttattgtttccaacggccaatggccacaccctggcaggtagcaagagtaggagagaggagacacccactccgagcacaggttgggtttggagcccggccttggggcactctgtcactcaaaggcagagtggggagtgggcactgggccttaggaggtactgggtccagtgaggcagagatgcccctgccccacccccaccttgtggcttcttccctggcctggccagagctgtctggccgccatggggccctgtgtctcctgccttgacctcccagagggcagccgaggcccaggggaggcctggggacttagcctctcagggcaggacctgtctgcaggagtaggtgggtgctgggggtcccagtggtaatgaggcatcaggcagtgtgggaaggggcccatccggcccaccccagggcctctgggcaggttgcaggttgtagcgctggatctaggctcctgcccagactgtaggttcaaccaagaatggcatgggagcccagcctgctgtttgctttattaaatctgccctgtagctgggggaggggcttactttgatcatcactatgtcattgatataaaaatagaggctcagagaggtgaatgaacctgcccaaagtcacacagcaaagtgtggagatgagatactgactcagggctgtggacactgaagcctgtgctctaacgccagtggctgtcgctccctgaggcattctctcccgaacaacacagttattatattacaaaatattatcactatatttatatatcttataataccttattattacaataaaaccttattactctacctttcaaaatgaattatttaaaaagcagtatttgctcattgcagagagtctagaaactatagaaaagcaagggaaaagcaataggaccagccccaaggtcccagcatgcacagataaccttagtaatactgggacgtgtgcttcctttttaacatctgagcccgtgtaggtcctgaagcccagcttctttctaagtccattgtcatcttgaccctggagcctggccgattttgctggggaggcccttgccagccgagagcggctcctgcctgtgccggcgtggcgcgcccctctgctgaggctgggcaggacaggggctgggccagctctgtttctcacccttggctcttgtgtctctcgtttcaggaaattaaaatgcatgacagatagcgagtccgccccgcccgactggccctattacctagccattgatgggattctggccaaggtccccgagtcctgtgatggcaaactgccggacagccagccgccggggccctccacgtcccagaccgaggcgtccctgtcgccgcccgctaagtccacccctctgtacttcccgtataaccagtgctcctacgaaggccgcttcgaggatgatcgctccgacagctcctccagcttactgtcccttaagttcaggtagtgtgtctgcttgtccttcccctgccctggggtatctcagcccccaccatttagagaaagggactgggagtggcaaggccggcggcggcggccacagtggttgcagaggccgtggctgcgggcagcgcctccagggacaggcggcctcagaccagggagggctttagtgtccacaggcagaccgagtttgtctcccagctccatcacttttgagctgcacggaaagttccttgacttctctggcctcagtctccctcctataaaatgggggtaaatcagtacctttctcagagggtggctgggagcatcacaggagagaagacgcagcatggggcccggcacacggagggagaccaagccccagaccccagaatgcgccccctggcctcccttagcccacacagaccccaccctcacaggctagctgccctctcagcactggggagggtgtcgggctgcacctcatcacgtgttgccgtgggcatgacccgtcccctctgccatccatcccacacctcagacccgtcccgtgctggccacgtgactgtgcctgcaagatgctcacagggcagccgggagccaggcagcatgcaggacagacacctgcggggtgggcctggggagcccagagaaggtgcttttgaggaggggacatttggggtgggctttcaaggtaaaatagaagttggccatttggaggcaagaacaggaagattgtggatttgagtcacagcttctcccctgccctggtcttcaagtctttctgacaggaggtgtcagaaaagtatctttagtagagaaggcgtctccgaggagggtccctctcatgccgggggccgctgcttgactcaggatttctcattgaagacctgagacaaaaacgcttttgctggcagctagaaggaaccagcaggaggcctgagatttgtggctgttgttcccgtggactgagcccagttctcagactcagctgcctggggccttgcacaggactggggcgtgggggctgccctccctgatcaggcccaaagcgcggatctcacgcccctgaggttggctgtaccctctcagctcagagcagagtgtgggccagggatgagcaggcactggagcagggccctggggtctgtgggttttggcagctccctgcccttcagggaggtctgctgagaccacgggtggcccctaccccagcagcagagctctcaggaggcgcccacagggctggactgcctttactcaccacctctaccagagctctgaggtcctggggagagagcccaggcctcttgtgggccccacaccctctaggtgcctgtccttctgcctctctaccaaggtgtgccggccccatttctaggccgccgggagataagggggctcacatctcaggcccttccttctgggacctcagtttccccatctgcctaaggccgggtggggctggtggtcttggcttccctacaggggtcctgagtactctgcactacccagcaccccccacccctgccttcatctctccctgggggtggtctctccacccctggcccccaactggggctgagcccccacctgcccagtttggtgggtgaagggtgctccctggcaggatatgcccctctgcagcccagaacatcccaccctttccagaccgaaggggtgtggattgtcctgggaccctggtcattggggtcatccgctagtcgcaaaggacggcaatgcctgtggcctctctttctttctttttctttttttttttttttgagacggagtctcgctcttgtgcagagagcagtggcgcgatcttggctcactgcaacctccgcctcgtgggttcaagcgattctcctgcctcagcctcccgagtagctgggattacaggcacccgccacaacgcctggctaatttttgtatttttagtagagatggggtttcaccatgttggccaggctggtcttgaactcctgacctcaggtgatccacctgcctctgcctcccaaagtgctgggattacaggcataagcctccacacccggccacccctgttactttctgtcaaaggcggtgggttctggcccctcctttgcacatggaatatgagaccctgagtaagtgacctgactccctggggcctcagtttccccatttgcccagtaggattgtcgggagggtccggtgaggcccctggtgtgcccaggctctgtggccagcacgtccacagccggcactgtccttccaggtcggaggagcggccggtgaagaagcgcaaggtgcagagctgccacctgcagaagaagcagctgcggctgctggaggccatggtggaggagcagcgccggctgagccgcgccgtggaggagacctgccgcgaggtgcgccgcgtgctggaccagcagcacatcctgcaggtgcagagcctgcagctgcaggagcgcatgatgagtctgctggagaggatcatcaccaagtccagcgtctaggccagcaggcggcggcggcggcggggccgggcggctggtggtactgctcaggccacccagggcaggccactcaggccaggcgggcaagggggccgccccgcgagcggagaccgccttccacctggcctctggcaggatgtcccttctgaggggtattttgaggaacccccaggccctggggaccgtgaggctccagtctccagcatgaatgcccttcctcggacacaggccagggcctctggggttcactccgagtaagaacgtcctagagccactctccagtgtcgttactatcaatgatacttgacgtggctttgatattaaacgtatactttttcattcttgcctggaacgcacagtttgctgttgctggcttggtgaggatgccctgattgatggatcccgaaaatgaaagcagatggaaacgggttggggcaggctggagctgggggagctctctcctgaagggaaccctgtgtcctccctcaccaggacctctgcgtctctccttaaatggcctctgacgcctgatgaaaaccccagcgaccttccaggaggcttttattcagctctgtttggagcatcaggtgtttccactgcctccttagcaatgacactaataaaagtcgtaacacctgttcacatgcacagccctgttgagtgttctgggtgctggagatatcatggtggatgacacaaaggccctggcctcttggagcttatgctcccatgcggggaagacacatgggtcagtagagaaatggttgcaggttgtgataagtgctggaagggaggggttggcctgaggacacggaggcagacatacgtggagctgggaacagtggccacacagggaacggccagtgcgaaggcccagaggcagaggacactggagcaagcccaggagcagctaggaggctggtggccagcagccaggccacggaagcccgtgcagcccgtggggaggagtgttcatgcttttcaagcttagtgggagtcttttggccagtgcagctctgggtctgacatcggtgggggacagaggggtggtggagcggccacagctgcaagctcacctcactgccggcccttccaccagtttcaaactctttctagaagctccagctttcccaaagctgaattctctatgagcctccttggccgggactcgggcgtctggttgccctggctgcaaaggaggctggggccaggtgtgtttgagtcacctcctggaattaggcaagttgctgcccaaatagaaggttgttggcaggtgggtcagcaggtgaacagcatggtttgactcagggttcagaaaaatctccctctggctgccaagcgagcaggccgtggagacaggtgcagaggcaggtgtggcagcaggcatcctgccaggcagtgctgcagtcatcctgcgacaagcagcagcagctcatcctaccctctagggggtcttgaggtcagccaggcaagagagcagcttggactccactgggtgtgggaccagcctgtggaccatggtggtgtggagggtgccctcggcctgcctgtgtgaaggagaggccggcgtgttctgtggagcccaaaggggagctgggcaagcaggattcacttcactctgagggtcctggagctcccaccctcctcagccatctccccagagcctgtgtgccgaggactcggcccatgttgctgtgggatgagaggcagagtgtcgtgagggtgtaaggagcggcggcagtggtgggaggagggagcagcagccagcgctacggtgccagtttccagctgccagatgacgccgctgaccctgtggttgagaagagatgcacagagccagctcttgcaagccagtgtggctgccatagcacctgccgagaagcagaaggaagggtggccccaggaggacagaggatgcgggcacatctgatgcgggcctgagttttgggagcttttgctctagccagtttccagctccgggacccacccgcctcgtaggcaagacaccacccaagaaatcatttgcttaacaaacacactgggctccaactggacacctgtgccaccctagatgctgggaacccagccatgacacaggcacctgcccccagctgctgaccactgaggctggctagcagctcccatggggccagtgtggggttccccagcctcctaacagggagccagtcacaagccctcgagagggaagggtgcccgcggccctggcaggaaggttaggctggacgctcccacaagacataacagatggaggttctaaatgatgtagcaacttcttcaccctgaaactgctgtagagtcagccatgacgcaccggtacttcagtaactgccaggcatccgggacagcacaccgcgagtcgctgctgtgcttgggttagaagtggtttggtctgttttcttctcgccctctctaatcagagtcagtgattcatgcccttccatcaccttagagaaggggcaggcgctgcccgaccttctccaggctggagcagcatcgcctcatgtcagcagaactcagctgtagaatatcgtggggttggtgcctttcatcagcagcatgtccttaacaactttctgatttcttccttagttgttggtccattaaggagaaaaaaaatgatctcagccattgctaaaatatttgataagattcagcaaagcagcatgttaacattgaaaactagaatcaggagccaggcagatgtgcttgcttttcacctgtagtatttcatgttgttttgacgtttttagctaatgcattaagataaataaacaaaagccgggcacggtggttcacgcctgtaatcccagcactttgggaggctgaggcgggaggatcctctgaggtcaggagttcaagaccagcctgaccaacatggagaaacctcgtcattactaaaaatacaaaattagctgggcgtggtggtgcatgcctgtaatcccagctacttgggaggctgaggcaggagaatcgcttgaacccgggaggcggaggttgcagtgagctgagattgcaccactgcactccagcctgggtgacagtgaaactcggtctcaaaaaaaaaaaaaaattaaaaaaagataaataaaataagcaggataagaaatgaagaaagtagagttacctttgttttcagatttcatttttgtatacccagaaagccaaatgtacaaaagactgggagctctttaaaccagcttaaacttgttgaaaatgaggatgaagaaatatcccattcagagttggaatgaatttaacccagaaggaacaggacctctactgaagagaactatgcagtcttactgaaaaatctaaataatacctgagcgctggagaaacttcgcacactcctgaaagctccaaagtcaatgtcatcattttattaatgtcattccaaacatagtctcaataatatcacttcttggttttgacatggacgcgatgatgtttaaattcatatgaaaaaagaacggggccaaaagtccaaggccagtcagcgtgagaagaccgctcggcctccctcggagtcggggagttggaaccgcagactgagatcatgtggctgctggaggccaggacgaacgtcgggaaatggagactcctgcgttgctggtgggatgtggtgcagccgcttccaggagcaatttggtgtcccgtcctaaagctgaagaaacgcatttcctctggtcagtgccactcctagacaggccaccctgcggcagccgtcctcaaactggtctgaggacccctcaacgctcttaaaaatcattaaaagtgggccaggtgcggtggctcacacctgtaatcccagcactttgggaggccaagacaggcggatcacgaggtcaggacattgagatcatcctggctaacacggtgaaaccccgtctctactaaaaatacaaaaaattagccgggcgtggtggcgggcgcctgtagtcccagctacttgggaggctgagccaggagaatggcgtgaacccaggaggtggagcttgcagtgagctgagatcactccactgcactccagcctgggcagcagagcgagactctgtctcaaaaaaaaataataaataaataaataaaaataaaataaaataaaattcattaaaagtgccaaagaacttttgcttatgtgagttctaatgaccaatattaatacacattagaatatcttattagaaattaaacctgagacctttagaaaacatgtattcatttcaaaatagcaataaacccatgacatattaacataaataacaattgtatgaaaaatatattttccaaaacaaaaagttttcgggagaagtgtggcatagttttacatggtcgtaaatctctggcttaagagaagcccactggcctctcagcaggctctgggtccgtccactttgggggtgttttggttgtgaagtataggagtgaatggagaagctcattcttacccagatgtgtatttgaaaagaaaaggaacattttaataacctttgcaaataatcggtatattcttccgtgatcctattccaacactggacaggtggtggtttgttttttttttttggagacggagtcccgctctgtcactcaggctggagtgcagtggcgcgatttcagctcactgcaagctccgcctcc

SEQ ID NO: 2 - RNA, 13481 nt, Homo sapiens
  source 1..13481: mol_type = mRNA
  CDS 146..9580: protein_id = 95; translation = MATLEKLMKAFESLKSFQQQQQQQQQQQQQQQQQQQQQQQPPPPPPPPPPPQLPQPPPQAQPLLPQPQPPPPPPPPPPGPAVAEEPLHRPKKELSATKKDRVNHCLTICENIVAQSVRNSPEFQKLLGIAMELFLLCSDDAESDVRMVADECLNKVIKALMDSNLPRLQLELYKEIKKNGAPRSLRAALWRFAELAHLVRPQKCRPYLVNLLPCLTRTSKRPEESVQETLAAAVPKIMASFGNFANDNEIKVLLKAFIANLKSSSPTIRRTAAGSAVSICQHSRRTQYFYSWLLNVLLGLLVPVEDEHSTLLILGVLLTLRYLVPLLQQQVKDTSLKGSFGVTRKEMEVSPSAEQLVQVYELTLHHTQHQDHNVVTGALELLQQLFRTPPPELLQTLTAVGGIGQLTAAKEESGGRSRSGSIVELIAGGGSSCSPVLSRKQKGKVLLGEEEALEDDSESRSDVSSSALTASVKDEISGELAASSGVSTPGSAGHDIITEQPRSQHTLQADSVDLASCDLTSSATDGDEEDILSHSSSQVSAVPSDPAMDLNDGTQASSPISDSSQTTTEGPDSAVTPSDSSEIVLDGTDNQYLGLQIGQPQDEDEEATGILPDEASEAFRNSSMALQQAHLLKNMSHCRQPSDSSVDKFVLRDEATEPGDQENKPCRIKGDIGQSTDDDSAPLVHCVRLLSASFLLTGGKNVLVPDRDVRVSVKALALSCVGAAVALHPESFFSKLYKVPLDTTEYPEEQYVSDILNYIDHGDPQVRGATAILCGTLICSILSRSRFHVGDWMGTIRTLTGNTFSLADCIPLLRKTLKDESSVTCKLACTAVRNCVMSLCSSSYSELGLQLIIDVLTLRNSSYWLVRTELLETLAEIDFRLVSFLEAKAENLHRGAHHYTGLLKLQERVLNNVVIHLLGDEDPRVRHVAAASLIRLVPKLFYKCDQGQADPVVAVARDQSSVYLKLLMHETQPPSHFSVSTITRIYRGYNLLPSITDVTMENNLSRVIAAVSHELITSTTRALTFGCCEALCLLSTAFPVCIWSLGWHCGVPPLSASDESRKSCTVGMATMILTLLSSAWFPLDLSAHQDALILAGNLLAASAPKSLRSSWASEEEANPAATKQEEVWPALGDRALVPMVEQLFSHLLKVINICAHVLDDVAPGPAIKAALPSLTNPPSLSPIRRKGKEKEPGEQASVPLSPKKGSEASAASRQSDTSGPVTTSKSSSLGSFYHLPSYLKLHDVLKATHANYKVTLDLQNSTEKFGGFLRSALDVLSQILELATLQDIGKCVEEILGYLKSCFSREPMMATVCVQQLLKTLFGTNLASQFDGLSSNPSKSQGRAQRLGSSSVRPGLYHYCFMAPYTHFTQALADASLRNMVQAEQENDTSGWFDVLQKVSTQLKTNLTSVTKNRADKNAIHNHIRLFEPLVIKALKQYTTTTCVQLQKQVLDLLAQLVQLRVNYCLLDSDQVFIGFVLKQFEYIEVGQFRESEAIIPNIFFFLVLLSYERYHSKQIIGIPKIIQLCDGIMASGRKAVTHAIPALQPIVHDLFVLRGTNKADAGKELETQKEVVVSMLLRLIQYHQVLEMFILVLQQCHKENEDKWKRLSRQIADIILPMLAKQQMHIDSHEALGVLNTLFEILAPSSLRPVDMLLRSMFVTPNTMASVSTVQLWISGILAILRVLISQSTEDIVLSRIQELSFSPYLISCTVINRLRDGDSTSTLEEHSEGKQIKNLPEETFSRFLLQLVGILLEDIVTKQLKVEMSEQQHTFYCQELGTLLMCLIHIFKSGMFRRITAAATRLFRSDGCGGSFYTLDSLNLRARSMITTHPALVLLWCQILLLVNHTDYRWWAEVQQTPKRHSLSSTKLLSPQMSGEEEDSDLAAKLGMCNREIVRRGALILFCDYVCQNLHDSEHLTWLIVNHIQDLISLSHEPPVQDFISAVHRNSAASGLFIQAIQSRCENLSTPTMLKKTLQCLEGIHLSQSGAVLTLYVDRLLCTPFRVLARMVDILACRRVEMLLAANLQSSMAQLPMEELNRIQEYLQSSGLAQRHQRLYSLLDRFRLSTMQDSLSPSPPVSSHPLDGDGHVSLETVSPDKDWYVHLVKSQCWTRSDSALLEGAELVNRIPAEDMNAFMMNSEFNLSLLAPCLSLGMSEISGGQKSALFEAAREVTLARVSGTVQQLPAVHHVFQPELPAEPAAYWSKLNDLFGDAALYQSLPTLARALAQYLVVVSKLPSHLHLPPEKEKDIVKFVVATLEALSWHLIHEQIPLSLDLQAGLDCCCLALQLPGLWSVVSSTEFVTHACSLIYCVHFILEAVAVQPGEQLLSPERRTNTPKAISEEEEEVDPNTQNPKYITAACEMVAEMVESLQSVLALGHKRNSGVPAFLTPLLRNIIISLARLPLVNSYTRVPPLVWKLGWSPKPGGDFGTAFPEIPVEFLQEKEVFKEFIYRINTLGWTSRTQFEETWATLLGVLVTQPLVMEQEESPPEEDTERTQINVLAVQAITSLVLSAMTVPVAGNPAVSCLEQQPRNKPLKALDTRFGRKLSIIRGIVEQEIQAMVSKRENIATHHLYQAWDPVPSLSPATTGALISHEKLLLQINPERELGSMSYKLGQVSIHSVWLGNSITPLREEEWDEEEEEEADAPAPSSPPTSPVNSRKHRAGVDIHSCSQFLLELYSRWILPSSSARRTPAILISEVVRSLLVVSDLFTERNQFELMYVTLTELRRVHPSEDEILAQYLVPATCKAAAVLGMDKAVAEPVSRLLESTLRSSHLPSRVGALHGVLYVLECDLLDDTAKQLIPVISDYLLSNLKGIAHCVNIHSQQHVLVMCATAFYLIENYPLDVGPEFSASIIQMCGVMLSGSEESTPSIIYHCALRGLERLLLSEQLSRLDAESLVKLSVDRVNVHSPHRAMAALGLMLTCMYTGKEKVSPGRTSDPNPAAPDSESVIVAMERVSVLFDRIRKGFPCEARVVARILPQFLDDFFPPQDIMNKVIGEFLSNQQPYPQFMATVVYKVFQTLHSTGQSSMVRDWVMLSLSNFTQRAPVAMATWSLSCFFVSASTSPWVAAILPHVISRMGKLEQVDVNLFCLVATDFYRHQIEEELDRRAFQSVLEVVAAPGSPYHRLLTCLRNVHKVTTC
gctgccgggacgggtccaagatggacggccgctcaggttctgcttttacctgcggcccagagccccattcattgccccggtgctgagcggcgccgcgagtcggcccgaggcctccggggactgccgtgccgggcgggagaccgccatggcgaccctggaaaagctgatgaaggccttcgagtccctcaagtccttccagcagcagcagcagcagcagcagcagcagcagcagcagcagcagcagcagcagcagcagcagcaacagccgccaccgccgccgccgccgccgccgcctcctcagcttcctcagccgccgccgcaggcacagccgctgctgcctcagccgcagccgcccccgccgccgcccccgccgccacccggcccggctgtggctgaggagccgctgcaccgaccaaagaaagaactttcagctaccaagaaagaccgtgtgaatcattgtctgacaatatgtgaaaacatagtggcacagtctgtcagaaattctccagaatttcagaaacttctgggcatcgctatggaactttttctgctgtgcagtgatgacgcagagtcagatgtcaggatggtggctgacgaatgcctcaacaaagttatcaaagctttgatggattctaatcttccaaggttacagctcgagctctataaggaaattaaaaagaatggtgcccctcggagtttgcgtgctgccctgtggaggtttgctgagctggctcacctggttcggcctcagaaatgcaggccttacctggtgaaccttctgccgtgcctgactcgaacaagcaagagacccgaagaatcagtccaggagaccttggctgcagctgttcccaaaattatggcttcttttggcaattttgcaaatgacaatgaaattaaggttttgttaaaggccttcatagcgaacctgaagtcaagctcccccaccattcggcggacagcggctggatcagcagtgagcatctgccagcactcaagaaggacacaatatttctatagttggctactaaatgtgctcttaggcttactcgttcctgtcgaggatgaacactccactctgctgattcttggcgtgctgctcaccctgaggtatttggtgcccttgctgcagcagcaggtcaaggacacaagcctgaaaggcagcttcggagtgacaaggaaagaaatggaagtctctccttctgcagagcagcttgtccaggtttatgaactgacgttacatcatacacagcaccaagaccacaatgttgtgaccggagccctggagctgttgcagcagctcttcagaacgcctccacccgagcttctgcaaaccctgaccgcagtcgggggcattgggcagctcaccgctgctaaggaggagtctggtggccgaagccgtagtgggagtattgtggaacttatagctggagggggttcctcatgcagccctgtcctttcaagaaaacaaaaaggcaaagtgctcttaggagaagaagaagccttggaggatgactctgaatcgagatcggatgtcagcagctctgccttaacagcctcagtgaaggatgagatcagtggagagctggctgcttcttcaggggtttccactccagggtcagcaggtcatgacatcatcacagaacagccacggtcacagcacacactgcaggcggactcagtggatctggccagctgtgacttgacaagctctgccactgatggggatgaggaggatatcttgagccacagctccagccaggtcagcgccgtcccatctgaccctgccatggacctgaatgatgggacccaggcctcgtcgcccatcagcgacagctcccagaccaccaccgaagggcctgattcagctgttaccccttcagacagttctgaaattgtgttagacggtaccgacaaccagtatttgggcctgcagattggacagccccaggatgaagatgaggaagccacaggtattcttcctgatgaagcctcggaggccttcaggaactcttccatggcccttcaacaggcacatttattgaaaaacatgagtcactgcaggcagccttctgacagcagtgttgataaatttgtgttgagagatgaagctactgaaccgggtgatcaagaaaacaagccttgccgcatcaaaggtgacattggacagtccactgatgatgactctgcacctcttgtccattgtgtccgccttttatctgcttcgtttttgctaacagggggaaaaaatgtgctggttccggacagggatgtgagggtcagcgtgaaggccctggccctcagctgtgtgggagcagctgtggccctccacccggaatctttcttcagcaaactctataaagttcctcttgacaccacggaataccctgaggaacagtatgtctcagacatcttgaactacatcgatcatggagacccacaggttcgaggagccactgccattctctgtgggaccctcatctgctccatcctcagcaggtcccgcttccacgtgggagattggatgggcaccattagaaccctcacaggaaatacattttctttggcggattgcattcctttgctgcggaaaacactgaaggatgagtcttctgttacttgcaagttagcttgtacagctgtgaggaactgtgtcatgagtctctgcagcagcagctacagtgagttaggactgcagctgatcatcgatgtgctgactctgaggaacagttcctattggctggtgaggacagagcttctggaaacccttgcagagattgacttcaggctggtgagctttttggaggcaaaagcagaaaacttacacagaggggctcatcattatacagggcttttaaaactgcaagaacgagtgctcaataatgttgtcatccatttgcttggagatgaagaccccagggtgcgacatgttgccgcagcatcactaattaggcttgtcccaaagctgttttataaatgtgaccaaggacaagctgatccagtagtggccgtggcaagagatcaaagcagtgtttacctgaaacttctcatgcatgagacgcagcctccatctcatttctccgtcagcacaataaccagaatatatagaggctataacctactaccaagcataacagacgtcactatggaaaataacctttcaagagttattgcagcagtttctcatgaactaatcacatcaaccaccagagcactcacatttggatgctgtgaagctttgtgtcttctttccactgccttcccagtttgcatttggagtttaggttggcactgtggagtgcctccactgagtgcctcagatgagtctaggaagagctgtaccgttgggatggccacaatgattctgaccctgctctcgtcagcttggttcccattggatctctcagcccatcaagatgctttgattttggccggaaacttgcttgcagccagtgctcccaaatctctgagaagttcatgggcctctgaagaagaagccaacccagcagccaccaagcaagaggaggtctggccagccctgggggaccgggccctggtgcccatggtggagcagctcttctctcacctgctgaaggtgattaacatttgtgcccacgtcctggatgacgtggctcctggacccgcaataaaggcagccttgccttctctaacaaaccccccttctctaagtcccatccgacgaaaggggaaggagaaagaaccaggagaacaagcatctgtaccgttgagtcccaagaaaggcagtgaggccagtgcagcttctagacaatctgatacctcaggtcctgttacaacaagtaaatcctcatcactggggagtttctatcatcttccttcatacctcaaactgcatgatgtcctgaaagctacacacgctaactacaaggtcacgctggatcttcagaacagcacggaaaagtttggagggtttctccgctcagccttggatgttctttctcagatactagagctggccacactgcaggacattgggaagtgtgttgaagagatcctaggatacctgaaatcctgctttagtcgagaaccaatgatggcaactgtttgtgttcaacaattgttgaagactctctttggcacaaacttggcctcccagtttgatggcttatcttccaaccccagcaagtcacaaggccgagcacagcgccttggctcctccagtgtgaggccaggcttgtaccactactgcttcatggccccgtacacccacttcacccaggccctcgctgacgccagcctgaggaacatggtgcaggcggagcaggagaacgacacctcgggatggtttgatgtcctccagaaagtgtctacccagttgaagacaaacctcacgagtgtcacaaagaaccgtgcagataagaatgctattcataatcacattcgtttgtttgaacctcttgttataaaagctttaaaacagtacacgactacaacatgtgtgcagttacagaagcaggttttagatttgctggcgcagctggttcagttacgggttaattactgtcttctggattcagatcaggtgtttattggctttgtattgaaacagtttgaatacattgaagtgggccagttcagggaatcagaggcaatcattccaaacatctttttcttcttggtattactatcttatgaacgctatcattcaaaacagatcattggaattcctaaaatcattcagctctgtgatggcatcatggccagtggaaggaaggctgtgacacatgccataccggctctgcagcccatagtccacgacctctttgtattaagaggaacaaataaagctgatgcaggaaaagagcttgaaacccaaaaagaggtggtggtgtcaatgttactgagactcatccagtaccatcaggtgttggagatgttcattcttgtcctgcagcagtgccacaaggagaatgaagacaagtggaagcgactgtctcgacagatagctgacatcatcctcccaatgttagccaaacagcagatgcacattgactctcatgaagcccttggagtgttaaatacattatttgagattttggccccttcctccctccgtccggtagacatgcttttacggagtatgttcgtcactccaaacacaatggcgtccgtgagcactgttcaactgtggatatcgggaattctggccattttgagggttctgatttcccagtcaactgaagatattgttctttctcgtattcaggagctctccttctctccgtatttaatctcctgtacagtaattaataggttaagagatggggacagtacttcaacgctagaagaacacagtgaagggaaacaaataaagaatttgccagaagaaacattttcaaggtttctattacaactggttggtattcttttagaagacattgttacaaaacagctgaaggtggaaatgagtgagcagcaacatactttctattgccaggaactaggcacactgctaatgtgtctgatccacatcttcaagtctggaatgttccggagaatcacagcagctgccactaggctgttccgcagtgatggctgtggcggcagtttctacaccctggacagcttgaacttgcgggctcgttccatgatcaccacccacccggccctggtgctgctctggtgtcagatactgctgcttgtcaaccacaccgactaccgctggtgggcagaagtgcagcagaccccgaaaagacacagtctgtccagcacaaagttacttagtccccagatgtctggagaagaggaggattctgacttggcagccaaacttggaatgtgcaatagagaaatagtacgaagaggggctctcattctcttctgtgattatgtctgtcagaacctccatgactccgagcacttaacgtggctcattgtaaatcacattcaagatctgatcagcctttcccacgagcctccagtacaggacttcatcagtgccgttcatcggaactctgctgccagcggcctgttcatccaggcaattcagtctcgttgtgaaaacctttcaactccaaccatgctgaagaaaactcttcagtgcttggaggggatccatctcagccagtcgggagctgtgctcacgctgtatgtggacaggcttctgtgcacccctttccgtgtgctggctcgcatggtcgacatccttgcttgtcgccgggtagaaatgcttctggctgcaaatttacagagcagcatggcccagttgccaatggaagaactcaacagaatccaggaataccttcagagcagcgggctcgctcagagacaccaaaggctctattccctgctggacaggtttcgtctctccaccatgcaagactcacttagtccctctcctccagtctcttcccacccgctggacggggatgggcacgtgtcactggaaacagtgagtccggacaaagactggtacgttcatcttgtcaaatcccagtgttggaccaggtcagattctgcactgctggaaggtgcagagctggtgaatcggattcctgctgaagatatgaatgccttcatgatgaactcggagttcaacctaagcctgctagctccatgcttaagcctagggatgagtgaaatttctggtggccagaagagtgccctttttgaagcagcccgtgaggtgactctggcccgtgtgagcggcaccgtgcagcagctccctgctgtccatcatgtcttccagcccgagctgcctgcagagccggcggcctactggagcaagttgaatgatctgtttggggatgctgcactgtatcagtccctgcccactctggcccgggccctggcacagtacctggtggtggtctccaaactgcccagtcatttgcaccttcctcctgagaaagagaaggacattgtgaaattcgtggtggcaacccttgaggccctgtcctggcatttgatccatgagcagatcccgctgagtctggatctccaggcagggctggactgctgctgcctggccctgcagctgcctggcctctggagcgtggtctcctccacagagtttgtgacccacgcctgctccctcatctactgtgtgcacttcatcctggaggccgttgcagtgcagcctggagagcagcttcttagtccagaaagaaggacaaataccccaaaagccatcagcgaggaggaggaggaagtagatccaaacacacagaatcctaagtatatcactgcagcctgtgagatggtggcagaaatggtggagtctctgcagtcggtgttggccttgggtcataaaaggaatagcggcgtgccggcgtttctcacgccattgctaaggaacatcatcatcagcctggcccgcctgccccttgtcaacagctacacacgtgtgcccccactggtgtggaagcttggatggtcacccaaaccgggaggggattttggcacagcattccctgagatccccgtggagttcctccaggaaaaggaagtctttaaggagttcatctaccgcatcaacacactaggctggaccagtcgtactcagtttgaagaaacttgggccaccctccttggtgtcctggtgacgcagcccctcgtgatggagcaggaggagagcccaccagaagaagacacagagaggacccagatcaacgtcctggccgtgcaggccatcacctcactggtgctcagtgcaatgactgtgcctgtggccggcaacccagctgtaagctgcttggagcagcagccccggaacaagcctctgaaagctctcgacaccaggtttgggaggaagctgagcattatcagagggattgtggagcaagagattcaagcaatggtttcaaagagagagaatattgccacccatcatttatatcaggcatgggatcctgtcccttctctgtctccggctactacaggtgccctcatcagccacgagaagctgctgctacagatcaaccccgagcgggagctggggagcatgagctacaaactcggccaggtgtccatacactccgtgtggctggggaacagcatcacacccctgagggaggaggaatgggacgaggaagaggaggaggaggccgacgcccctgcaccttcgtcaccacccacgtctccagtcaactccaggaaacaccgggctggagttgacatccactcctgttcgcagtttttgcttgagttgtacagccgctggatcctgccgtccagctcagccaggaggaccccggccatcctgatcagtgaggtggtcagatcccttctagtggtctcagacttgttcaccgagcgcaaccagtttgagctgatgtatgtgacgctgacagaactgcgaagggtgcacccttcagaagacgagatcctcgctcagtacctggtgcctgccacctgcaaggcagctgccgtccttgggatggacaaggccgtggcggagcctgtcagccgcctgctggagagcacgctcaggagcagccacctgcccagcagggttggagccctgcacggcgtcctctatgtgctggagtgcgacctgctggacgacactgccaagcagctcatcccggtcatcagcgactatctcctctccaacctgaaagggatcgcccactgcgtgaacattcacagccagcagcacgtactggtcatgtgtgccactgcgttttacctcattgagaactatcctctggacgtagggccggaattttcagcatcaataatacagatgtgtggggtgatgctgtctggaagtgaggagtccaccccctccatcatttaccactgtgccctcagaggcctggagcgcctcctgctctctgagcagctctcccgcctggatgcagaatcgctggtcaagctgagtgtggacagagtgaacgtgcacagcccgcaccgggccatggcggctctgggcctgatgctcacctgcatgtacacaggaaaggagaaagtcagtccgggtagaacttcagaccctaatcctgcagcccccgacagcgagtcagtgattgttgctatggagcgggtatctgttctttttgataggatcaggaaaggctttccttgtgaagccagagtggtggccaggatcctgccccagtttctagacgacttcttcccaccccaggacatcatgaacaaagtcatcggagagtttctgtccaaccagcagccatacccccagttcatggccaccgtggtgtataaggtgtttcagactctgcacagcaccgggcagtcgtccatggtccgggactgggtcatgctgtccctctccaacttcacgcagagggccccggtcgccatggccacgtggagcctctcctgcttctttgtcagcgcgtccaccagcccgtgggtcgcggcgatcctcccacatgtcatcagcaggatgggcaagctggagcaggtggacgtgaaccttttctgcctggtcgccacagacttctacagacaccagatagaggaggagctcgaccgcagggccttccagtctgtgcttgaggtggttgcagccccaggaagcccatatcaccggctgctgacttgtttacgaaatgtccacaaggtcaccacctgctgagcgccatggtgggagagactgtgaggcggcagctggggccggagcctttggaagtctgcgcccttgtgccctgcctccaccgagccagcttggtccctatgggcttccgcacatgccgcgggcggccaggcaacgtgcgtgtctctgccatgtggcagaagtgctctttgtggcagtggccaggcagggagtgtctgcagtcctggtggggctgagcctgaggccttccagaaagcaggagcagctgtgctgcaccccatgtgggtgaccaggtcctttctcctgatagtcacctgctggttgttgccaggttgcagctgctcttgcatctgggccagaagtcctccctcctgcaggctggctgttggcccctctgctgtcctgcagtagaaggtgccgtgagcaggctttgggaacactggcctgggtctccctggtggggtgtgcatgccacgccccgtgtctggatgcacagatgccatggcctgtgctgggccagtggctgggggtgctagacacccggcaccattctcccttctctcttttcttctcaggatttaaaatttaattatatcagtaaagagattaattttaacgtaactctttctatgcccgtgtaaagtatgtgaatcgcaaggcctgtgctgcatgcgacagcgtccggggtggtggacagggcccccggccacgctccctctcctgtagccactggcatagccctcctgagcacccgctgacatttccgttgtacatgttcctgtttatgcattcacaaggtgactgggatgtagagaggcgttagtgggcaggtggccacagcaggactgaggacaggcccccattatcctaggggtgcgctcacctgcagcccctcctcctcgggcacagacgactgtcgttctccacccaccagtcagggacagcagcctccctgtcactcagctgagaaggccagccctccctggctgtgagcagcctccactgtgtccagagacatgggcctcccactcctgttccttgctagccctggggtggcgtctgcctaggagctggctggcaggtgttgggacctgctgctccatggatgcatgccctaagagtgtcactgagctgtgttttgtctgagcctctctcggtcaacagcaaagcttggtgtcttggcactgttagtgacagagcccagcatcccttctgcccccgttccagctgacatcttgcacggtgaccccttttagtcaggagagtgcagatctgtgctcatcggagactgccccacggccctgtcagagccgccactcctatccccaggccaggtccctggaccagcctcctgtttgcaggcccagaggagccaagtcattaaaatggaagtggattctggatggccgggctgctgctgatgtaggagctggatttgggagctctgcttgccgactggctgtgagacgaggcaggggctctgcttcctcagccctagaggcgagccaggcaaggttggcgactgtcatgtggcttggtttggtcatgcccgtcgatgttttgggtattgaatgtggtaagtggaggaaatgttggaactctgtgcaggtgctgccttgagacccccaagcttccacctgtccctctcctatgtggcagctggggagcagctgagatgtggacttgtatgctgcccacatacgtgagggggagctgaaagggagcccctcctctgagcagcctctgccaggcctgtatgaggcttttcccaccagctcccaacagaggcctcccccagccaggaccacctcgtcctcgtggcggggcagcaggagcggtagaaaggggtccgatgtttgaggaggcccttaagggaagctactgaattataacacgtaagaaaatcaccattccgtattggttgggggctcctgtttctcatcctagctttttcctggaaagcccgctagaaggtttgggaacgaggggaaagttctcagaactgttggctgctccccacccgcctcccgcctcccccgcaggttatgtcagcagctctgagacagcagtatcacaggccagatgttgttcctggctagatgtttacatttgtaagaaataacactgtgaatgtaaaacagagccattcccttggaatgcatatcgctgggctcaacatagagtttgtcttcctcttgtttacgacgtgatctaaaccagtccttagcaaggggctcagaacaccccgctctggcagtaggtgtcccccacccccaaagacctgcctgtgtgctccggagatgaatatgagctcattagtaaaaatgacttcacccacgcatatacataaagtatccatgcatgtgcatatagacacatctataattttacacacacacctctcaagacggagatgcatggcctctaagagtgcccgtgtcggttcttcctggaagttgactttccttagacccgccaggtcaagttagccgcgtgacggacatccaggcgtgggacgtggtcagggcagggctcattcattgcccactaggatcccactggcgaagatggtctccatatcagctctctgcagaagggaggaagactttatcatgttcctaaaaatctgtggcaagcacccatcgtattatccaaattttgttgcaaatgtgattaatttggttgtcaagttttgggggtgggctgtggggagattgcttttgttttcctgctggtaatatcgggaaagattttaatgaaaccagggtagaattgtttggcaatgcactgaagcgtgtttctttcccaaaatgtgcctcccttccgctgcgggcccagctgagtctatgtaggtgatgtttccagctgccaagtgctctttgttactgtccaccctcatttctgccagcgcatgtgtcctttcaaggggaaaatgtgaagctgaaccccctccagacacccagaatgtagcatctgagaaggccctgtgccctaaaggacacccctcgcccccatcttcatggagggggtcatttcagagccctcggagccaatgaacagctcctcctcttggagctgagatgagccccacgtggagctcgggacggatagtagacagcaataactcggtgtgtggccgcctggcaggtggaacttcctcccgttgcggggtggagtgaggttagttctgtgtgtctggtgggtggagtcaggcttctcttgctacctgtgagcatccttcccagcagacatcctcatcgggctttgtccctcccccgcttcctccctctgcggggaggacccgggaccacagctgctggccagggtagacttggagctgtcctccagaggggtcacgtgtaggagtgagaagaaggaagatcttgagagctgctgagggaccttggagagctcaggatggctcagacgaggacactcgcttgccgggcctgggcctcctgggaaggagggagctgctcagaatgccgcatgacaactgaaggcaacctggaaggttcaggggccgctcttcccccatgtgcctgtcacgctctggtgcagtcaaaggaacgccttcccctcagttgtttctaagagcagagtctcccgctgcaatctgggtggtaactgccagccttggaggatcgtggccaacgtggacctgcctacggagggtgggctctgacccaagtggggcctccttgtccaggtctcactgctttgcaccgtggtcagagggactgtcagctgagcttgagctcccctggagccagcagggctgtgatgggcgagtcccggagccccacccagacctgaatgcttctgagagcaaagggaaggactgacgagagatgtatatttaattttttaactgctgcaaacattgtacatccaaattaaaggaaaaaaatggaaaccatca

SEQ ID NO: 3 - DNA, 20 bp, synthetic construct
  source 1..20: mol_type = other DNA
gggaccctgatcaacaccat

SEQ ID NO: 4 - DNA, 24 bp, synthetic construct
  source 1..24: mol_type = other DNA
ccagttcttgattttgtcgaaaca

SEQ ID NO: 5 - DNA, 18 bp, synthetic construct
  source 1..18: mol_type = other DNA
tgggtggtctccgcggcc

SEQ ID NO: 6-8 - skipped (3 entries)

SEQ ID NO: 9 - DNA, 20 bp, synthetic construct
  source 1..20: mol_type = other DNA
ccttccctgaaggttcctcc

SEQ ID NO: 10 - DNA, 15 bp, synthetic construct
  source 1..15: mol_type = other DNA
taaattgtcatcacc

SEQ ID NO: 11 - DNA, 15 bp, synthetic construct
  source 1..15: mol_type = other DNA
  modified_base 8: mod_base = OTHER; note = uracil
taaattgtcatcacc

SEQ ID NO: 12 - DNA, 15 bp, synthetic construct
  source 1..15: mol_type = other DNA
taaattgncatcacc

SEQ ID NO: 13 - DNA, 15 bp, synthetic construct
  source 1..15: mol_type = other DNA
  modified_base 5: mod_base = OTHER; note = uracil
taaattgtcatcacc

SEQ ID NO: 14 - DNA, 16 bp, synthetic construct
  source 1..16: mol_type = other DNA
taaattgtcatcacca

SEQ ID NO: 15 - DNA, 18 bp, synthetic construct
  source 1..18: mol_type = other DNA
taaattgtcatcacctta

SEQ ID NO: 16 - DNA, 20 bp, synthetic construct
  source 1..20: mol_type = other DNA
taaattgtcatcaccattta

SEQ ID NO: 17 - DNA, 17 bp, synthetic construct
  source 1..17: mol_type = other DNA
taaattgtcatcaccta

SEQ ID NO: 18 - DNA, 19 bp, synthetic construct
  source 1..19: mol_type = other DNA
taaattgtcatcaccttta

SEQ ID NO: 19 - DNA, 16 bp, synthetic construct
  source 1..16: mol_type = other DNA
gtaaattgtcatcacc

SEQ ID NO: 20 - DNA, 17 bp, synthetic construct
  source 1..17: mol_type = other DNA
ggtaaattgtcatcacc

SEQ ID NO: 21 - DNA, 18 bp, synthetic construct
  source 1..18: mol_type = other DNA
ggttaaattgtcatcacc

SEQ ID NO: 22 - DNA, 19 bp, synthetic construct
  source 1..19: mol_type = other DNA
ggtgtaaattgtcatcacc

SEQ ID NO: 23 - DNA, 20 bp, synthetic construct
  source 1..20: mol_type = other DNA
ggtgataaattgtcatcacc

SEQ ID NO: 24 - DNA, 21 bp, synthetic construct
  source 1..21: mol_type = other DNA
ggctaaattgtcatcaccgcc

SEQ ID NO: 25 - DNA, 19 bp, synthetic construct
  source 1..19: mol_type = other DNA
gctaaattgtcatcaccgc

SEQ ID NO: 26 - DNA, 21 bp, synthetic construct
  source 1..21: mol_type = other DNA
taataaattgtcatcacctta

SEQ ID NO: 27 - DNA, 19 bp, synthetic construct
  source 1..19: mol_type = other DNA
aataaattgtcatcacctt

SEQ ID NO: 28 - DNA, 21 bp, synthetic construct
  source 1..21: mol_type = other DNA
tcttaaattgtcatcaccaga

SEQ ID NO: 29 - DNA, 19 bp, synthetic construct
  source 1..19: mol_type = other DNA
cttaaattgtcatcaccag

SEQ ID NO: 30 - DNA, 18 bp, synthetic construct
  source 1..18: mol_type = other DNA
taataaattgtcatcacc

SEQ ID NO: 31 - DNA, 17 bp, synthetic construct
  source 1..17: mol_type = other DNA
aataaattgtcatcacc

SEQ ID NO: 32 - DNA, 17 bp, synthetic construct
  source 1..17: mol_type = other DNA
ataaattgtcatcacca

SEQ ID NO: 33 - DNA, 17 bp, synthetic construct
  source 1..17: mol_type = other DNA
ataaattctcatcacca

SEQ ID NO: 34 - DNA, 17 bp, synthetic construct
  source 1..17: mol_type = other DNA
ataaatagtcatcacca

SEQ ID NO: 35 - DNA, 17 bp, synthetic construct
  source 1..17: mol_type = other DNA
ataaattgtgatcacca

SEQ ID NO: 36 - DNA, 17 bp, synthetic construct
  source 1..17: mol_type = other DNA
ataaattgtcttcacca

SEQ ID NO: 37 - DNA, 17 bp, synthetic construct
  source 1..17: mol_type = other DNA
ataaattgtcaacacca

SEQ ID NO: 38 - DNA, 15 bp, synthetic construct
  source 1..15: mol_type = other DNA
taaattctcatcacc

SEQ ID NO: 39 - DNA, 15 bp, synthetic construct
  source 1..15: mol_type = other DNA
taaaatgtcatcacc

SEQ ID NO: 40 - DNA, 15 bp, synthetic construct
  source 1..15: mol_type = other DNA
taaattgtgatcacc

SEQ ID NO: 41 - DNA, 15 bp, synthetic construct
  source 1..15: mol_type = other DNA
taaattgtcttcacc

SEQ ID NO: 42 - DNA, 15 bp, synthetic construct
  source 1..15: mol_type = other DNA
taaattgtcaacacc

SEQ ID NO: 43 - DNA, 17 bp, synthetic construct
  source 1..17: mol_type = other DNA
ttaaattgtcatcacca

SEQ ID NO: 44 - DNA, 17 bp, synthetic construct
  source 1..17: mol_type = other DNA
aaaaattgtcatcacca

SEQ ID NO: 45 - DNA, 17 bp, synthetic construct
  source 1..17: mol_type = other DNA
attaattgtcatcacca

SEQ ID NO: 46 - DNA, 17 bp, synthetic construct
  source 1..17: mol_type = other DNA
atatattgtcatcacca

SEQ ID NO: 47 - DNA, 17 bp, synthetic construct
  source 1..17: mol_type = other DNA
ataatttgtcatcacca

SEQ ID NO: 48 - DNA, 17 bp, synthetic construct
  source 1..17: mol_type = other DNA
ataaattgtcatgacca

SEQ ID NO: 49 - DNA, 17 bp, synthetic construct
  source 1..17: mol_type = other DNA
ataaattgtcatctcca

SEQ ID NO: 50 - DNA, 17 bp, synthetic construct
  source 1..17: mol_type = other DNA
ataaattgtcatcagca

SEQ ID NO: 51 - DNA, 17 bp, synthetic construct
  source 1..17: mol_type = other DNA
ataaattgtcatcacga

SEQ ID NO: 52 - DNA, 17 bp, synthetic construct
  source 1..17: mol_type = other DNA
ataaattgtcatcacct

SEQ ID NO: 53 - DNA, 15 bp, synthetic construct
  source 1..15: mol_type = other DNA
taagttgtcatcacc

SEQ ID NO: 54 - DNA, 15 bp, synthetic construct
  source 1..15: mol_type = other DNA
taaagtgtcatcacc

SEQ ID NO: 55 - DNA, 15 bp, synthetic construct
  source 1..15: mol_type = other DNA
taaatggtcatcacc

SEQ ID NO: 56 - DNA, 20 bp, synthetic construct
  source 1..20: mol_type = other DNA
tctctattgcacattccaag

SEQ ID NO: 57 - DNA, 20 bp, synthetic construct
  source 1..20: mol_type = other DNA
ccttccctgaaggttcctcc

SEQ ID NO: 58 - DNA, 17 bp, synthetic construct
  source 1..17: mol_type = other DNA
aattgtcatcaccagaa

SEQ ID NO: 59 - DNA, 17 bp, synthetic construct
  source 1..17: mol_type = other DNA
aattgtcatcaccagaa

SEQ ID NO: 60 - DNA, 17 bp, synthetic construct
  source 1..17: mol_type = other DNA
aaattgtcatcaccaga

SEQ ID NO: 61 - DNA, 17 bp, synthetic construct
  source 1..17: mol_type = other DNA
taaattgtcatcaccag

SEQ ID NO: 62 - DNA, 17 bp, synthetic construct
  source 1..17: mol_type = other DNA
aataaattgtcatcacc

SEQ ID NO: 63 - DNA, 17 bp, synthetic construct
  source 1..17: mol_type = other DNA
taataaattgtcatcac

SEQ ID NO: 64 - DNA, 17 bp, synthetic construct
  source 1..17: mol_type = other DNA
ttaataaattgtcatca

SEQ ID NO: 65 - DNA, 15 bp, synthetic construct
  source 1..15: mol_type = other DNA
attgtcatcaccaga

SEQ ID NO: 66 - DNA, 15 bp, synthetic construct
  source 1..15: mol_type = other DNA
ttaataaattgtcat

SEQ ID NO: 67 - DNA, 15 bp, synthetic construct
  source 1..15: mol_type = other DNA
ttgtcatcaccagaa

SEQ ID NO: 68 - DNA, 15 bp, synthetic construct
  source 1..15: mol_type = other DNA
aattgtcatcaccag

SEQ ID NO: 69 - DNA, 15 bp, synthetic construct
  source 1..15: mol_type = other DNA
aaattgtcatcacca

SEQ ID NO: 70 - DNA, 15 bp, synthetic construct
  source 1..15: mol_type = other DNA
aataaattgtcatca

SEQ ID NO: 71 - DNA, 15 bp, synthetic construct
  source 1..15: mol_type = other DNA
attaataaattgtca

SEQ ID NO: 72 - DNA, 15 bp, synthetic construct
  source 1..15: mol_type = other DNA
tattaataaattgtc

SEQ ID NO: 73 - DNA, 15 bp, synthetic construct
  source 1..15: mol_type = other DNA
gtcatcaccagaaaa

SEQ ID NO: 74 - DNA, 15 bp, synthetic construct
  source 1..15: mol_type = other DNA
tgtcatcaccagaaa

SEQ ID NO: 75 - DNA, 15 bp, synthetic construct
  source 1..15: mol_type = other DNA
ataaattgtcatcac

SEQ ID NO: 76 - DNA, 15 bp, synthetic construct
  source 1..15: mol_type = other DNA
taataaattgtcatc

SEQ ID NO: 77 - DNA, 17 bp, synthetic construct
  source 1..17: mol_type = other DNA
ataaaatgtcatcacca

SEQ ID NO: 78 - DNA, 15 bp, synthetic construct
  source 1..15: mol_type = other DNA
taaatagtcatcacc

SEQ ID NO: 79 - DNA, 20 bp, synthetic construct
  source 1..20: mol_type = other DNA
ctcgactaaagcaggatttc

SEQ ID NO: 80 - DNA, 19 bp, synthetic construct
  source 1..19: mol_type = other DNA
aataaattgtcatcaccag

SEQ ID NO: 81 - DNA, 19 bp, synthetic construct
  source 1..19: mol_type = other DNA
cacagtgctacccaacctt

SEQ ID NO: 82 - DNA, 19 bp, synthetic construct
  source 1..19: mol_type = other DNA
tcacagctatcttctcatc

SEQ ID NO: 83 - DNA, 20 bp, synthetic construct
  source 1..20: mol_type = other DNA
tcccatttcaggagacctgg

SEQ ID NO: 84 - DNA, 20 bp, synthetic construct
  source 1..20: mol_type = other DNA
gctgattagagagaggtccc

SEQ ID NO: 85 - DNA, 16 bp, synthetic construct
  source 1..16: mol_type = other DNA
atcatggctgcagctt

SEQ ID NO: 86 - DNA, 16 bp, synthetic construct
  source 1..16: mol_type = other DNA
ttcagtcatgacttcc

SEQ ID NO: 87 - DNA, 16 bp, synthetic construct
  source 1..16: mol_type = other DNA
tggctgcagcttccga

SEQ ID NO: 88 - DNA, 16 bp, synthetic construct
  source 1..16: mol_type = other DNA
atggctgcagcttccg

SEQ ID NO: 89 - DNA, 16 bp, synthetic construct
  source 1..16: mol_type = other DNA
catggctgcagcttcc

SEQ ID NO: 90 - DNA, 16 bp, synthetic construct
  source 1..16: mol_type = other DNA
tcatggctgcagcttc

SEQ ID NO: 91 - DNA, 16 bp, synthetic construct
  source 1..16: mol_type = other DNA
catcatggctgcagct

SEQ ID NO: 92 - DNA, 16 bp, synthetic construct
  source 1..16: mol_type = other DNA
ccatcatggctgcagc

SEQ ID NO: 93 - DNA, 16 bp, synthetic construct
  source 1..16: mol_type = other DNA
tccatcatggctgcag

SEQ ID NO: 94 - DNA, 16 bp, synthetic construct
  source 1..16: mol_type = other DNA
ttccatcatggctgca

SEQ ID NO: 95 - protein, 3144 aa, Homo sapiens
MATLEKLMKAFESLKSFQQQQQQQQQQQQQQQQQQQQQQQPPPPPPPPPPPQLPQPPPQAQPLLPQPQPPPPPPPPPPGPAVAEEPLHRPKKELSATKKDRVNHCLTICENIVAQSVRNSPEFQKLLGIAMELFLLCSDDAESDVRMVADECLNKVIKALMDSNLPRLQLELYKEIKKNGAPRSLRAALWRFAELAHLVRPQKCRPYLVNLLPCLTRTSKRPEESVQETLAAAVPKIMASFGNFANDNEIKVLLKAFIANLKSSSPTIRRTAAGSAVSICQHSRRTQYFYSWLLNVLLGLLVPVEDEHSTLLILGVLLTLRYLVPLLQQQVKDTSLKGSFGVTRKEMEVSPSAEQLVQVYELTLHHTQHQDHNVVTGALELLQQLFRTPPPELLQTLTAVGGIGQLTAAKEESGGRSRSGSIVELIAGGGSSCSPVLSRKQKGKVLLGEEEALEDDSESRSDVSSSALTASVKDEISGELAASSGVSTPGSAGHDIITEQPRSQHTLQADSVDLASCDLTSSATDGDEEDILSHSSSQVSAVPSDPAMDLNDGTQASSPISDSSQTTTEGPDSAVTPSDSSEIVLDGTDNQYLGLQIGQPQDEDEEATGILPDEASEAFRNSSMALQQAHLLKNMSHCRQPSDSSVDKFVLRDEATEPGDQENKPCRIKGDIGQSTDDDSAPLVHCVRLLSASFLLTGGKNVLVPDRDVRVSVKALALSCVGAAVALHPESFFSKLYKVPLDTTEYPEEQYVSDILNYIDHGDPQVRGATAILCGTLICSILSRSRFHVGDWMGTIRTLTGNTFSLADCIPLLRKTLKDESSVTCKLACTAVRNCVMSLCSSSYSELGLQLIIDVLTLRNSSYWLVRTELLETLAEIDFRLVSFLEAKAENLHRGAHHYTGLLKLQERVLNNVVIHLLGDEDPRVRHVAAASLIRLVPKLFYKCDQGQADPVVAVARDQSSVYLKLLMHETQPPSHFSVSTITRIYRGYNLLPSITDVTMENNLSRVIAAVSHELITSTTRALTFGCCEALCLLSTAFPVCIWSLGWHCGVPPLSASDESRKSCTVGMATMILTLLSSAWFPLDLSAHQDALILAGNLLAASAPKSLRSSWASEEEANPAATKQEEVWPALGDRALVPMVEQLFSHLLKVINICAHVLDDVAPGPAIKAALPSLTNPPSLSPIRRKGKEKEPGEQASVPLSPKKGSEASAASRQSDTSGPVTTSKSSSLGSFYHLPSYLKLHDVLKATHANYKVTLDLQNSTEKFGGFLRSALDVLSQILELATLQDIGKCVEEILGYLKSCFSREPMMATVCVQQLLKTLFGTNLASQFDGLSSNPSKSQGRAQRLGSSSVRPGLYHYCFMAPYTHFTQALADASLRNMVQAEQENDTSGWFDVLQKVSTQLKTNLTSVTKNRADKNAIHNHIRLFEPLVIKALKQYTTTTCVQLQKQVLDLLAQLVQLRVNYCLLDSDQVFIGFVLKQFEYIEVGQFRESEAIIPNIFFFLVLLSYERYHSKQIIGIPKIIQLCDGIMASGRKAVTHAIPALQPIVHDLFVLRGTNKADAGKELETQKEVVVSMLLRLIQYHQVLEMFILVLQQCHKENEDKWKRLSRQIADIILPMLAKQQMHIDSHEALGVLNTLFEILAPSSLRPVDMLLRSMFVTPNTMASVSTVQLWISGILAILRVLISQSTEDIVLSRIQELSFSPYLISCTVINRLRDGDSTSTLEEHSEGKQIKNLPEETFSRFLLQLVGILLEDIVTKQLKVEMSEQQHTFYCQELGTLLMCLIHIFKSGMFRRITAAATRLFRSDGCGGSFYTLDSLNLRARSMITTHPALVLLWCQILLLVNHTDYRWWAEVQQTPKRHSLSSTKLLSPQMSGEEEDSDLAAKLGMCNREIVRRGALILFCDYVCQNLHDSEHLTWLIVNHIQDLISLSHEPPVQDFISAVHRNSAASGLFIQAIQSRCENLSTPTMLKKTLQCLEGIHLSQSGAVLTLYVDRLLCTPFRVLARMVDILACRRVEMLLAANLQSSMAQLPMEELNRIQEYLQSSGLAQRHQRLYSLLDRFRLSTMQDSLSPSPPVSSHPLDGDGHVSLETVSPDKDWYVHLVKSQCWTRSDSALLEGAELVNRIPAEDMNAFMMNSEFNLSLLAPCLSLGMSEISGGQKSALFEAAREVTLARVSGTVQQLPAVHHVFQPELPAEPAAYWSKLNDLFGDAALYQSLPTLARALAQYLVVVSKLPSHLHLPPEKEKDIVKFVVATLEALSWHLIHEQIPLSLDLQAGLDCCCLALQLPGLWSVVSSTEFVTHACSLIYCVHFILEAVAVQPGEQLLSPERRTNTPKAISEEEEEVDPNTQNPKYITAACEMVAEMVESLQSVLALGHKRNSGVPAFLTPLLRNIIISLARLPLVNSYTRVPPLVWKLGWSPKPGGDFGTAFPEIPVEFLQEKEVFKEFIYRINTLGWTSRTQFEETWATLLGVLVTQPLVMEQEESPPEEDTERTQINVLAVQAITSLVLSAMTVPVAGNPAVSCLEQQPRNKPLKALDTRFGRKLSIIRGIVEQEIQAMVSKRENIATHHLYQAWDPVPSLSPATTGALISHEKLLLQINPERELGSMSYKLGQVSIHSVWLGNSITPLREEEWDEEEEEEADAPAPSSPPTSPVNSRKHRAGVDIHSCSQFLLELYSRWILPSSSARRTPAILISEVVRSLLVVSDLFTERNQFELMYVTLTELRRVHPSEDEILAQYLVPATCKAAAVLGMDKAVAEPVSRLLESTLRSSHLPSRVGALHGVLYVLECDLLDDTAKQLIPVISDYLLSNLKGIAHCVNIHSQQHVLVMCATAFYLIENYPLDVGPEFSASIIQMCGVMLSGSEESTPSIIYHCALRGLERLLLSEQLSRLDAESLVKLSVDRVNVHSPHRAMAALGLMLTCMYTGKEKVSPGRTSDPNPAAPDSESVIVAMERVSVLFDRIRKGFPCEARVVARILPQFLDDFFPPQDIMNKVIGEFLSNQQPYPQFMATVVYKVFQTLHSTGQSSMVRDWVMLSLSNFTQRAPVAMATWSLSCFFVSASTSPWVAAILPHVISRMGKLEQVDVNLFCLVATDFYRHQIEEELDRRAFQSVLEVVAAPGSPYHRLLTCLRNVHKVTTC